European Patent Specification EP 3 803 402 B1, published April 26, 2023. Title: Anti-cancer treatment of preselected subjects and screening methods to identify susceptible subjects. Applicant: Technische Universität Dresden. The sequence listing filed with the application follows.

SEQUENCE LISTING (106 sequences)

SEQ ID NO: 1 - DNA, 747 bp, Homo sapiens
atggccggcctcaactccctggaggcggtgaaacgcaagatccaggccctgcagcagcaggcggacgaggcggaagaccgcgcgcagggcctgcagcgggagctggacggcgagcgcgagcggcgcgagaaagctgaaggtgatgtggccgccctcaaccgacgcatccagctcgttgaggaggagttggacagggctcaggaacgactggccacggccctgcagaagctggaggaggcagaaaaagctgcagatgagagtgagagaggaatgaaggtgatagaaaaccgggccatgaaggatgaggagaagatggagattcaggagatgcagctcaaagaggccaagcacattgcggaagaggctgaccgcaaatacgaggaggtagctcgtaagctggtcatcctggagggtgagctggagagggcagaggagcgtgcggaggtgtctgaactaaaatgtggtgacctggaagaagaactcaagaatgttactaacaatctgaaatctctggaggctgcatctgaaaagtattctgaaaaggaggacaaatatgaagaagaaattaaacttctgtctgacaaactgaaagaggctgagacccgtgctgaatttgcagagagaacggttgcaaaactggaaaagacaattgatgacctggaagagaaacttgcccaggccaaagaagagaacgtgggcttacatcagacactggatcagacactaaacgaacttaactgtatataa

SEQ ID NO: 2 - protein, 248 aa, Homo sapiens
MAGLNSLEAVKRKIQALQQQADEAEDRAQGLQRELDGERERREKAEGDVAALNRRIQLVEEELDRAQERLATALQKLEEAEKAADESERGMKVIENRAMKDEEKMEIQEMQLKEAKHIAEEADRKYEEVARKLVILEGELERAEERAEVSELKCGDLEEELKNVTNNLKSLEAASEKYSEKEDKYEEEIKLLSDKLKEAETRAEFAERTVAKLEKTIDDLEEKLAQAKEENVGLHQTLDQTLNELNCI

SEQ ID NO: 3 - DNA, 855 bp, Homo sapiens
atggaggccatcaagaagaaaatgcagatgctgaagttggacaaggagaatgccatcgaccgcgcggagcaggcggaggcggataagaaagccgctgaggacaagtgcaagcaggtggaggaggagctgacgcacctccagaagaaactaaaagggacagaggacgagctggataaatattccgaggacctgaaggacgcgcaggagaagctggagctcacggagaagaaggcctccgacgctgaaggtgatgtggccgccctcaaccgacgcatccagctcgttgaggaggagttggacagggctcaggaacgactggccacggccctgcagaagctggaggaggcagaaaaagctgcagatgagagtgagagaggaatgaaggtgatagaaaaccgggccatgaaggatgaggagaagatggagattcaggagatgcagctcaaagaggccaagcacattgcggaagaggctgaccgcaaatacgaggaggtagctcgtaagctggtcatcctggagggtgagctggagagggcagaggagcgtgcggaggtgtctgaactaaaatgtggtgacctggaagaagaactcaagaatgttactaacaatctgaaatctctggaggctgcatctgaaaagtattctgaaaaggaggacaaatatgaagaagaaattaaacttctgtctgacaaactgaaagaggctgagacccgtgctgaatttgcagagagaacggttgcaaaactggaaaagacaattgatgacctggaagagaaacttgcccaggccaaagaagagaacgtgggcttacatcagacactggatcagacactaaacgaacttaactgtatataa

SEQ ID NO: 4 - protein, 284 aa, Homo sapiens
MEAIKKKMQMLKLDKENAIDRAEQAEADKKAAEDKCKQVEEELTHLQKKLKGTEDELDKYSEDLKDAQEKLELTEKKASDAEGDVAALNRRIQLVEEELDRAQERLATALQKLEEAEKAADESERGMKVIENRAMKDEEKMEIQEMQLKEAKHIAEEADRKYEEVARKLVILEGELERAEERAEVSELKCGDLEEELKNVTNNLKSLEAASEKYSEKEDKYEEEIKLLSDKLKEAETRAEFAERTVAKLEKTIDDLEEKLAQAKEENVGLHQTLDQTLNELNCI

SEQ ID NO: 5 - DNA, 747 bp, Homo sapiens; identical to SEQ ID NO: 1

SEQ ID NO: 6 - protein, 248 aa, Homo sapiens; identical to SEQ ID NO: 2

SEQ ID NO: 7 - DNA, 855 bp, Homo sapiens; identical to SEQ ID NO: 3

SEQ ID NO: 8 - protein, 284 aa, Homo sapiens; identical to SEQ ID NO: 4

SEQ ID NO: 9 - DNA, 681 bp, Homo sapiens
atggagcgagccaggcggattgaaggatggaattccaacgaggctcccccgcctcgtcccaccttggctgaaggtgatgtggccgccctcaaccgacgcatccagctcgttgaggaggagttggacagggctcaggaacgactggccacggccctgcagaagctggaggaggcagaaaaagctgcagatgagagtgagagaggaatgaaggtgatagaaaaccgggccatgaaggatgaggagaagatggagattcaggagatgcagctcaaagaggccaagcacattgcggaagaggctgaccgcaaatacgaggaggtagctcgtaagctggtcatcctggagggtgagctggagagggcagaggagcgtgcggaggtgtctgaactaaaatgtggtgacctggaagaagaactcaagaatgttactaacaatctgaaatctctggaggctgcatctgaaaagtattctgaaaaggaggacaaatatgaagaagaaattaaacttctgtctgacaaactgaaagaggctgagacccgtgctgaatttgcagagagaacggttgcaaaactggaaaagacaattgatgacctggaagagaaacttgcccaggccaaagaagagaacgtgggcttacatcagacactggatcagacactaaacgaacttaactgtatataa

SEQ ID NO: 10 - protein, 226 aa, Homo sapiens
MERARRIEGWNSNEAPPPRPTLAEGDVAALNRRIQLVEEELDRAQERLATALQKLEEAEKAADESERGMKVIENRAMKDEEKMEIQEMQLKEAKHIAEEADRKYEEVARKLVILEGELERAEERAEVSELKCGDLEEELKNVTNNLKSLEAASEKYSEKEDKYEEEIKLLSDKLKEAETRAEFAERTVAKLEKTIDDLEEKLAQAKEENVGLHQTLDQTLNELNCI

SEQ ID NO: 11 - DNA, 270 bp, Homo sapiens
atgaaggtgatagaaaaccgggccatgaaggatgaggagaagatggagattcaggagatgcagctcaaagaggccaagcacattgcggaagaggctgaccgcaaatacgaggaggtagctcgtaagctggtcatcctggagggtgagctggagagggcagaggagcgtgcggaggtgtctgaactaaaatgtggtgacctggaagaagaactcaagaatgttactaacaatctgaaatctctggaggctgcatctgaaaagtattctgaa

SEQ ID NO: 12 - protein, 90 aa, Homo sapiens
MKVIENRAMKDEEKMEIQEMQLKEAKHIAEEADRKYEEVARKLVILEGELERAEERAEVSELKCGDLEEELKNVTNNLKSLEAASEKYSE

SEQ ID NO: 13 - DNA, 744 bp, Homo sapiens
atggtggaggaggagctgacgcacctccagaagaaactaaaagggacagaggacgagctggataaatattccgaggacctgaaggacgcgcaggagaagctggagctcacggagaagaaggcctccgacgctgaaggtgatgtggccgccctcaaccgacgcatccagctcgttgaggaggagttggacagggctcaggaacgactggccacggccctgcagaagctggaggaggcagaaaaagctgcagatgagagtgagagaggaatgaaggtgatagaaaaccgggccatgaaggatgaggagaagatggagattcaggagatgcagctcaaagaggccaagcacattgcggaagaggctgaccgcaaatacgaggaggtagctcgtaagctggtcatcctggagggtgagctggagagggcagaggagcgtgcggaggtgtctgaactaaaatgtggtgacctggaagaagaactcaagaatgttactaacaatctgaaatctctggaggctgcatctgaaaagtattctgaaaaggaggacaaatatgaagaagaaattaaacttctgtctgacaaactgaaagaggctgagacccgtgctgaatttgcagagagaacggttgcaaaactggaaaagacaattgatgacctggaagagaaacttgcccaggccaaagaagagaacgtgggcttacatcagacactggatcagacactaaacgaacttaactgtatataa

SEQ ID NO: 14 - protein, 247 aa, Homo sapiens
MVEEELTHLQKKLKGTEDELDKYSEDLKDAQEKLELTEKKASDAEGDVAALNRRIQLVEEELDRAQERLATALQKLEEAEKAADESERGMKVIENRAMKDEEKMEIQEMQLKEAKHIAEEADRKYEEVARKLVILEGELERAEERAEVSELKCGDLEEELKNVTNNLKSLEAASEKYSEKEDKYEEEIKLLSDKLKEAETRAEFAERTVAKLEKTIDDLEEKLAQAKEENVGLHQTLDQTLNELNCI

SEQ ID NO: 15 - DNA, 663 bp, Homno sapiens
  misc_feature (1)..(2): n is a, c, g, or t
nngggcctgcagcgggagctggacggcgagcgcgagcggcgcgagaaagctgaaggtgatgtggccgccctcaaccgacgcatccagctcgttgaggaggagttggacagggctcaggaacgactggccacggccctgcagaagctggaggaggcagaaaaagctgcagatgagagtgagagaggaatgaaggtgatagaaaaccgggccatgaaggatgaggagaagatggagattcaggagatgcagctcaaagaggccaagcacattgcggaagaggctgaccgcaaatacgaggaggtagctcgtaagctggtcatcctggagggtgagctggagagggcagaggagcgtgcggaggtgtctgaactaaaatgtggtgacctggaagaagaactcaagaatgttactaacaatctgaaatctctggaggctgcatctgaaaagtattctgaaaaggaggacaaatatgaagaagaaattaaacttctgtctgacaaactgaaagaggctgagacccgtgctgaatttgcagagagaacggttgcaaaactggaaaagacaattgatgacctggaagatgagttatacgctcagaagctcaagtacaaagctatcagcgaggaactggaccacgctctcaacgacatgacctctctctga

SEQ ID NO: 16 - protein, 220 aa, Homo sapiens
  misc_feature (1)..(1): Xaa can be any naturally occurring amino acid
XGLQRELDGERERREKAEGDVAALNRRIQLVEEELDRAQERLATALQKLEEAEKAADESERGMKVIENRAMKDEEKMEIQEMQLKEAKHIAEEADRKYEEVARKLVILEGELERAEERAEVSELKCGDLEEELKNVTNNLKSLEAASEKYSEKEDKYEEEIKLLSDKLKEAETRAEFAERTVAKLEKTIDDLEDELYAQKLKYKAISEELDHALNDMTSL

SEQ ID NO: 17 - DNA, 50 bp, Homo sapiens
atgaaggtgatagaaaaccgggccatgaaggatgaggagaagatggagat

SEQ ID NO: 18 - protein, 16 aa, Homo sapiens
MKVIENRAMKDEEKME

SEQ ID NO: 19 - DNA, 511 bp, Homo sapiens
atggggtcctgggctggaagaggggtgacgatcggacccacccccagcagggccagtgcgaacaaagtggaggaggagctgacgcacctccagaagaaactaaaagggacagaggacgagctggataaatattccgaggacctgaaggacgcgcaggagaagctggagctcacggagaagaaggcctccgacgctgaaggtgatgtggccgccctcaaccgacgcatccagctcgttgaggaggagttggacagggctcaggaacgactggccacggccctgcagaagctggaggaggcagaaaaagctgcagatgagagtgagagaggaatgaaggtgatagaaaaccgggccatgaaggatgaggagaagatggagattcaggagatgcagctcaaagaggccaagcacattgcggaagaggctgaccgcaaatacgaggaggtagctcgtaagctggtcatcctggagggtgagctggagagggcagaggagcgtgcggaggtgtctg

SEQ ID NO: 20 - protein, 170 aa, Homo sapiens
MGSWAGRGVTIGPTPSRASANKVEEELTHLQKKLKGTEDELDKYSEDLKDAQEKLELTEKKASDAEGDVAALNRRIQLVEEELDRAQERLATALQKLEEAEKAADESERGMKVIENRAMKDEEKMEIQEMQLKEAKHIAEEADRKYEEVARKLVILEGELERAEERAEVS

SEQ ID NO: 21 - DNA, 307 bp, Homo sapiens
atgaaggtgatagaaaaccgggccatgaaggatgaggagaagatggagattcaggagatgcagctcaaagaggccaagcacattgcggaagaggctgaccgcaaatacgaggaggtagctcgtaagctggtcatcctggagggtgagctggagagggcagaggagcgtgcggaggtgtctgaactaaaatgtggtgacctggaagaagaactcaagaatgttactaacaatctgaaatctctggaggctgcatctgaaaagtattctgaaaaggaggacaaatatgaagaagaaattaaacttctgt

SEQ ID NO: 22 - protein, 102 aa, Homo sapiens
MKVIENRAMKDEEKMEIQEMQLKEAKHIAEEADRKYEEVARKLVILEGELERAEERAEVSELKCGDLEEELKNVTNNLKSLEAASEKYSEKEDKYEEEIKLL

SEQ ID NO: 23 - DNA, 209 bp, Homo sapiens
atggaggccatcaagaagaaaatgcagatgctgaagttggacaaggagaatgccatcgaccgcgcggagcaggcggaggcggataagaaagccgctgaggacaagtgcaagcaggtggaggaggagctgacgcacctccagaagaaactaaaagggacagaggacgagctggataaatattccgaggacctgaaggacgcgcaggagaa

SEQ ID NO: 24 - protein, 69 aa, Homo sapiens
MEAIKKKMQMLKLDKENAIDRAEQAEADKKAAEDKCKQVEEELTHLQKKLKGTEDELDKYSEDLKDAQE

SEQ ID NO: 25 - DNA, 415 bp, Homo sapiens
atgtcttccatgcctgcaaccaagttttctttccctttccatatctttttgtcctgccatctctcagccaggcggattgaaggatggaattccaacgaggctcccccgcctcgtcccaccttggctgaaggtgatgtggccgccctcaaccgacgcatccagctcgttgaggaggagttggacagggctcaggaacgactggccacggccctgcagaagctggaggaggcagaaaaagctgcagatgagagtgagagaggaatgaaggtgatagaaaaccgggccatgaaggatgaggagaagatggagattcaggagatgcagctcaaagaggccaagcacattgcggaagaggctgaccgcaaatacgaggaggtagctcgtaagctggtcatcctggagggtgagctggaga

SEQ ID NO: 26 - protein, 138 aa, Homo sapiens
MSSMPATKFSFPFHIFLSCHLSARRIEGWNSNEAPPPRPTLAEGDVAALNRRIQLVEEELDRAQERLATALQKLEEAEKAADESERGMKVIENRAMKDEEKMEIQEMQLKEAKHIAEEADRKYEEVARKLVILEGELE

SEQ ID NO: 27 - DNA, 290 bp, Homo sapiens
atgaaggtgatagaaaaccgggccatgaaggatgaggagaagatggagattcaggagatgcagctcaaagaggccaagcacattgcggaagaggctgaccgcaaatacgaggaggtagctcgtaagctggtcatcctggagggtgagctggagagggcagaggagcgtgcggaggtgtctgaactaaaatgtggtgacctggaagaagaactcaagaatgttactaacaatctgaaatctctggaggctgcatctgaaaagtattctgaaaaggaggacaaatatgaaga

SEQ ID NO: 28 - protein, 96 aa, Homo sapiens
MKVIENRAMKDEEKMEIQEMQLKEAKHIAEEADRKYEEVARKLVILEGELERAEERAEVSELKCGDLEEELKNVTNNLKSLEAASEKYSEKEDKYE

SEQ ID NO: 29 - DNA, 747 bp, Homo sapiens
atggccggcctcaactccctggaggcggtgaaacgcaagatccaggccctgcagcagcaggcggacgaggcggaagaccgcgcgcagggcctgcagcgggagctggacggcgagcgcgagcggcgcgagaaagctgaaggtgatgtggccgccctcaaccgacgcatccagctcgttgaggaggagttggacagggctcaggaacgactggccacggccctgcagaagctggaggaggcagaaaaagctgcagatgagagtgagagaggaatgaaggtgatagaaaaccgggccatgaaggatgaggagaagatggagattcaggagatgcagctcaaagaggccaagcacattgcggaagaggctgaccgcaaatacgaggaggtagctcgtaagctggtcatcctggagggtgagctggagagggcagaggagcgtgcggaggtgtctgaactaaaatgtggtgacctggaagaagaactcaagaatgttactaacaatctgaaatctctggaggctgcatctgaaaagtattctgaaaaggaggacaaatatgaagaagaaattaaacttctgtctgacaaactgaaagaggctgagacccgtgctgaatttgcagagagaacggttgcaaaactggaaaagacaattgatgacctggaagatgagttatacgctcagaagctcaagtacaaagctatcagcgaggaactggaccacgctctcaacgacatgacctctctctga

SEQ ID NO: 30 - protein, 248 aa, Homo sapiens
MAGLNSLEAVKRKIQALQQQADEAEDRAQGLQRELDGERERREKAEGDVAALNRRIQLVEEELDRAQERLATALQKLEEAEKAADESERGMKVIENRAMKDEEKMEIQEMQLKEAKHIAEEADRKYEEVARKLVILEGELERAEERAEVSELKCGDLEEELKNVTNNLKSLEAASEKYSEKEDKYEEEIKLLSDKLKEAETRAEFAERTVAKLEKTIDDLEDELYAQKLKYKAISEELDHALNDMTSL

SEQ ID NO: 31 - DNA, 747 bp, Homo sapiens; identical to SEQ ID NO: 29

SEQ ID NO: 32 - protein, 248 aa, Homo sapiens; identical to SEQ ID NO: 30

SEQ ID NO: 33 - DNA, 552 bp, Homo sapiens
atggccggcctcaactccctggaggcggtgaaacgcaagatccaggccctgcagcagcaggcggacgaggcggaagaccgcgcgcagggcctgcagcgggagctggacggcgagcgcgagcggcgcgagaaagctgaaggtgatgtggccgccctcaaccgacgcatccagctcgttgaggaggagttggacagggctcaggaacgactggccacggccctgcagaagctggaggaggcagaaaaagctgcagatgagagtgagagaggaatgaaggtgatagaaaaccgggccatgaaggatgaggagaagatggagattcaggagatgcagctcaaagaggccaagcacattgcggaagaggctgaccgcaaatacgaggaggtagctcgtaagctggtcatcctggagggtgagctggagagggcagaggagcgtgcggaggtgtctgaactaaaatgtggtgacctggaagaagaactcaagaatgttactaacaatctgaaatctctggaggctgcatctgaaaagagacggggtctcactatgtga

SEQ ID NO: 34 - protein, 183 aa, Homo sapiens
MAGLNSLEAVKRKIQALQQQADEAEDRAQGLQRELDGERERREKAEGDVAALNRRIQLVEEELDRAQERLATALQKLEEAEKAADESERGMKVIENRAMKDEEKMEIQEMQLKEAKHIAEEADRKYEEVARKLVILEGELERAEERAEVSELKCGDLEEELKNVTNNLKSLEAASEKRRGLTM

SEQ ID NO: 35 - DNA, 522 bp, Homo sapiens
  misc_feature (1)..(2): n is a, c, g, or t
nngaagaaactaaaagggacagaggacgagctggataaatattccgaggacctgaaggacgcgcaggagaagctggagctcacggagaagaaggcctccgacgctgaaggtgatgtggccgccctcaaccgacgcatccagctcgttgaggaggagttggacagggctcaggaacgactggccacggccctgcagaagctggaggaggcagaaaaagctgcagatgagagtgagagaggaatgaaggtgatagaaaaccgggccatgaaggatgaggagaagatggagattcaggagatgcagctcaaagaggccaagcacattgcggaagaggctgaccgcaaatacgaggaggtagctcgtaagctggtcatcctggagggtgagctggagagggcagaggagcgtgcggaggtgtctgaactaaaatgtggtgacctggaagaagaactcaagaatgttactaacaatctgaaatctctggaggctgcatctgaaaagagacggggtctcactatgtga

SEQ ID NO: 36 - protein, 173 aa, Homo sapiens
  misc_feature (1)..(1): Xaa can be any naturally occurring amino acid
XKKLKGTEDELDKYSEDLKDAQEKLELTEKKASDAEGDVAALNRRIQLVEEELDRAQERLATALQKLEEAEKAADESERGMKVIENRAMKDEEKMEIQEMQLKEAKHIAEEADRKYEEVARKLVILEGELERAEERAEVSELKCGDLEEELKNVTNNLKSLEAASEKRRGLTM

SEQ ID NO: 37 - DNA, 333 bp, Homo sapiens
  misc_feature (1)..(2): n is a, c, g, or t
nngctggagagggcagaggagcgtgcggaggtgtctgaactaaaatgtggtgacctggaagaagaactcaagaatgttactaacaatctgaaatctctggaggctgcatctgaaaagtattctgaaaaggaggacaaatatgaagaagaaattaaacttctgtctgacaaactgaaagaggctgagacccgtgctgaatttgcagagagaacggttgcaaaactggaaaagacaattgatgacctggaagagaaacttgcccaggccaaagaagagaacgtgggcttacatcagacactggatcagacactaaacgaacttaactgtatataa

SEQ ID NO: 38 - protein, 110 aa, Homo sapiens
  misc_feature (1)..(1): Xaa can be any naturally occurring amino acid
XLERAEERAEVSELKCGDLEEELKNVTNNLKSLEAASEKYSEKEDKYEEEIKLLSDKLKEAETRAEFAERTVAKLEKTIDDLEEKLAQAKEENVGLHQTLDQTLNELNCI

SEQ ID NO: 39 - DNA, 1686 bp, Homo sapiens
atgtgtggcatttgggcgctgtttggcagtgatgattgcctttctgttcagtgtctgagtgctatgaagattgcacacagaggtccagatgcattccgttttgagaatgtcaatggatacaccaactgctgctttggatttcaccggttggcggtagttgacccgctgtttggaatgcagccaattcgagtgaagaaatatccgtatttgtggctctgttacaatggtgaaatctacaaccataagaagatgcaacagcattttgaatttgaataccagaccaaagtggatggtgagataatccttcatctttatgacaaaggaggaattgagcaaacaatttgtatgttggatggtgtgtttgcatttgttttactggatactgccaataagaaagtgttcctgggtagagatacatatggagtcagacctttgtttaaagcaatgacagaagatggatttttggctgtatgttcagaagctaaaggtcttgttacattgaagcactccgcgactccctttttaaaagtggagccttttcttcctggacactatgaagttttggatttaaagccaaatggcaaagttgcatccgtggaaatggttaaatatcatcactgtcgggatgtacccctgcacgccctctatgacaatgtggagaaactctttccaggttttgagatagaaactgtgaagaacaacctcaggatcctttttaataatgctgtaaagaaacgtttgatgacagacagaaggattggctgccttttatcagggggcttggactccagcttggttgctgccactctgttgaagcagctgaaagaagcccaagtacagtatcctctccagacatttgcaattggcatggaagacagccccgatttactggctgctagaaaggtggcagatcatattggaagtgaacattatgaagtcctttttaactctgaggaaggcattcaggctctggatgaagtcatattttccttggaaacttatgacattacaacagttcgtgcttcagtaggtatgtatttaatttccaagtatattcggaagaacacagatagcgtggtgatcttctctggagaaggatcagatgaacttacgcagggttacatatattttcacaaggctccttctcctgaaaaagccgaggaggagagtgagaggcttctgagggaactctatttgtttgatgttctccgcgcagatcgaactactgctgcccatggtcttgaactgagagtcccatttctagatcatcgattttcttcctattacttgtctctgccaccagaaatgagaattccaaagaatgggatagaaaaacatctcctgagagagacgtttgaggattccaatctgatacccaaagagattctctggcgaccaaaagaagccttcagtgatggaataacttcagttaagaattcctggtttaagattttacaggaatacgttgaacatcaggttgatgatgcaatgatggcaaatgcagcccagaaatttcccttcaatactcctaaaaccaaagaaggatattactaccgtcaagtctttgaacgccattacccaggccgggctgactggctgagccattactggatgcccaagtggatcaatgccactgacccttctgcccgcacgctgacccactacaagtcagctgtcaaagcttag

SEQ ID NO: 40 - protein, 561 aa, Homo sapiens
MCGIWALFGSDDCLSVQCLSAMKIAHRGPDAFRFENVNGYTNCCFGFHRLAVVDPLFGMQPIRVKKYPYLWLCYNGEIYNHKKMQQHFEFEYQTKVDGEIILHLYDKGGIEQTICMLDGVFAFVLLDTANKKVFLGRDTYGVRPLFKAMTEDGFLAVCSEAKGLVTLKHSATPFLKVEPFLPGHYEVLDLKPNGKVASVEMVKYHHCRDVPLHALYDNVEKLFPGFEIETVKNNLRILFNNAVKKRLMTDRRIGCLLSGGLDSSLVAATLLKQLKEAQVQYPLQTFAIGMEDSPDLLAARKVADHIGSEHYEVLFNSEEGIQALDEVIFSLETYDITTVRASVGMYLISKYIRKNTDSVVIFSGEGSDELTQGYIYFHKAPSPEKAEEESERLLRELYLFDVLRADRTTAAHGLELRVPFLDHRFSSYYLSLPPEMRIPKNGIEKHLLRETFEDSNLIPKEILWRPKEAFSDGITSVKNSWFKILQEYVEHQVDDAMMANAAQKFPFNTPKTKEGYYYRQVFERHYPGRADWLSHYWMPKWINATDPSARTLTHYKSAVKA

SEQ ID NO: 41 - DNA, 1686 bp, Homo sapiens; identical to SEQ ID NO: 39

SEQ ID NO: 42 - protein, 561 aa, Homo sapiens; identical to SEQ ID NO: 40

SEQ ID NO: 43 - DNA, 1686 bp, Homo sapiens; identical to SEQ ID NO: 39

SEQ ID NO: 44 - protein, 561 aa, Homo sapiens; identical to SEQ ID NO: 40

SEQ ID NO: 45 - DNA, 1623 bp, Homo sapiens
atgaagattgcacacagaggtccagatgcattccgttttgagaatgtcaatggatacaccaactgctgctttggatttcaccggttggcggtagttgacccgctgtttggaatgcagccaattcgagtgaagaaatatccgtatttgtggctctgttacaatggtgaaatctacaaccataagaagatgcaacagcattttgaatttgaataccagaccaaagtggatggtgagataatccttcatctttatgacaaaggaggaattgagcaaacaatttgtatgttggatggtgtgtttgcatttgttttactggatactgccaataagaaagtgttcctgggtagagatacatatggagtcagacctttgtttaaagcaatgacagaagatggatttttggctgtatgttcagaagctaaaggtcttgttacattgaagcactccgcgactccctttttaaaagtggagccttttcttcctggacactatgaagttttggatttaaagccaaatggcaaagttgcatccgtggaaatggttaaatatcatcactgtcgggatgtacccctgcacgccctctatgacaatgtggagaaactctttccaggttttgagatagaaactgtgaagaacaacctcaggatcctttttaataatgctgtaaagaaacgtttgatgacagacagaaggattggctgccttttatcagggggcttggactccagcttggttgctgccactctgttgaagcagctgaaagaagcccaagtacagtatcctctccagacatttgcaattggcatggaagacagccccgatttactggctgctagaaaggtggcagatcatattggaagtgaacattatgaagtcctttttaactctgaggaaggcattcaggctctggatgaagtcatattttccttggaaacttatgacattacaacagttcgtgcttcagtaggtatgtatttaatttccaagtatattcggaagaacacagatagcgtggtgatcttctctggagaaggatcagatgaacttacgcagggttacatatattttcacaaggctccttctcctgaaaaagccgaggaggagagtgagaggcttctgagggaactctatttgtttgatgttctccgcgcagatcgaactactgctgcccatggtcttgaactgagagtcccatttctagatcatcgattttcttcctattacttgtctctgccaccagaaatgagaattccaaagaatgggatagaaaaacatctcctgagagagacgtttgaggattccaatctgatacccaaagagattctctggcgaccaaaagaagccttcagtgatggaataacttcagttaagaattcctggtttaagattttacaggaatacgttgaacatcaggttgatgatgcaatgatggcaaatgcagcccagaaatttcccttcaatactcctaaaaccaaagaaggatattactaccgtcaagtctttgaacgccattacccaggccgggctgactggctgagccattactggatgcccaagtggatcaatgccactgacccttctgcccgcacgctgacccactacaagtcagctgtcaaagcttag

SEQ ID NO: 46 - protein, 540 aa, Homo sapiens
MKIAHRGPDAFRFENVNGYTNCCFGFHRLAVVDPLFGMQPIRVKKYPYLWLCYNGEIYNHKKMQQHFEFEYQTKVDGEIILHLYDKGGIEQTICMLDGVFAFVLLDTANKKVFLGRDTYGVRPLFKAMTEDGFLAVCSEAKGLVTLKHSATPFLKVEPFLPGHYEVLDLKPNGKVASVEMVKYHHCRDVPLHALYDNVEKLFPGFEIETVKNNLRILFNNAVKKRLMTDRRIGCLLSGGLDSSLVAATLLKQLKEAQVQYPLQTFAIGMEDSPDLLAARKVADHIGSEHYEVLFNSEEGIQALDEVIFSLETYDITTVRASVGMYLISKYIRKNTDSVVIFSGEGSDELTQGYIYFHKAPSPEKAEEESERLLRELYLFDVLRADRTTAAHGLELRVPFLDHRFSSYYLSLPPEMRIPKNGIEKHLLRETFEDSNLIPKEILWRPKEAFSDGITSVKNSWFKILQEYVEHQVDDAMMANAAQKFPFNTPKTKEGYYYRQVFERHYPGRADWLSHYWMPKWINATDPSARTLTHYKSAVKA

SEQ ID NO: 47 - DNA, 1623 bp, homo sapiens; identical to SEQ ID NO: 45

SEQ ID NO: 48 - protein, 540 aa, Homo sapiens; identical to SEQ ID NO: 46

SEQ ID NO: 49 - DNA, 1437 bp, Homo sapiens
atgcaacagcattttgaatttgaataccagaccaaagtggatggtgagataatccttcatctttatgacaaaggaggaattgagcaaacaatttgtatgttggatggtgtgtttgcatttgttttactggatactgccaataagaaagtgttcctgggtagagatacatatggagtcagacctttgtttaaagcaatgacagaagatggatttttggctgtatgttcagaagctaaaggtcttgttacattgaagcactccgcgactccctttttaaaagtggagccttttcttcctggacactatgaagttttggatttaaagccaaatggcaaagttgcatccgtggaaatggttaaatatcatcactgtcgggatgtacccctgcacgccctctatgacaatgtggagaaactctttccaggttttgagatagaaactgtgaagaacaacctcaggatcctttttaataatgctgtaaagaaacgtttgatgacagacagaaggattggctgccttttatcagggggcttggactccagcttggttgctgccactctgttgaagcagctgaaagaagcccaagtacagtatcctctccagacatttgcaattggcatggaagacagccccgatttactggctgctagaaaggtggcagatcatattggaagtgaacattatgaagtcctttttaactctgaggaaggcattcaggctctggatgaagtcatattttccttggaaacttatgacattacaacagttcgtgcttcagtaggtatgtatttaatttccaagtatattcggaagaacacagatagcgtggtgatcttctctggagaaggatcagatgaacttacgcagggttacatatattttcacaaggctccttctcctgaaaaagccgaggaggagagtgagaggcttctgagggaactctatttgtttgatgttctccgcgcagatcgaactactgctgcccatggtcttgaactgagagtcccatttctagatcatcgattttcttcctattacttgtctctgccaccagaaatgagaattccaaagaatgggatagaaaaacatctcctgagagagacgtttgaggattccaatctgatacccaaagagattctctggcgaccaaaagaagccttcagtgatggaataacttcagttaagaattcctggtttaagattttacaggaatacgttgaacatcaggttgatgatgcaatgatggcaaatgcagcccagaaatttcccttcaatactcctaaaaccaaagaaggatattactaccgtcaagtctttgaacgccattacccaggccgggctgactggctgagccattactggatgcccaagtggatcaatgccactgacccttctgcccgcacgctgacccactacaagtcagctgtcaaagcttag

SEQ ID NO: 50 - protein, 478 aa, Homo sapiens
MQQHFEFEYQTKVDGEIILHLYDKGGIEQTICMLDGVFAFVLLDTANKKVFLGRDTYGVRPLFKAMTEDGFLAVCSEAKGLVTLKHSATPFLKVEPFLPGHYEVLDLKPNGKVASVEMVKYHHCRDVPLHALYDNVEKLFPGFEIETVKNNLRILFNNAVKKRLMTDRRIGCLLSGGLDSSLVAATLLKQLKEAQVQYPLQTFAIGMEDSPDLLAARKVADHIGSEHYEVLFNSEEGIQALDEVIFSLETYDITTVRASVGMYLISKYIRKNTDSVVIFSGEGSDELTQGYIYFHKAPSPEKAEEESERLLRELYLFDVLRADRTTAAHGLELRVPFLDHRFSSYYLSLPPEMRIPKNGIEKHLLRETFEDSNLIPKEILWRPKEAFSDGITSVKNSWFKILQEYVEHQVDDAMMANAAQKFPFNTPKTKEGYYYRQVFERHYPGRADWLSHYWMPKWINATDPSARTLTHYKSAVKA

SEQ ID NO: 51 - DNA, 1437 bp, Homo sapiens; identical to SEQ ID NO: 49

SEQ ID NO: 52 - protein, 478 aa, Homo sapiens; identical to SEQ ID NO: 50

SEQ ID NO: 53 - DNA, 644 bp, Homo sapiens
atgtgtggcatttgggcgctgtttggcagtgatgattgcctttctgttcagtgtctgagtgctatgaagattgcacacagaggtccagatgcattccgttttgagaatgtcaatggatacaccaactgctgctttggatttcaccggttggcggtagttgacccgctgtttggaatgcagccaattcgagtgaagaaatatccgtatttgtggctctgttacaatggtgaaatctacaaccataagaagatgcaacagcattttgaatttgaataccagaccaaagtggatggtgagataatccttcatctttatgacaaaggaggaattgagcaaacaatttgtatgttggatggtgtgtttgcatttgttttactggatactgccaataagaaagtgttcctgggtagagatacatatggagtcagacctttgtttaaagcaatgacagaagatggatttttggctgtatgttcagaagctaaaggtcttgttacattgaagcactccgcgactccctttttaaaagtggagccttttcttcctggacactatgaagttttggatttaaagccaaatggcaaagttgcatccgtggaaatggttaaatatcatcactgtcgggatgtacccctgcacgccct

SEQ ID NO: 54 - protein, 214 aa, Homo sapiens
MCGIWALFGSDDCLSVQCLSAMKIAHRGPDAFRFENVNGYTNCCFGFHRLAVVDPLFGMQPIRVKKYPYLWLCYNGEIYNHKKMQQHFEFEYQTKVDGEIILHLYDKGGIEQTICMLDGVFAFVLLDTANKKVFLGRDTYGVRPLFKAMTEDGFLAVCSEAKGLVTLKHSATPFLKVEPFLPGHYEVLDLKPNGKVASVEMVKYHHCRDVPLHA

SEQ ID NO: 55 - DNA, 487 bp, Homo sapiens
atgtgtggcatttgggcgctgtttggcagtgatgattgcctttctgttcagtgtctgagtgctatgaagattgcacacagaggtccagatgcattccgttttgagaatgtcaatggatacaccaactgctgctttggatttcaccggttggcggtagttgacccgctgtttggaatgcagccaattcgagtgaagaaatatccgtatttgtggctctgttacaatggtgaaatctacaaccataagaagatgcaacagcattttgaatttgaataccagaccaaagtggatggtgagataatccttcatctttatgacaaaggaggaattgagcaaacaatttgtatgttggatggtgtgtttgcatttgttttactggatactgccaataagaaagtgttcctgggtagagatacatatggagtcagacctttgtttaaagcaatgacagaagatggatttttggctgtatgttcagaagctaaag

SEQ ID NO: 56 - protein, 162 aa, Homo sapiens
MCGIWALFGSDDCLSVQCLSAMKIAHRGPDAFRFENVNGYTNCCFGFHRLAVVDPLFGMQPIRVKKYPYLWLCYNGEIYNHKKMQQHFEFEYQTKVDGEIILHLYDKGGIEQTICMLDGVFAFVLLDTANKKVFLGRDTYGVRPLFKAMTEDGFLAVCSEAK

SEQ ID NO: 57 - DNA, 85 bp, Homo sapiens
atgtgtggcatttgggcgctgtttggcagtgatgattgcctttctgttcagtgtctgagtgctatgaagattgcacacagaggtc

SEQ ID NO: 58 - protein, 28 aa, Homo sapiens
MCGIWALFGSDDCLSVQCLSAMKIAHRG

SEQ ID NO: 59 - DNA, 356 bp, Homo sapiens
atgtgtggcatttgggcgctgtttggcagtgatgattgcctttctgttcagtgtctgagtgctatgaagattgcacacagaggtccagatgcattccgttttgagaatgtcaatggatacaccaactgctgctttggatttcaccggttggcggtagttgacccgctgtttggaatgcagccaattcgagtgaagaaatatccgtatttgtggctctgttacaatggtgaaatctacaaccataagaagatgcaacagcattttgaatttgaataccagaccaaagtggatggtgagataatccttcatctttatgacaaaggaggaattgagcaaacaatttgtatgttggatgg

SEQ ID NO: 60 - protein, 118 aa, Homo sapiens
MCGIWALFGSDDCLSVQCLSAMKIAHRGPDAFRFENVNGYTNCCFGFHRLAVVDPLFGMQPIRVKKYPYLWLCYNGEIYNHKKMQQHFEFEYQTKVDGEIILHLYDKGGIEQTICMLD

SEQ ID NO: 61 - DNA, 189 bp, Homo sapiens
atgaagattgcacacagaggtccagatgcattccgttttgagaatgtcaatggatacaccaactgctgctttggatttcaccggttggcggtagttgacccgctgtttggaatgcagccaattcgagtgaagaaatatccgtatttgtggctctgttacaatggtgaaatctacaaccataagaaggtg

SEQ ID NO: 62 - protein, 63 aa, Homo sapiens
MKIAHRGPDAFRFENVNGYTNCCFGFHRLAVVDPLFGMQPIRVKKYPYLWLCYNGEIYNHKKV

SEQ ID NO: 63 - DNA, 98 bp, Homo sapiens
atgtgtggcatttgggcgctgtttggcagtgatgattgcctttctgttcagtgtctgagtgctatgaagattgcacacagaggtccagatgcattccg

SEQ ID NO: 64 - protein, 32 aa, Homo sapiens
MCGIWALFGSDDCLSVQCLSAMKIAHRGPDAF

SEQ ID NO: 65 - DNA, 1206 bp, Homo sapiens
atgtgtggcatttgggcgctgtttggcagtgatgattgcctttctgttcagtgtctgagtgctatgaagattgcacacagaggtccagatgcattccgttttgagaatgtcaatggatacaccaactgctgctttggatttcaccggttggcggtagttgacccgctgtttggaatgcagccaattcgagtgaagaaatatccgtatttgtggctctgttacaatggtgaaatctacaaccataagaagatgcaacagcattttgaatttgaataccagaccaaagtggatggtgagataatccttcatctttatgacaaaggaggaattgagcaaacaatttgtatgttggatggtgtgtttgcatttgttttactggatactgccaataagaaagtgttcctgggtagagatacatatggagtcagacctttgtttaaagcaatgacagaagatggatttttggctgtatgttcagaagctaaaggtcttgttacattgaagcactccgcgactccctttttaaaagtggagccttttcttcctggacactatgaagttttggatttaaagccaaatggcaaagttgcatccgtggaaatggttaaatatcatcactgtcgggatgtacccctgcacgccctctatgacaatgtggagaaactctttccaggttttgagatagaaactgtgaagaacaacctcaggatcctttttaataatgctgtaaagaaacgtttgatgacagacagaaggattggctgccttttatcagggggcttggactccagcttggttgctgccactctgttgaagcagctgaaagaagcccaagtacagtatcctctccagacatttgcaattggcatggaagacagccccgatttactggctgctagaaaggtggcagatcatattggaagtgaacattatgaagtcctttttaactctgaggaaggcattcaggctctggatgaagtcatattttccttggaaacttatgacattacaacagttcgtgcttcagtaggtatgtatttaatttccaagtatattcggaagaacacagatagcgtggtgatcttctctggagaaggatcagatgaacttacgcagggttacatatattttcacaaggattggagagggagaaagaaaaactgctttgtgtgccaaaagcaaaactcttggtgtttttgtttgtga

SEQ ID NO: 66 - protein, 401 aa, Homo sapiens
MCGIWALFGSDDCLSVQCLSAMKIAHRGPDAFRFENVNGYTNCCFGFHRLAVVDPLFGMQPIRVKKYPYLWLCYNGEIYNHKKMQQHFEFEYQTKVDGEIILHLYDKGGIEQTICMLDGVFAFVLLDTANKKVFLGRDTYGVRPLFKAMTEDGFLAVCSEAKGLVTLKHSATPFLKVEPFLPGHYEVLDLKPNGKVASVEMVKYHHCRDVPLHALYDNVEKLFPGFEIETVKNNLRILFNNAVKKRLMTDRRIGCLLSGGLDSSLVAATLLKQLKEAQVQYPLQTFAIGMEDSPDLLAARKVADHIGSEHYEVLFNSEEGIQALDEVIFSLETYDITTVRASVGMYLISKYIRKNTDSVVIFSGEGSDELTQGYIYFHKDWRGRKKNCFVCQKQNSWCFCL

SEQ ID NO: 67 - DNA, 888 bp, Homo sapiens
atggagacccctgcctggccccgggtcccgcgccccgagaccgccgtcgctcggacgctcctgctcggctgggtcttcgcccaggtggccggcgcttcaggcactacaaatactgtggcagcatataatttaacttggaaatcaactaatttcaagacaattttggagtgggaacccaaacccgtcaatcaagtctacactgttcaaataagcactaagtcaggagattggaaaagcaaatgcttttacacaacagacacagagtgtgacctcaccgacgagattgtgaaggatgtgaagcagacgtacttggcacgggtcttctcctacccggcagggaatgtggagagcaccggttctgctggggagcctctgtatgagaactccccagagttcacaccttacctggagacaaacctcggacagccaacaattcagagttttgaacaggtgggaacaaaagtgaatgtgaccgtagaagatgaacggactttagtcagaaggaacaacactttcctaagcctccgggatgtttttggcaaggacttaatttatacactttattattggaaatcttcaagttcaggaaagaaaacagccaaaacaaacactaatgagtttttgattgatgtggataaaggagaaaactactgtttcagtgttcaagcagtgattccctcccgaacagttaaccggaagagtacagacagcccggtagagtgtatgggccaggagaaaggggaattcagagaaatattctacatcattggagctgtggtatttgtggtcatcatccttgtcatcatcctggctatatctctacacaagtgtagaaaggcaggagtggggcagagctggaaggagaactccccactgaatgtttcataa

SEQ ID NO: 68 - protein, 295 aa, Homo sapiens
METPAWPRVPRPETAVARTLLLGWVFAQVAGASGTTNTVAAYNLTWKSTNFKTILEWEPKPVNQVYTVQISTKSGDWKSKCFYTTDTECDLTDEIVKDVKQTYLARVFSYPAGNVESTGSAGEPLYENSPEFTPYLETNLGQPTIQSFEQVGTKVNVTVEDERTLVRRNNTFLSLRDVFGKDLIYTLYYWKSSSSGKKTAKTNTNEFLIDVDKGENYCFSVQAVIPSRTVNRKSTDSPVECMGQEKGEFREIFYIIGAVVFVVIILVIILAISLHKCRKAGVGQSWKENSPLNVS

SEQ ID NO: 69 - DNA, 717 bp, Homo sapiens
atggagacccctgcctggccccgggtcccgcgccccgagaccgccgtcgctcggacgctcctgctcggctgggtcttcgcccaggtggccggcgcttcaggcactacaaatactgtggcagcatataatttaacttggaaatcaactaatttcaagacaattttggagtgggaacccaaacccgtcaatcaagtctacactgttcaaataagcactaagtcaggagattggaaaagcaaatgcttttacacaacagacacagagtgtgacctcaccgacgagattgtgaaggatgtgaagcagacgtacttggcacgggtcttctcctacccggcagggaatgtggagagcaccggttctgctggggagcctctgtatgagaactccccagagttcacaccttacctggagacaaacctcggacagccaacaattcagagttttgaacaggtgggaacaaaagtgaatgtgaccgtagaagatgaacggactttagtcagaaggaacaacactttcctaagcctccgggatgtttttggcaaggacttaatttatacactttattattggaaatcttcaagttcaggaaagaaatattctacatcattggagctgtggtatttgtggtcatcatccttgtcatcatcctggctatatctctacacaagtgtagaaaggcaggagtggggcagagctggaaggagaactccccactga

SEQ ID NO: 70 - protein, 238 aa, Homo sapiens
METPAWPRVPRPETAVARTLLLGWVFAQVAGASGTTNTVAAYNLTWKSTNFKTILEWEPKPVNQVYTVQISTKSGDWKSKCFYTTDTECDLTDEIVKDVKQTYLARVFSYPAGNVESTGSAGEPLYENSPEFTPYLETNLGQPTIQSFEQVGTKVNVTVEDERTLVRRNNTFLSLRDVFGKDLIYTLYYWKSSSSGKKYSTSLELWYLWSSSLSSSWLYLYTSVERQEWGRAGRRTPH

SEQ ID NO: 71 - DNA, 2460 bp, Homo sapiens
atggggtctggcgcgcgctttccctcggggacccttcgtgtccggtggttgctgttgcttggcctggtgggcccagtcctcggtgcggcgcggccaggctttcaacagacctcacatctttcttcttatgaaattataactccttggagattaactagagaaagaagagaagcccctaggccctattcaaaacaagtatcttatgttattcaggctgaaggaaaagagcatattattcacttggaaaggaacaaagaccttttgcctgaagattttgtggtttatacttacaacaaggaagggactttaatcactgaccatcccaatatacagaatcattgtcattatcggggctatgtggagggagttcataattcatccattgctcttagcgactgttttggactcagaggattgctgcatttagagaatgcgagttatgggattgaacccctgcagaacagctctcattttgagcacatcatttatcgaatggatgatgtctacaaagagcctctgaaatgtggagtttccaacaaggatatagagaaagaaactgcaaaggatgaagaggaagagcctcccagcatgactcagctacttcgaagaagaagagctgtcttgccacagacccggtatgtggagctgttcattgtcgtagacaaggaaaggtatgacatgatgggaagaaatcagactgctgtgagagaagagatgattctcctggcaaactacttggatagtatgtatattatgttaaatattcgaattgtgctagttggactggagatttggaccaatggaaacctgatcaacatagttgggggtgctggtgatgtgctggggaacttcgtgcagtggcgggaaaagtttcttatcacacgtcggagacatgacagtgcacagctagttctaaagaaaggttttggtggaactgcaggaatggcatttgtgggaacagtgtgttcaaggagccacgcaggcgggattaatgtgtttggacaaatcactgtggagacatttgcttccattgttgctcatgaattgggtcataatcttggaatgaatcacgatgatgggagagattgttcctgtggagcaaagagctgcatcatgaattcaggagcatcgggttccagaaactttagcagttgcagtgcagaggactttgagaagttaactttaaataaaggaggaaactgccttcttaatattccaaagcctgatgaagcctatagtgctccctcctgtggtaataagttggtggacgctggggaagagtgtgactgtggtactccaaaggaatgtgaattggacccttgctgcgaaggaagtacctgtaagcttaaatcatttgctgagtgtgcatatggtgactgttgtaaagactgtcggttccttccaggaggtactttatgccgaggaaaaaccagtgagtgtgatgttccagagtactgcaatggttcttctcagttctgtcagccagatgtttttattcagaatggatatccttgccagaataacaaagcctattgctacaacggcatgtgccagtattatgatgctcaatgtcaagtcatctttggctcaaaagccaaggctgcccccaaagattgtttcattgaagtgaattctaaaggtgacagatttggcaattgtggtttctctggcaatgaatacaagaagtgtgccactgggaatgctttgtgtggaaagcttcagtgtgagaatgtacaagagatacctgtatttggaattgtgcctgctattattcaaacgcctagtcgaggcaccaaatgttggggtgtggatttccagctaggatcagatgttccagatcctgggatggttaacgaaggcacaaaatgtggtgctggaaagatctgtagaaacttccagtgtgtagatgcttctgttctgaattatgactgtgatgttcagaaaaagtgtcatggacatggggtatgtaatagcaataagaattgtcactgtgaaaatggctgggctcccccaaattgtgagactaaaggatacggaggaagtgtggacagtggacctacatacaatgaaatgaatactgcattgagggacggacttctggtcttcttcttcctaattgttccccttattgtctgtgctatttttatcttcatcaagagggatcaactgtggagaagctacttcagaaagaagagatcacaaacatatgagtcagatggcaaaaatcaagcaaacccttctagacagccggggagtgttcctcgacatgtttctccagtgacacctcccagagaagttcctatatatgcaaacagatttgcagtaccaacctatgcagccaagcaacctcagcagttcccatcaaggccacctccaccacaaccgaaagtatcatctcagggaaacttaattcctgcccgtcctgctcctgcacctcctttatatagttccctcacttga

SEQ ID NO: 72 - protein, 819 aa, Homo sapiens
MGSGARFPSGTLRVRWLLLLGLVGPVLGAARPGFQQTSHLSSYEIITPWRLTRERREAPRPYSKQVSYVIQAEGKEHIIHLERNKDLLPEDFVVYTYNKEGTLITDHPNIQNHCHYRGYVEGVHNSSIALSDCFGLRGLLHLENASYGIEPLQNSSHFEHIIYRMDDVYKEPLKCGVSNKDIEKETAKDEEEEPPSMTQLLRRRRAVLPQTRYVELFIVVDKERYDMMGRNQTAVREEMILLANYLDSMYIMLNIRIVLVGLEIWTNGNLINIVGGAGDVLGNFVQWREKFLITRRRHDSAQLVLKKGFGGTAGMAFVGTVCSRSHAGGINVFGQITVETFASIVAHELGHNLGMNHDDGRDCSCGAKSCIMNSGASGSRNFSSCSAEDFEKLTLNKGGNCLLNIPKPDEAYSAPSCGNKLVDAGEECDCGTPKECELDPCCEGSTCKLKSFAECAYGDCCKDCRFLPGGTLCRGKTSECDVPEYCNGSSQFCQPDVFIQNGYPCQNNKAYCYNGMCQYYDAQCQVIFGSKAKAAPKDCFIEVNSKGDRFGNCGFSGNEYKKCATGNALCGKLQCENVQEIPVFGIVPAIIQTPSRGTKCWGVDFQLGSDVPDPGMVNEGTKCGAGKICRNFQCVDASVLNYDCDVQKKCHGHGVCNSNKNCHCENGWAPPNCETKGYGGSVDSGPTYNEMNTALRDGLLVFFFLIVPLIVCAIFIFIKRDQLWRSYFRKKRSQTYESDGKNQANPSRQPGSVPRHVSPVTPPREVPIYANRFAVPTYAAKQPQQFPSRPPPPQPKVSSQGNLIPARPAPAPPLYSSLT

SEQ ID NO: 73 - DNA, 387 bp, Homo sapiens
atggggtctggcgcgcgctttccctcggggacccttcgtgtccggtggttgctgttgcttggcctggtgggcccagtcctcggtgcggcgcggccaggctttcaacagacctcacatctttcttcttatgaaattataactccttggagattaactagagaaagaagagaagcccctaggccctattcaaaacaagtatcttatgttattcaggctgaaggaaaagagcatattattcacttggaaaggaacaaagaccttttgcctgaagattttgtggtttatacttacaacaaggaagggactttaatcactgaccatcccaatatacaggtaatgtatttttctcttgatcccatagcaaattttaaaacaattataatttaa

SEQ ID NO: 74 - protein, 128 aa, Homo sapiens
MGSGARFPSGTLRVRWLLLLGLVGPVLGAARPGFQQTSHLSSYEIITPWRLTRERREAPRPYSKQVSYVIQAEGKEHIIHLERNKDLLPEDFVVYTYNKEGTLITDHPNIQVMYFSLDPIANFKTIII

SEQ ID NO: 75 - DNA, 444 bp, Homo sapiens
atggggtctggcgcgcgctttccctcggggacccttcgtgtccggtggttgctgttgcttggcctggtgggcccagtcctcggtgcggcgcggccaggctttcaacagacctcacatctttcttcttatgaaattataactccttggagattaactagagaaagaagagaagcccctaggccctattcaaaacaagtatcttatgttattcaggctgaaggaaaagagcatattattcacttggaaaggaacaaagaccttttgcctgaagattttgtggtttatacttacaacaaggaagggactttaatcactgaccatcccaatatacagaggtgtggtcctctctgcatcagagaacagagtactcctggggacagagctggccagaatacccaaaataattggcagatgtcaaatttggctttctgtgtttattactag

SEQ ID NO: 76 - protein, 147 aa, Homo sapiens
MGSGARFPSGTLRVRWLLLLGLVGPVLGAARPGFQQTSHLSSYEIITPWRLTRERREAPRPYSKQVSYVIQAEGKEHIIHLERNKDLLPEDFVVYTYNKEGTLITDHPNIQRCGPLCIREQSTPGDRAGQNTQNNWQMSNLAFCVYY

SEQ ID NO: 77 - DNA, 1968 bp, Homo sapiens
atggggtctggcgcgcgctttccctcggggacccttcgtgtccggtggttgctgttgcttggcctggtgggcccagtcctcggtgcggcgcggccaggctttcaacagacctcacatctttcttcttatgaaattataactccttggagattaactagagaaagaagagaagcccctaggccctattcaaaacaagtatcttatgttattcaggctgaaggaaaagagcatattattcacttggaaaggaacaaagaccttttgcctgaagattttgtggtttatacttacaacaaggaagggactttaatcactgaccatcccaatatacagaatcattgtcattatcggggctatgtggagggagttcataattcatccattgctcttagcgactgttttggactcagaggattgctgcatttagagaatgcgagttatgggattgaacccctgcagaacagctctcattttgagcacatcatttatcgaatggatgatgtctacaaagagcctctgaaatgtggagtttccaacaaggatatagagaaagaaactgcaaaggatgaagaggaagagcctcccagcatgactcagctacttcgaagaagaagagctgtcttgccacagacccggtatgtggagctgttcattgtcgtagacaaggaaaggtatgacatgatgggaagaaatcagactgctgtgagagaagagatgattctcctggcaaactacttggatagtatgtatattatgttaaatattcgaattgtgctagttggactggagatttggaccaatggaaacctgatcaacatagttgggggtgctggtgatgtgctggggaacttcgtgcagtggcgggaaaagtttcttatcacacgtcggagacatgacagtgcacagctagttctaaagaaaggttttggtggaactgcaggaatggcatttgtgggaacagtgtgttcaaggagccacgcaggcgggattaatgtgtttggacaaatcactgtggagacatttgcttccattgttgctcatgaattgggtcataatcttggaatgaatcacgatgatgggagagattgttcctgtggagcaaagagctgcatcatgaattcaggagcatcgggttccagaaactttagcagttgcagtgcagaggactttgagaagttaactttaaataaaggaggaaactgccttcttaatattccaaagcctgatgaagcctatagtgctccctcctgtggtaataagttggtggacgctggggaagagtgtgactgtggtactccaaaggaatgtgaattggacccttgctgcgaaggaagtacctgtaagcttaaatcatttgctgagtgtgcatatggtgactgttgtaaagactgtcggttccttccaggaggtactttatgccgaggaaaaaccagtgagtgtgatgttccagagtactgcaatggttcttctcagttctgtcagccagatgtttttattcagaatggatatccttgccagaataacaaagcctattgctacaacggcatgtgccagtattatgatgctcaatgtcaagtcatctttggctcaaaagccaaggctgcccccaaagattgtttcattgaagtgaattctaaaggtgacagatttggcaattgtggtttctctggcaatgaatacaagaagtgtgccactgggaatgctttgtgtggaaagcttcagtgtgagaatgtacaagagatacctgtatttggaattgtgcctgctattattcaaacgcctagtcgaggcaccaaatgttggggtgtggatttccagctaggatcagatgttccagatcctgggatggttaacgaaggcacaaaatgtggtgctggaaagatctgtagaaacttccagtgtgtagatgcttctgttctgaattatgactgtgatgttcagaaaaagtgtcatggacatgggaaatga

SEQ ID NO: 78 - protein, 655 aa, Homo sapiens
MGSGARFPSGTLRVRWLLLLGLVGPVLGAARPGFQQTSHLSSYEIITPWRLTRERREAPRPYSKQVSYVIQAEGKEHIIHLERNKDLLPEDFVVYTYNKEGTLITDHPNIQNHCHYRGYVEGVHNSSIALSDCFGLRGLLHLENASYGIEPLQNSSHFEHIIYRMDDVYKEPLKCGVSNKDIEKETAKDEEEEPPSMTQLLRRRRAVLPQTRYVELFIVVDKERYDMMGRNQTAVREEMILLANYLDSMYIMLNIRIVLVGLEIWTNGNLINIVGGAGDVLGNFVQWREKFLITRRRHDSAQLVLKKGFGGTAGMAFVGTVCSRSHAGGINVFGQITVETFASIVAHELGHNLGMNHDDGRDCSCGAKSCIMNSGASGSRNFSSCSAEDFEKLTLNKGGNCLLNIPKPDEAYSAPSCGNKLVDAGEECDCGTPKECELDPCCEGSTCKLKSFAECAYGDCCKDCRFLPGGTLCRGKTSECDVPEYCNGSSQFCQPDVFIQNGYPCQNNKAYCYNGMCQYYDAQCQVIFGSKAKAAPKDCFIEVNSKGDRFGNCGFSGNEYKKCATGNALCGKLQCENVQEIPVFGIVPAIIQTPSRGTKCWGVDFQLGSDVPDPGMVNEGTKCGAGKICRNFQCVDASVLNYDCDVQKKCHGHGK

SEQ ID NO: 79 - DNA, 2139 bp, Homo sapiens
atggggtctggcgcgcgctttccctcggggacccttcgtgtccggtggttgctgttgcttggcctggtgggcccagtcctcggtgcggcgcggccaggctttcaacagacctcacatctttcttcttatgaaattataactccttggagattaactagagaaagaagagaagcccctaggccctattcaaaacaagtatcttatgttattcaggctgaaggaaaagagcatattattcacttggaaaggaacaaagaccttttgcctgaagattttgtggtttatacttacaacaaggaagggactttaatcactgaccatcccaatatacagaatcattgtcattatcggggctatgtggagggagttcataattcatccattgctcttagcgactgttttggactcagaggattgctgcatttagagaatgcgagttatgggattgaacccctgcagaacagctctcattttgagcacatcatttatcgaatggatgatgtctacaaagagcctctgaaatgtggagtttccaacaaggatatagagaaagaaactgcaaaggatgaagaggaagagcctcccagcatgactcagctacttcgaagaagaagagctgtcttgccacagacccggtatgtggagctgttcattgtcgtagacaaggaaaggtatgacatgatgggaagaaatcagactgctgtgagagaagagatgattctcctggcaaactacttggatagtatgtatattatgttaaatattcgaattgtgctagttggactggagatttggaccaatggaaacctgatcaacatagttgggggtgctggtgatgtgctggggaacttcgtgcagtggcgggaaaagtttcttatcacacgtcggagacatgacagtgcacagctagttctaaagaaaggttttggtggaactgcaggaatggcatttgtgggaacagtgtgttcaaggagccacgcaggcgggattaatgtgtttggacaaatcactgtggagacatttgcttccattgttgctcatgaattgggtcataatcttggaatgaatcacgatgatgggagagattgttcctgtggagcaaagagctgcatcatgaattcaggagcatcgggttccagaaactttagcagttgcagtgcagaggactttgagaagttaactttaaataaaggaggaaactgccttcttaatattccaaagcctgatgaagcctatagtgctccctcctgtggtaataagttggtggacgctggggaagagtgtgactgtggtactccaaaggaatgtgaattggacccttgctgcgaaggaagtacctgtaagcttaaatcatttgctgagtgtgcatatggtgactgttgtaaagactgtcggttccttccaggaggtactttatgccgaggaaaaaccagtgagtgtgatgttccagagtactgcaatggttcttctcagttctgtcagccagatgtttttattcagaatggatatccttgccagaataacaaagcctattgctacaacggcatgtgccagtattatgatgctcaatgtcaagtcatctttggctcaaaagccaaggctgcccccaaagattgtttcattgaagtgaattctaaaggtgacagatttggcaattgtggtttctctggcaatgaatacaagaagtgtgccactgggaatgctttgtgtggaaagcttcagtgtgagaatgtacaagagatacctgtatttggaattgtgcctgctattattcaaacgcctagtcgaggcaccaaatgttggggtgtggatttccagctaggatcagatgttccagatcctgggatggttaacgaaggcacaaaatgtggtgctggaaagatctgtagaaacttccagtgtgtagatgcttctgttctgaattatgactgtgatgttcagaaaaagtgtcatggacatggggtatgtaatagcaataagaattgtcactgtgaaaatggctgggctcccccaaattgtgagactaaaggatacggaggaagtgtggacagtggacctacatacaatggtcagatggcaaaaatcaagcaaacccttctagacagccggggagtgttcctcgacatgtttctccagtga

SEQ ID NO: 80 - protein, 712 aa, Homo sapiens
MGSGARFPSGTLRVRWLLLLGLVGPVLGAARPGFQQTSHLSSYEIITPWRLTRERREAPRPYSKQVSYVIQAEGKEHIIHLERNKDLLPEDFVVYTYNKEGTLITDHPNIQNHCHYRGYVEGVHNSSIALSDCFGLRGLLHLENASYGIEPLQNSSHFEHIIYRMDDVYKEPLKCGVSNKDIEKETAKDEEEEPPSMTQLLRRRRAVLPQTRYVELFIVVDKERYDMMGRNQTAVREEMILLANYLDSMYIMLNIRIVLVGLEIWTNGNLINIVGGAGDVLGNFVQWREKFLITRRRHDSAQLVLKKGFGGTAGMAFVGTVCSRSHAGGINVFGQITVETFASIVAHELGHNLGMNHDDGRDCSCGAKSCIMNSGASGSRNFSSCSAEDFEKLTLNKGGNCLLNIPKPDEAYSAPSCGNKLVDAGEECDCGTPKECELDPCCEGSTCKLKSFAECAYGDCCKDCRFLPGGTLCRGKTSECDVPEYCNGSSQFCQPDVFIQNGYPCQNNKAYCYNGMCQYYDAQCQVIFGSKAKAAPKDCFIEVNSKGDRFGNCGFSGNEYKKCATGNALCGKLQCENVQEIPVFGIVPAIIQTPSRGTKCWGVDFQLGSDVPDPGMVNEGTKCGAGKICRNFQCVDASVLNYDCDVQKKCHGHGVCNSNKNCHCENGWAPPNCETKGYGGSVDSGPTYNGQMAKIKQTLLDSRGVFLDMFLQ

SEQ ID NO: 81 - DNA, 1887 bp, Homo sapiens
atggggtctggcgcgcgctttccctcggggacccttcgtgtccggtggttgctgttgcttggcctggtgggcccagtcctcggtgcggcgcggccaggctttcaacagacctcacatctttcttcttatgaaattataactccttggagattaactagagaaagaagagaagcccctaggccctattcaaaacaagtatcttatgttattcaggctgaaggaaaagagcatattattcacttggaaaggaacaaagaccttttgcctgaagattttgtggtttatacttacaacaaggaagggactttaatcactgaccatcccaatatacagaatcattgtcattatcggggctatgtggagggagttcataattcatccattgctcttagcgactgttttggactcagaggattgctgcatttagagaatgcgagttatgggattgaacccctgcagaacagctctcattttgagcacatcatttatcgaatggatgatgtctacaaagagcctctgaaatgtggagtttccaacaaggatatagagaaagaaactgcaaaggatgaagaggaagagcctcccagcatgactcagctacttcgaagaagaagagctgtcttgccacagacccggtatgtggagctgttcattgtcgtagacaaggaaaggtatgacatgatgggaagaaatcagactgctgtgagagaagagatgattctcctggcaaactacttggatagtatgtatattatgttaaatattcgaattgtgctagttggactggagatttggaccaatggaaacctgatcaacatagttgggggtgctggtgatgtgctggggaacttcgtgcagtggcgggaaaagtttcttatcacacgtcggagacatgacagtgcacagctagttctaaagaaaggttttggtggaactgcaggaatggcatttgtgggaacagtgtgttcaaggagccacgcaggcgggattaatgtgtttggacaaatcactgtggagacatttgcttccattgttgctcatgaattgggtcataatcttggaatgaatcacgatgatgggagagattgttcctgtggagcaaagagctgcatcatgaattcaggagcatcgggttccagaaactttagcagttgcagtgcagaggactttgagaagttaactttaaataaaggaggaaactgccttcttaatattccaaagcctgatgaagcctatagtgctccctcctgtggtaataagttggtggacgctggggaagagtgtgactgtggtactccaaaggaatgtgaattggacccttgctgcgaaggaagtacctgtaagcttaaatcatttgctgagtgtgcatatggtgactgttgtaaagactgtcggttccttccaggaggtactttatgccgaggaaaaaccagtgagtgtgatgttccagagtactgcaatggttcttctcagttctgtcagccagatgtttttattcagaatggatatccttgccagaataacaaagcctattgctacaacggcatgtgccagtattatgatgctcaatgtcaagtcatctttggctcaaaagccaaggctgcccccaaagattgtttcattgaagtgaattctaaaggtgacagatttggcaattgtggtttctctggcaatgaatacaagaagtgtgccactgggaatgctttgtgtggaaagcttcagtgtgagaatgtacaagagatacctgtatttggaattgtgcctgctattattcaaacgcctagtcgaggcaccaaatgttggggtgtggatttccagctaggatcagatgttccagatcctgggatggttaacgaaggcacaaaatgtggtgctggaaagaaatga

SEQ ID NO: 82 - protein, 628 aa, Homo sapiens
MGSGARFPSGTLRVRWLLLLGLVGPVLGAARPGFQQTSHLSSYEIITPWRLTRERREAPRPYSKQVSYVIQAEGKEHIIHLERNKDLLPEDFVVYTYNKEGTLITDHPNIQNHCHYRGYVEGVHNSSIALSDCFGLRGLLHLENASYGIEPLQNSSHFEHIIYRMDDVYKEPLKCGVSNKDIEKETAKDEEEEPPSMTQLLRRRRAVLPQTRYVELFIVVDKERYDMMGRNQTAVREEMILLANYLDSMYIMLNIRIVLVGLEIWTNGNLINIVGGAGDVLGNFVQWREKFLITRRRHDSAQLVLKKGFGGTAGMAFVGTVCSRSHAGGINVFGQITVETFASIVAHELGHNLGMNHDDGRDCSCGAKSCIMNSGASGSRNFSSCSAEDFEKLTLNKGGNCLLNIPKPDEAYSAPSCGNKLVDAGEECDCGTPKECELDPCCEGSTCKLKSFAECAYGDCCKDCRFLPGGTLCRGKTSECDVPEYCNGSSQFCQPDVFIQNGYPCQNNKAYCYNGMCQYYDAQCQVIFGSKAKAAPKDCFIEVNSKGDRFGNCGFSGNEYKKCATGNALCGKLQCENVQEIPVFGIVPAIIQTPSRGTKCWGVDFQLGSDVPDPGMVNEGTKCGAGKK

SEQ ID NO: 83 - DNA, 2901 bp, Homo sapiens
atggcggcggtagcggcagtggcggcgcgtaggaggcggtcttgggcgtctttggtactggcttttttaggggtctgcctggggattacccttgctgtggatagaagcaactttaagacctgtgaagagagttctttctgcaagcgacagagaagcatacggccaggcctctctccataccgagccttgctggactctctacagcttggtcctgattccctcacggtccatctgatccatgaggtcaccaaggtgttgctggtgctagagcttcaggggcttcaaaagaacatgactcggttcaggattgatgagctggagcctcggcgaccccgataccgtgtaccagatgttttggtggctgatccaccaatagcccggctttctgtctctggtcgtgatgagaacagtgtggagttaaccatggctgagggaccctacaagatcatcttgacagcacggccattccgccttgacctactagaggaccgaagtcttttgcttagtgtcaatgcccgaggactcttggagtttgagcatcagagggcccctagggtctctttctcggataaggttaatctcacgcttggtagcatatgggataagatcaagaaccttttctctaggcaaggatcaaaagacccagctgagggcgatggggcccagcctgaggaaacacccagggatggcgacaagccagaggagactcaggggaaggcagagaaagatgagccaggagcctgggaggagacattcaaaactcactctgacagcaagccgtatggccccatgtctgtgggtttggacttctctctgccaggcatggagcatgtctatgggatccctgagcatgcagacaacctgaggctgaaggtcactgagggtggggagccatatcgcctctacaatttggatgtgttccagtatgagctgtacaacccaatggccttgtatgggtctgtgcctgtgctcctggcacacaaccctcatcgcgacttgggcatcttctggctcaatgctgcagagacctgggttgatatatcttccaacactgccgggaagaccctgtttgggaagatgatggactacctgcagggctctggggagaccccacagacagatgttcgctggatgtcagagactggcatcattgacgtcttcctgctgctggggccctccatctctgatgttttccggcaatatgctagtctcacaggaacccaggcgttgcccccactcttctccctcggctaccaccagagccgttggaactaccgggacgaggctgatgtgctggaagtggatcagggctttgatgatcacaacctgccctgtgatgtcatctggctagacattgaacatgctgatggcaagcggtatttcacctgggaccccagtcgcttccctcagccccgcaccatgcttgagcgcttggcttctaagaggcggaagctggtggccatcgtagacccccacatcaaggtggactccggctaccgagttcacgaggagctgcggaacctggggctgtatgttaaaacccgggatggctctgactatgagggctggtgctggccaggctcagctggttaccctgacttcactaatcccacgatgagggcctggtgggctaacatgttcagctatgacaattatgagggctcagctcccaacctctttgtctggaatgacatgaacgaaccatctgtgttcaatggtcctgaggtcaccatgctcaaggatgcccagcattatgggggctgggagcaccgggatgtgcataacatctatggcctttatgtgcacatggcgactgctgatgggctgagacagcgctctgggggcatggaacgcccctttgtcctggccagggccttcttcgctggctcccagcgctttggagccgtgtggacaggggacaacactgccgagtgggaccatttgaagatctctattcctatgtgtctcagcttggggctggtgggactttccttctgtggggcggatgtgggtggcttcttcaaaaacccagagccagagctgcttgtgcgctggtaccagatgggtgcttaccagccattcttccgggcacatgcccacttggacactgggcgacgagagccatggctgttaccatctcagcacaatgatataatccgagatgccttgggccagcgatattctttgctgcccttctggtacaccctcttatatcaggcccatcgggaaggcattcctgtcatgaggcccctgtgggtgcagtaccctcaggatgtgactaccttcaatatagatgatcagtacttgcttggggatgcgttgctggttcaccctgtatcagactctggagcccatggtgtccaggtctatctgcctggccaaggggaggtgtggtatgacattcaaagctaccagaagcatcatggtccccagaccctgtacctgcctgtaactctaagcagtatccctgtgttccagcgtggagggacaatcgtgcctcgatggatgcgagtgcggcggtcttcagaatgtatgaaggatgaccccatcactctctttgttgcacttagccctcagggtacagctcaaggagagctctttctggatgatgggcacacgttcaactatcagactcgccaagagttcctgctgcgtcgattctcattctctggcaacacccttgtctccagctcagcagaccctgaaggacactttgagacaccaatctggattgagcgggtggtgataataggggctggaaagccagcagctgtggtactccagacaaaaggatctccagaaagccgcctgtccttccagcatgaccctgagacctctgtgttggtcctgcgcaagcctggcatcaatgtggcatctgattggagtattcacctgcgataa

SEQ ID NO: 84 - protein, 966 aa, Homo sapiens
MAAVAAVAARRRRSWASLVLAFLGVCLGITLAVDRSNFKTCEESSFCKRQRSIRPGLSPYRALLDSLQLGPDSLTVHLIHEVTKVLLVLELQGLQKNMTRFRIDELEPRRPRYRVPDVLVADPPIARLSVSGRDENSVELTMAEGPYKIILTARPFRLDLLEDRSLLLSVNARGLLEFEHQRAPRVSFSDKVNLTLGSIWDKIKNLFSRQGSKDPAEGDGAQPEETPRDGDKPEETQGKAEKDEPGAWEETFKTHSDSKPYGPMSVGLDFSLPGMEHVYGIPEHADNLRLKVTEGGEPYRLYNLDVFQYELYNPMALYGSVPVLLAHNPHRDLGIFWLNAAETWVDISSNTAGKTLFGKMMDYLQGSGETPQTDVRWMSETGIIDVFLLLGPSISDVFRQYASLTGTQALPPLFSLGYHQSRWNYRDEADVLEVDQGFDDHNLPCDVIWLDIEHADGKRYFTWDPSRFPQPRTMLERLASKRRKLVAIVDPHIKVDSGYRVHEELRNLGLYVKTRDGSDYEGWCWPGSAGYPDFTNPTMRAWWANMFSYDNYEGSAPNLFVWNDMNEPSVFNGPEVTMLKDAQHYGGWEHRDVHNIYGLYVHMATADGLRQRSGGMERPFVLARAFFAGSQRFGAVWTGDNTAEWDHLKISIPMCLSLGLVGLSFCGADVGGFFKNPEPELLVRWYQMGAYQPFFRAHAHLDTGRREPWLLPSQHNDIIRDALGQRYSLLPFWYTLLYQAHREGIPVMRPLWVQYPQDVTTFNIDDQYLLGDALLVHPVSDSGAHGVQVYLPGQGEVWYDIQSYQKHHGPQTLYLPVTLSSIPVFQRGGTIVPRWMRVRRSSECMKDDPITLFVALSPQGTAQGELFLDDGHTFNYQTRQEFLLRRFSFSGNTLVSSSADPEGHFETPIWIERVVIIGAGKPAAVVLQTKGSPESRLSFQHDPETSVLVLRKPGINVASDWSIHLR

SEQ ID NO: 85 - DNA, 2544 bp, Homo sapiens
atgactcggttcaggattgatgagctggagcctcggcgaccccgataccgtgtaccagatgttttggtggctgatccaccaatagcccggctttctgtctctggtcgtgatgagaacagtgtggagttaaccatggctgagggaccctacaagatcatcttgacagcacggccattccgccttgacctactagaggaccgaagtcttttgcttagtgtcaatgcccgaggactcttggagtttgagcatcagagggcccctagggtctcgcaaggatcaaaagacccagctgagggcgatggggcccagcctgaggaaacacccagggatggcgacaagccagaggagactcaggggaaggcagagaaagatgagccaggagcctgggaggagacattcaaaactcactctgacagcaagccgtatggccccatgtctgtgggtttggacttctctctgccaggcatggagcatgtctatgggatccctgagcatgcagacaacctgaggctgaaggtcactgagggtggggagccatatcgcctctacaatttggatgtgttccagtatgagctgtacaacccaatggccttgtatgggtctgtgcctgtgctcctggcacacaaccctcatcgcgacttgggcatcttctggctcaatgctgcagagacctgggttgatatatcttccaacactgccgggaagaccctgtttgggaagatgatggactacctgcagggctctggggagaccccacagacagatgttcgctggatgtcagagactggcatcattgacgtcttcctgctgctggggccctccatctctgatgttttccggcaatatgctagtctcacaggaacccaggcgttgcccccactcttctccctcggctaccaccagagccgttggaactaccgggacgaggctgatgtgctggaagtggatcagggctttgatgatcacaacctgccctgtgatgtcatctggctagacattgaacatgctgatggcaagcggtatttcacctgggaccccagtcgcttccctcagccccgcaccatgcttgagcgcttggcttctaagaggcggaagctggtggccatcgtagacccccacatcaaggtggactccggctaccgagttcacgaggagctgcggaacctggggctgtatgttaaaacccgggatggctctgactatgagggctggtgctggccaggctcagctggttaccctgacttcactaatcccacgatgagggcctggtgggctaacatgttcagctatgacaattatgagggctcagctcccaacctctttgtctggaatgacatgaacgaaccatctgtgttcaatggtcctgaggtcaccatgctcaaggatgcccagcattatgggggctgggagcaccgggatgtgcataacatctatggcctttatgtgcacatggcgactgctgatgggctgagacagcgctctgggggcatggaacgcccctttgtcctggccagggccttcttcgctggctcccagcgctttggagccgtgtggacaggggacaacactgccgagtgggaccatttgaagatctctattcctatgtgtctcagcttggggctggtgggactttccttctgtggggcggatgtgggtggcttcttcaaaaacccagagccagagctgcttgtgcgctggtaccagatgggtgcttaccagccattcttccgggcacatgcccacttggacactgggcgacgagagccatggctgttaccatctcagcacaatgatataatccgagatgccttgggccagcgatattctttgctgcccttctggtacaccctcttatatcaggcccatcgggaaggcattcctgtcatgaggcccctgtgggtgcagtaccctcaggatgtgactaccttcaatatagatgatcagtacttgcttggggatgcgttgctggttcaccctgtatcagactctggagcccatggtgtccaggtctatctgcctggccaaggggaggtgtggtatgacattcaaagctaccagaagcatcatggtccccagaccctgtacctgcctgtaactctaagcagtatccctgtgttccagcgtggagggacaatcgtgcctcgatggatgcgagtgcggcggtcttcagaatgtatgaaggatgaccccatcactctctttgttgcacttagccctcagggtacagctcaaggagagctctttctggatgatgggcacacgttcaactatcagactcgccaagagttcctgctgcgtcgattctcattctctggcaacacccttgtctccagctcagcagaccctgaaggacactttgagacaccaatctggattgagcgggtggtgataataggggctggaaagccagcagctgtggtactccagacaaaaggatctccagaaagccgcctgtccttccagcatgaccctgagacctctgtgttggtcctgcgcaagcctggcatcaatgtggcatctgattggagtattcacctgcgataa

SEQ ID NO: 86 - protein, 847 aa, Homo sapiens
MTRFRIDELEPRRPRYRVPDVLVADPPIARLSVSGRDENSVELTMAEGPYKIILTARPFRLDLLEDRSLLLSVNARGLLEFEHQRAPRVSQGSKDPAEGDGAQPEETPRDGDKPEETQGKAEKDEPGAWEETFKTHSDSKPYGPMSVGLDFSLPGMEHVYGIPEHADNLRLKVTEGGEPYRLYNLDVFQYELYNPMALYGSVPVLLAHNPHRDLGIFWLNAAETWVDISSNTAGKTLFGKMMDYLQGSGETPQTDVRWMSETGIIDVFLLLGPSISDVFRQYASLTGTQALPPLFSLGYHQSRWNYRDEADVLEVDQGFDDHNLPCDVIWLDIEHADGKRYFTWDPSRFPQPRTMLERLASKRRKLVAIVDPHIKVDSGYRVHEELRNLGLYVKTRDGSDYEGWCWPGSAGYPDFTNPTMRAWWANMFSYDNYEGSAPNLFVWNDMNEPSVFNGPEVTMLKDAQHYGGWEHRDVHNIYGLYVHMATADGLRQRSGGMERPFVLARAFFAGSQRFGAVWTGDNTAEWDHLKISIPMCLSLGLVGLSFCGADVGGFFKNPEPELLVRWYQMGAYQPFFRAHAHLDTGRREPWLLPSQHNDIIRDALGQRYSLLPFWYTLLYQAHREGIPVMRPLWVQYPQDVTTFNIDDQYLLGDALLVHPVSDSGAHGVQVYLPGQGEVWYDIQSYQKHHGPQTLYLPVTLSSIPVFQRGGTIVPRWMRVRRSSECMKDDPITLFVALSPQGTAQGELFLDDGHTFNYQTRQEFLLRRFSFSGNTLVSSSADPEGHFETPIWIERVVIIGAGKPAAVVLQTKGSPESRLSFQHDPETSVLVLRKPGINVASDWSIHLR

SEQ ID NO: 87 - DNA, 2835 bp, Homo sapiens
atggcggcggtagcggcagtggcggcgcgtaggaggcggtcttgggcgtctttggtactggcttttttaggggtctgcctggggattacccttgctgtggatagaagcaactttaagacctgtgaagagagttctttctgcaagcgacagagaagcatacggccaggcctctctccataccgagccttgctggactctctacagcttggtcctgattccctcacggtccatctgatccatgaggtcaccaaggtgttgctggtgctagagcttcaggggcttcaaaagaacatgactcggttcaggattgatgagctggagcctcggcgaccccgataccgtgtaccagatgttttggtggctgatccaccaatagcccggctttctgtctctggtcgtgatgagaacagtgtggagttaaccatggctgagggaccctacaagatcatcttgacagcacggccattccgccttgacctactagaggaccgaagtcttttgcttagtgtcaatgcccgaggactcttggagtttgagcatcagagggcccctagggtctcgcaaggatcaaaagacccagctgagggcgatggggcccagcctgaggaaacacccagggatggcgacaagccagaggagactcaggggaaggcagagaaagatgagccaggagcctgggaggagacattcaaaactcactctgacagcaagccgtatggccccatgtctgtgggtttggacttctctctgccaggcatggagcatgtctatgggatccctgagcatgcagacaacctgaggctgaaggtcactgagggtggggagccatatcgcctctacaatttggatgtgttccagtatgagctgtacaacccaatggccttgtatgggtctgtgcctgtgctcctggcacacaaccctcatcgcgacttgggcatcttctggctcaatgctgcagagacctgggttgatatatcttccaacactgccgggaagaccctgtttgggaagatgatggactacctgcagggctctggggagaccccacagacagatgttcgctggatgtcagagactggcatcattgacgtcttcctgctgctggggccctccatctctgatgttttccggcaatatgctagtctcacaggaacccaggcgttgcccccactcttctccctcggctaccaccagagccgttggaactaccgggacgaggctgatgtgctggaagtggatcagggctttgatgatcacaacctgccctgtgatgtcatctggctagacattgaacatgctgatggcaagcggtatttcacctgggaccccagtcgcttccctcagccccgcaccatgcttgagcgcttggcttctaagaggcggaagctggtggccatcgtagacccccacatcaaggtggactccggctaccgagttcacgaggagctgcggaacctggggctgtatgttaaaacccgggatggctctgactatgagggctggtgctggccaggctcagctggttaccctgacttcactaatcccacgatgagggcctggtgggctaacatgttcagctatgacaattatgagggctcagctcccaacctctttgtctggaatgacatgaacgaaccatctgtgttcaatggtcctgaggtcaccatgctcaaggatgcccagcattatgggggctgggagcaccgggatgtgcataacatctatggcctttatgtgcacatggcgactgctgatgggctgagacagcgctctgggggcatggaacgcccctttgtcctggccagggccttcttcgctggctcccagcgctttggagccgtgtggacaggggacaacactgccgagtgggaccatttgaagatctctattcctatgtgtctcagcttggggctggtgggactttccttctgtggggcggatgtgggtggcttcttcaaaaacccagagccagagctgcttgtgcgctggtaccagatgggtgcttaccagccattcttccgggcacatgcccacttggacactgggcgacgagagccatggctgttaccatctcagcacaatgatataatccgagatgccttgggccagcgatattctttgctgcccttctggtacaccctcttatatcaggcccatcgggaaggcattcctgtcatgaggcccctgtgggtgcagtaccctcaggatgtgactaccttcaatatagatgatcagtacttgcttggggatgcgttgctggttcaccctgtatcagactctggagcccatggtgtccaggtctatctgcctggccaaggggaggtgtggtatgacattcaaagctaccagaagcatcatggtccccagaccctgtacctgcctgtaactctaagcagtatccctgtgttccagcgtggagggacaatcgtgcctcgatggatgcgagtgcggcggtcttcagaatgtatgaaggatgaccccatcactctctttgttgcacttagccctcagggtacagctcaaggagagctctttctggatgatgggcacacgttcaactatcagactcgccaagagttcctgctgcgtcgattctcattctctggcaacacccttgtctccagctcagcagaccctgaaggacactttgagacaccaatctggattgagcgggtggtgataataggggctggaaagccagcagctgtggtactccagacaaaaggatctccagaaagccgcctgtccttccagcatgaccctgagacctctgtgttggtcctgcgcaagcctggcatcaatgtggcatctgattggagtattcacctgcgataa

SEQ ID NO: 88 - protein, 944 aa, Homo sapiens
MAAVAAVAARRRRSWASLVLAFLGVCLGITLAVDRSNFKTCEESSFCKRQRSIRPGLSPYRALLDSLQLGPDSLTVHLIHEVTKVLLVLELQGLQKNMTRFRIDELEPRRPRYRVPDVLVADPPIARLSVSGRDENSVELTMAEGPYKIILTARPFRLDLLEDRSLLLSVNARGLLEFEHQRAPRVSQGSKDPAEGDGAQPEETPRDGDKPEETQGKAEKDEPGAWEETFKTHSDSKPYGPMSVGLDFSLPGMEHVYGIPEHADNLRLKVTEGGEPYRLYNLDVFQYELYNPMALYGSVPVLLAHNPHRDLGIFWLNAAETWVDISSNTAGKTLFGKMMDYLQGSGETPQTDVRWMSETGIIDVFLLLGPSISDVFRQYASLTGTQALPPLFSLGYHQSRWNYRDEADVLEVDQGFDDHNLPCDVIWLDIEHADGKRYFTWDPSRFPQPRTMLERLASKRRKLVAIVDPHIKVDSGYRVHEELRNLGLYVKTRDGSDYEGWCWPGSAGYPDFTNPTMRAWWANMFSYDNYEGSAPNLFVWNDMNEPSVFNGPEVTMLKDAQHYGGWEHRDVHNIYGLYVHMATADGLRQRSGGMERPFVLARAFFAGSQRFGAVWTGDNTAEWDHLKISIPMCLSLGLVGLSFCGADVGGFFKNPEPELLVRWYQMGAYQPFFRAHAHLDTGRREPWLLPSQHNDIIRDALGQRYSLLPFWYTLLYQAHREGIPVMRPLWVQYPQDVTTFNIDDQYLLGDALLVHPVSDSGAHGVQVYLPGQGEVWYDIQSYQKHHGPQTLYLPVTLSSIPVFQRGGTIVPRWMRVRRSSECMKDDPITLFVALSPQGTAQGELFLDDGHTFNYQTRQEFLLRRFSFSGNTLVSSSADPEGHFETPIWIERVVIIGAGKPAAVVLQTKGSPESRLSFQHDPETSVLVLRKPGINVASDWSIHLR

SEQ ID NO: 89 - DNA, 2559 bp, Homo sapiens
atggcggcggtagcggcagtggcggcgcgtaggaggcggctttctgtctctggtcgtgatgagaacagtgtggagttaaccatggctgagggaccctacaagatcatcttgacagcacggccattccgccttgacctactagaggaccgaagtcttttgcttagtgtcaatgcccgaggactcttggagtttgagcatcagagggcccctagggtctctttctcggataaggttaatctcacgcttggtagcatatgggataagatcaagaaccttttctctaggcaaggatcaaaagacccagctgagggcgatggggcccagcctgaggaaacacccagggatggcgacaagccagaggagactcaggggaaggcagagaaagatgagccaggagcctgggaggagacattcaaaactcactctgacagcaagccgtatggccccatgtctgtgggtttggacttctctctgccaggcatggagcatgtctatgggatccctgagcatgcagacaacctgaggctgaaggtcactgagggtggggagccatatcgcctctacaatttggatgtgttccagtatgagctgtacaacccaatggccttgtatgggtctgtgcctgtgctcctggcacacaaccctcatcgcgacttgggcatcttctggctcaatgctgcagagacctgggttgatatatcttccaacactgccgggaagaccctgtttgggaagatgatggactacctgcagggctctggggagaccccacagacagatgttcgctggatgtcagagactggcatcattgacgtcttcctgctgctggggccctccatctctgatgttttccggcaatatgctagtctcacaggaacccaggcgttgcccccactcttctccctcggctaccaccagagccgttggaactaccgggacgaggctgatgtgctggaagtggatcagggctttgatgatcacaacctgccctgtgatgtcatctggctagacattgaacatgctgatggcaagcggtatttcacctgggaccccagtcgcttccctcagccccgcaccatgcttgagcgcttggcttctaagaggcggaagctggtggccatcgtagacccccacatcaaggtggactccggctaccgagttcacgaggagctgcggaacctggggctgtatgttaaaacccgggatggctctgactatgagggctggtgctggccaggctcagctggttaccctgacttcactaatcccacgatgagggcctggtgggctaacatgttcagctatgacaattatgagggctcagctcccaacctctttgtctggaatgacatgaacgaaccatctgtgttcaatggtcctgaggtcaccatgctcaaggatgcccagcattatgggggctgggagcaccgggatgtgcataacatctatggcctttatgtgcacatggcgactgctgatgggctgagacagcgctctgggggcatggaacgcccctttgtcctggccagggccttcttcgctggctcccagcgctttggagccgtgtggacaggggacaacactgccgagtgggaccatttgaagatctctattcctatgtgtctcagcttggggctggtgggactttccttctgtggggcggatgtgggtggcttcttcaaaaacccagagccagagctgcttgtgcgctggtaccagatgggtgcttaccagccattcttccgggcacatgcccacttggacactgggcgacgagagccatggctgttaccatctcagcacaatgatataatccgagatgccttgggccagcgatattctttgctgcccttctggtacaccctcttatatcaggcccatcgggaaggcattcctgtcatgaggcccctgtgggtgcagtaccctcaggatgtgactaccttcaatatagatgatcagtacttgcttggggatgcgttgctggttcaccctgtatcagactctggagcccatggtgtccaggtctatctgcctggccaaggggaggtgtggtatgacattcaaagctaccagaagcatcatggtccccagaccctgtacctgcctgtaactctaagcagtatccctgtgttccagcgtggagggacaatcgtgcctcgatggatgcgagtgcggcggtcttcagaatgtatgaaggatgaccccatcactctctttgttgcacttagccctcagggtacagctcaaggagagctctttctggatgatgggcacacgttcaactatcagactcgccaagagttcctgctgcgtcgattctcattctctggcaacacccttgtctccagctcagcagaccctgaaggacactttgagacaccaatctggattgagcgggtggtgataataggggctggaaagccagcagctgtggtactccagacaaaaggatctccagaaagccgcctgtccttccagcatgaccctgagacctctgtgttggtcctgcgcaagcctggcatcaatgtggcatctgattggagtattcacctgcgataa

SEQ ID NO: 90 - protein, 852 aa, Homo sapiens
MAAVAAVAARRRRLSVSGRDENSVELTMAEGPYKIILTARPFRLDLLEDRSLLLSVNARGLLEFEHQRAPRVSFSDKVNLTLGSIWDKIKNLFSRQGSKDPAEGDGAQPEETPRDGDKPEETQGKAEKDEPGAWEETFKTHSDSKPYGPMSVGLDFSLPGMEHVYGIPEHADNLRLKVTEGGEPYRLYNLDVFQYELYNPMALYGSVPVLLAHNPHRDLGIFWLNAAETWVDISSNTAGKTLFGKMMDYLQGSGETPQTDVRWMSETGIIDVFLLLGPSISDVFRQYASLTGTQALPPLFSLGYHQSRWNYRDEADVLEVDQGFDDHNLPCDVIWLDIEHADGKRYFTWDPSRFPQPRTMLERLASKRRKLVAIVDPHIKVDSGYRVHEELRNLGLYVKTRDGSDYEGWCWPGSAGYPDFTNPTMRAWWANMFSYDNYEGSAPNLFVWNDMNEPSVFNGPEVTMLKDAQHYGGWEHRDVHNIYGLYVHMATADGLRQRSGGMERPFVLARAFFAGSQRFGAVWTGDNTAEWDHLKISIPMCLSLGLVGLSFCGADVGGFFKNPEPELLVRWYQMGAYQPFFRAHAHLDTGRREPWLLPSQHNDIIRDALGQRYSLLPFWYTLLYQAHREGIPVMRPLWVQYPQDVTTFNIDDQYLLGDALLVHPVSDSGAHGVQVYLPGQGEVWYDIQSYQKHHGPQTLYLPVTLSSIPVFQRGGTIVPRWMRVRRSSECMKDDPITLFVALSPQGTAQGELFLDDGHTFNYQTRQEFLLRRFSFSGNTLVSSSADPEGHFETPIWIERVVIIGAGKPAAVVLQTKGSPESRLSFQHDPETSVLVLRKPGINVASDWSIHLR

SEQ ID NO: 91 - DNA, 357 bp, Homo sapiens
atggcggcggtagcggcagtggcggcgcgtaggaggcggctttctgtctctggtcgtgatgagaacagtgtggagttaaccatggctgagggaccctacaagatcatcttgacagcacggccattccgccttgacctactagaggaccgaagtcttttgcttagtgtcaatgcccgaggactcttggagtttgagcatcagagggcccctagggtctctttctcggataaggttaatctcacgcttggtagcatatgggataagatcaagaaccttttctctaggcaaggatcaaaagacccagctgagggcgatggggcccagcctgaggaaacacccagggatggcgacaaggca

SEQ ID NO: 92 - protein, 119 aa, Homo sapiens
MAAVAAVAARRRRLSVSGRDENSVELTMAEGPYKIILTARPFRLDLLEDRSLLLSVNARGLLEFEHQRAPRVSFSDKVNLTLGSIWDKIKNLFSRQGSKDPAEGDGAQPEETPRDGDKA

SEQ ID NO: 93 - DNA, 159 bp, Homo sapiens
atggcggcggtagcggcagtggcggcgcgtaggaggcggtcttgggcgtctttggtactggcttttttaggggtctgcctggggattacccttgctgtggatagaagcaactttaagacctgtgaagagagttctttctgcaagtgttgctggtgctag

SEQ ID NO: 94 - protein, 52 aa, Homo sapiens
MAAVAAVAARRRRSWASLVLAFLGVCLGITLAVDRSNFKTCEESSFCKCCWC

SEQ ID NO: 95 - DNA, 159 bp, Homo sapiens; identical to SEQ ID NO: 93

SEQ ID NO: 96 - protein, 52 aa, Homo sapiens; identical to SEQ ID NO: 94

SEQ ID NO: 97 - DNA, 231 bp, Homo sapiens
atggcggcggtagcggcagtggcggcgcgtaggaggcggtcttgggcgtctttggtactggcttttttaggggtctgcctggggattacccttgctgtggatagaagcaactttaagacctgtgaagagagttctttctgcgacagagaagcatacggccaggcctctctccataccgagccttgctggactctctacagcttggtcctgattccctcacggtccatctga

SEQ ID NO: 98 - protein, 76 aa, Homo sapiens
MAAVAAVAARRRRSWASLVLAFLGVCLGITLAVDRSNFKTCEESSFCDREAYGQASLHTEPCWTLYSLVLIPSRSI

SEQ ID NO: 99 - DNA, 159 bp, Homo sapiens; identical to SEQ ID NO: 93

SEQ ID NO: 100 - protein, 52 aa, Homo sapiens; identical to SEQ ID NO: 94

SEQ ID NO: 101 - DNA, 37185 bp, Homo sapiens
ggtcaaggagatggacggcacaaaggcctgggggtgggaaaactggagtacaggggtccagtgtggagagagttgggggcagagtcttaagcggggagctaaggcactaaggccgtctcctgttctttgggaactggggagccacaccttgattcccagcacaagagggaggaaaggaagacctgagatctagagaggacagcaggagcctgccctgggctccaagagtttcagagatggcccagatcagttgattgagtggccttctccctgtcatgagccacaagcagtagaagccacaggggggcagaagagatggagagatggagagagacacagcgacagtcaccagaagagagacaggggcatggcagaaagaggtgggagaaatccaggaaggctccctgggggtggtggccggaaatagggtggaggcctaatccctgatactagagaggcaggacctagaggggaggagaaagcttgatgctaggcaggaagtccaaaagtctgtctaggaatccaggacggcttcctgaaggaggggccattggatctgggccttgaaagataaatagacgtttcctacatttcctaggcagagaaaagtgtgtgtgtgggcggtgggggaggggggaaacggggaattgctcattttacttaacaagtactttcccatttttaggggaccaggtactcagtgggccacagacaagaccaaggcagaaaagacaggcgcctccccacattgcagcaccgggaccccgagcccacccacagccctcttcattcctcccaacgatggatggggaaactgaggcagcccagagcagcccccaccctaggtcctgcccgggacacgcccacgcgggacctgtgtcaccaggttaaaaatggaaacagctaggaccttttttttttcttcctttaagaaaatcctaggtccaaataaggcgagggctgccgggagcacggtgagctggccaagtcctcctgagcaagcgagtggcggctggcccggccggcctgggcttgggcctcctccaagactcgcctggcaggagggcggaggcaccccgggaggctataaggccctctcctccaccctgccaggctcactctgccccacagccacagcccctgactgccgcagcccccacagagcccgccgcgcaccccacgtcccccacgccagcgcccagccatggaggccatcaagaagaaaatgcagatgctgaagttggacaaggagaatgccatcgaccgcgcggagcaggcggaggcggataagaaagccgctgaggacaagtgcaagcaggtgaggtgccctccgctgggccgctccgggctgctgggagtcctctctgtgcggaaggccggggtctggagcccagttgggggtcgcagacacctgcgggaggataggaggctgatgctttggcggaggaagagcgaggggaccattgccttccttggatggggtcctgggctggaagaggggtgacgatcggacccacccccagcagggccagtgcgaacaaagtgagtttgacagagagagagttggcgggggagggagagtgagaacgttcgtgagcgaggtgtcgtttgcgctgggaggttgtgtactagatagggcggttggggacatgctgtgtgtgtgtatttgcgtgtgtttgagcgtatgtgtgtgtacgtgtgtgtgtacgtgtgtgcgtgtttgcctctggtgtgtgtgtgcatgtgtgcgtgtgtgtgtgtgtgtgtgtgtgtttgagacagagtctcgctctgtggcccaggctggagtgcagtggcccaatctcggatcactgcaacctccgcctcctgcgttcaggcgattctcctgcctcagcctccgagtagctgggattacaggcacccaccatcacacccggctaattttgtatttttagtagagaccggatttcgccatgttggccggactggtctcaaactcctgacctcaagtgatccgcccgcgtctgcctcccaaagtgctgggattacaggcatgagccactgcgcccggccatttgtgtgtgtttgagcaattctctgtgtgtgtgcgtgagcatttctgtgtgtgtctgtgtgtgtatctgcatgtttgagcatttgtgtctgtgtgtacatgtattgtgtatgtttgagcgtgtgtctgtgtgtatctatgtgtttaagcatttctgcacatgtctgtgtgtgtacacatatttgtgtgtttgagcaattctctgtgcgtgtatctgtatgtgtttaagcatttctgcgtgtgtgtgtacacatatttgtgtgtgtgagagcagttctgtgtgtgtgtgagtgtatctgtgtgtgtttgagcctttctgtgtgtgcacatgtgttgtatgtgtctgttttacgtgtctatctgtacatgcacatatgtttcagctgaaaagagtgcggaggggtaaaggtgactgtgagaatgagtgtgtactaggagagctgtgtgtgggacgctgcgtgcggctgttggaaagtaggtgtgaaagagtgtgggtgtgtttgtgagcctgtgtgtagatggtgggggtctgtgagggtagcgggacaggctgactgtgtgtgtgcttgagcaaacgctggtatgacagtgattgaaagtacatgttgatgtggctatgtttgtgttggcatctgtgtatcagggtgatgggtttctgatggcgtgtgtgtgtgcacccacgcacatgtttggatgtgtgtttctgttgtgtgtattggtgactgtgcttctgttggggtgtgtgtgcatgtttagatgagtgtgtgtttctgttggtgtgtttatgtgtatgagtgtgtttctgttggtgtgtgtgaatgtgtatggatgagtgtgtgtttctgatggggtgtgtgtatggttgtgtgtttctattggtgtgtatgtgtgtggatgagtgtgtgtttctattggtgtgtgtgtatgagtgtgtgtttctgttggtgtgtatgtgtgtgaatgagtgtgtgtttctattggtgtgtgaatgtgtatggatgagtgtgtgtttctgatggggtgtgtgtatgattgtgtgtttctattggtgtgtatgtgtgttgtgtgtggatgagtgtgtgtttctattggtgtgtgtgtttctattggtgtgtgtggatgaatgtgtgtttctgttgctgtgtgtgtgtgggtgagtgtgtgtttctgttggtgtgtgtgtggatgagtgtgtgtttctgttggggtgtgtgtgtggataagtgtgtgtttttatggggttgcgtgtatgagtgtgtttctattggggggtgtgtgcatgtgtggatgagtgtgtgtttcgattggtgtgtgtgtgaatgagtgtgtgtttctgtcggggtgagtgtgtgtgtcagtgactgtttctgctggcgtgtgcatatggatgtgaggggggctgtgcgaacctgtgtgtgcgtgtaggtgacactatgcccctggatcaggaagcctccactgtgacagaagcccgctgtctcatgggcacctgcccaggagaatggcacggcatgtgtgtgtgtgtgtgtggtgggggcccagggctgtgacctgctgcaggggtgactgggtggggtctggggactgggatgggagtagagttgagagtgagtctgagaatctcattgtgtatgtgggggtgtccctgctaaaagcctggaggccggggcaggtgggctgcccgtggtggacggaggagagggaggccatttcccatctcctggcagccaagagcccacacagacccagaactttggagacaagagtcctgggaaccctggcaatgagaatgcattggagttccaaggccgtggccatggtttggggcagagcagacaggagcagtgggtgggaggaaggaagggagtcccctcccacagagccatgttccccacaatgtttatccacaccccgatgtcaactgccaagccctggggagcatccaggtctccgataaaccctgggagatgcctaggaccatggcaccgagtgcccagccccacccaggccaggagccaggccagcccggcagctaaaggcgaaagctcggagctcagactggccatgtttgagtcatggctcagtcgctaggtgtcccggacgcctgcatgagtgagatacggaagtgacagtagggcctcccttgccaccccatgacaggattagaggtgactgtacaggtggaacccttggcccggagcctagctcagagtaagcactcaataaatgtaggttgatttcctgccccgccctacttcccctttgggcctccccagccccccgtgccccagggctgccctaagagtatgtggcacattcgtgcaggccaagccccaccccagtgttccctgccacaagctctctccgccttctctgtgcccctccctggcaaacacagacattcatcctgtgctgggccagcttctagccatcatttagccctcaccatgagggacttagccagagattcggagagaaacaagtttatagcactaattcttactaaggtgtgagtggctatctcccaggacagccacaagttcaaaaaggaagaatcctcaaagcctccagccagctgcgtggccaaggaggttatgccttttttgtcccacaaagatgcccactggagtagacttgggctcaaagcaagtctacacagactagctttcaggcaaacctccatagactagcacatactttgtgtatatcagtctttaaatgtatttttattttttagagatgggggtctcactctgttgcccaggctggagtgcagtggtgcaatcacagcttactgcagcctcaaactcctagggctcaagcgatcctcccacctcagcctccccagtggaggtgcacacctccacgcccagctagttattttatttttagtagagacagggtctcactattgcccaggctagtcttgaactcctgggctcaagtgatccttccacctcaacctcccaaagtgctgggatcacagacttgagccacggagcctggtctttgtgactctcctagcttcatgactgaggacacgttcctgcacatttctgagccctcagtgtcctcatctgtgaaatgggaacacgtgaggccttctgaagttcaggtgtggaactcaagatcccagaattccgaagcagaagccagcgccccacaggagctaacggccagtcctgctggggaatagaggcacttagagcgcctgacgctgcaggaggccagagagagcagctctcgggccagcctgatcccagcagccaagcactgatttctggccctgcttacccagtgtgggaaaaggacaaagaggcccagcccggccgcttcctgcccactcccctcccagggcagcaacatcctccaccactggcctttgaccccacatcctgcctcagccctgccccaaggccccatttgcagggactaaggtaatcctatgacagatagggaaactgaggctcacagagggacaatgacgggcacgcgccaccaggcccggctaatttttgtatttttagtaaagacggggtttcaccatgttggtctggctggtctcaaactcctgacctcgtgatccgcccgcctcggcctcccgtagtgctggaattacaggcgtgagccactgcgcccagctctcatttattttttatcctcactgcctaccactgaagggtttggggttgtgtcttcgattcatcccaaacacttcctacagtgttctaatgctggggcccatagtggcctcagtcccagaactgaccctcaagaaactccaagctgagggagacagaccatgaatacctccagctcagaggtcagggccggaccagagggagggacagaggctgggacagctgtaggcgtggcgaaagctctgctcagggcagcagagcaggccaccagggttggggagccttgggactgagcatggagggacggtagatgccctcccagtgaaaagtagaaagtcattcttagcagtgggtccagcatggtctagaagtcaagcaaaccagctttggaatcagactaacaaagattcaaatcccccatctgtgtggcatcaggcaagtcccttcccctttcagagactcagtttgcccttctgtagtatggggcttccctgagacaatatttgtaacacgccctggccaggcatagtggctcacacctgtaatcccagcacttcaggaggctgaggtgggggatcacctgaggtcaggagttcgagaccagcctggcaaaaccctgtctctacaaaaaatacaaaaattaactgggcttggtggcatgagcctgtaatcccagctactagggaggttgaggcaggagaagcacttgagccagggaggtggaagttgcagtgagctgagatccagccactacactccagcctaggcaacagagcaagactctgtctcaaaaaatatatcaaaacaaattgtaacacgcccaacacattctaaatgccagatagccccctgtcggccttatccctgtcctcacatgttcttgcccaaacatttcccccaaaaaagtagtcaaaaccccaaaccaaacaaaaaaaccccaaaccagccaggtggggtggctcatgcctgttgtcccagctactcgggaggctgaagtgggaggatcccttgagcccaggagttcgagaccagcctggataacacagcgagatcctatctcaaaaaaacaaaaacaaaaacaaaacaaaacacccaaaccatcttcataccctgatgagtccatgctgtcagatttgctctcactcttcctacatgttaggagagtcctgtgttgggcacacagttggcacccaataaatgctgtgatccacagatctggaaggaagtcaggtggatgctgtaggtcagggttgacctatgaaacgtctttaaggaaactggctcattttctcagtcaaggcagaagttcaaaagcagctgccggaatgctcagagaccagcatgtcaaggtttctgttctgcagatggagaatctgaggccagaaaaggggacgggggtcgcagagcttggatttggagtcaggcttccaggctccccacccggaggtcaaggtcaggccctatagactctgaccctgccctgatcagctggccaccctggattgggccctgtcatctccccatagcttgggatgctcctgaggacttcagacaggatagccctccctgctctctgtcacatctcagctagagacccttgcaggtcacctcagtgacatcagctgaacctccagctgccagcctccaccccatcctccagctgacacccagcaggccgcaagatgggaagcctggagttcacactttccagctactcaggaggctgaggcgggaggatcgcttgagccgaggaggtcaaggctgcagtaagctatgatcacaccactgcactccagcctgggagacacaggaagaccatgtaaaaaaaaaaaaaaaaaaaaaacgcaaaaaaaaaaaataatgcacacacacacacagcaagatcaggttaaaaaaaaaaaaggcaaaaaaaaaacatacacacacacacacatatggggcacctggtacattttgcacatccactcaggggtgagcacgtagcccagacaggattcagagctcagtctagaagccacgggcacagcagcttttttaacataccctcttcaagaaaaaaaagaagagaagcaagtcagagagggaggaagggaagctggcctagtgtgaggaacagggccaagggctttgtctttgtcagctcaggcagttataacaaaacaccatagactgggtagcttcagtaatagacatttattgtttacagtctggaggctagatgtccaagatcaagatgctggcagattaaatgtctggtgagcgctctctagctagcttgcagacagccaccttcttgctgtgtcctcacattggaagaggataaccaagttctggcctcttctcataagggccttaatcccatcatggtgggtcaaccctcatgacctcacccaaacctcatcatcttccaaaggccccatcaccaattaccatcacatggagatgagggcttcaacacatgaattggagagggggcaaaagcaagcattcagttcattataggcttatattccagaagacctgggctcaaaccctgtgctgtgtgacctggggaaagtcatcccacctctctgagcctcctgctgtggggaggaagcaggagaatgaagctgggctcagtgggggctgtctgcccaccctgggagcaggaacaagatcagtgtcaaaccatctaaggcaaaagtcagatccaagccaggtgtggcgactcacgcctgcaatcccagcaatttgggaggccgaggcgggcagatcacttgaggtcaggagtttgagacctgcctggccaatattgcaaaaccctgtctctactgaaaatacaaaaattagtcagtcgtggtggtgtgcacctgtagtaccagctaccggggaggttgaggcaggagaatcacttgaacccaggaggcggaggttgcagtgagctgagatcgtgccactgcactccagccttggtgacagagcgagactctcaaaaaaaaaagtcagatccaggcatgagctggatatgatcaccctaatccagagttgggggcccagggagggagtttcagcctggaggtgacagaaaagtcttcttgagccaactctagaccggtgtggtggggggtgacaaagagaggtgatggggtctgtggtttgtaatccataggcctgagcttctcaaactaggagtgatgggaggataggactcttgggataaacagaggactgaaaatttagggaaagtaggggacatttttattaaaatgaacatggcctatatgcaaaaattttaaagatttaacccgagccttcaaagaaagtgatcctgtaggggcgagtctcttctagccaagctccccaaagcccagaaatgagggactaggtctgagcccttcagcccttcagagtattttggtaagacagtctaagaaccactgccttgggccatagggagccatagcaggttctaggcagaaagagggcaggcgtatttgttagaaagtttctctgaccccgtgttggggtcagaaccagagggagaaaggctggggacagggatgggcggagggatccacgcgcagagaatgagattgcttaactccagatcatggtgaggctgcacctctgaaactggaatgtgtgtatttctggaaaacatttggagtcttcagtttcccaaaagctgccattgatctccctagagtactggggaccccaataagcccaaaacagctggtcctcaggacgagggaaagatgtgaaaatcccactatcaggtagcatggatggcgtggtgcatgctatcgcaacccctgttctacagataaggaaactgatgcccagagagagacggaggactcttgtgaatattgggggggaccgcccctgcacctcggggacgtgaccccccccccaggctgacccgttcctcgctctgtcgtccccaggtggaggaggagctgacgcacctccagaagaaactaaaagggacagaggacgagctggataaatattccgaggacctgaaggacgcgcaggagaagctggagctcacggagaagaaggcctccgacgtacgtgtgcagggatgcgggagcccgcggcggggccaggccggagccccggggccgggaaggcggggagagccgcagggggaggaggaagaggaggaggagaaggcggcgcctcccagcgctttctccaaataagtcccgaaaaggggcactttccagcagctgtggccagcggtgccgacgtcaggccctcccccagcggtgctgacgtcggcggtccggccgggtgacctcatcgccccgacggcagccggcccggggggcggggagaggcgggggcggcccccgcgcaggcaaaggcttggggggccggggcgcggctgtgcagctctcgccggagccgagcccagccgagcgtccgccgctgcccgtgcgcctctgcgcctccgcgccatggccggcctcaactccctggaggcggtgaaacgcaagatccaggccctgcagcagcaggcggacgaggcggaagaccgcgcgcagggcctgcagcgggagctggacggcgagcgcgagcggcgcgagaaagtgagcgccccggcctcgggccccgcacccgcagcctcctcccccgcgcgccctcctttcttcccggcttcccgcgctgcccgcccgcgcgcagtcctcgggccgcctttttacgccctcggacgccgatcgccgacccacatccctgcgcccgcagccaggaccccctacttcctccgccgtcctccttcctgggcctgggacaggggagggggcgccgcctccgggtcgggcggggccggccaagcgggaaatggggggatggggcggagggggtgagcgatctccgggtggagaagtggagcggcgggagggggcgtatcgtgcaggctccgactccggggctggcgccggggtcccgggccgaggggaacccgcgaccggacttgtgggggagaatgaggatgaaaacgtggagcttccattgtctagggtttgaccggccgacagggatttcgacgggggaccggggatctggggagggggtcgcactttctcgcctctttcgcggcttcccggcttctgcttgcttccctgaccgttcccaggggcgcggcggcgacgtgtctgctccaggcggcgggggggatggggggtggaggaagttcagccccaagccgcccgcctttctccagctgattcctgcgggaaccggggcggcgggaccctgcctctctccagaaggccccgggaacgctggcgcggggccctgaacccacgatcgtttgagcgcctgctgtgcgcctccgccgcgagtcgcagggcccgagataaacaatgggtctgaaaaaggagggagtttcaccatcctctctgcatcatcctcctggctgtccctcgggacagatggtggcaccgccagggtctggggacagatttggattctggtcccatatcatgccacccacaggcttcatgacttggtatttgctctctaggagcttttttcccatctgcgagtaggactgataagaatcccgaccccccagagtagcagggagggtcccaggagtaaatctcaggcgtggagcctggcgctttgtaaataatcaattgtgttgttgttttttgttgttttgtttttgaggcagtctcactctgtcgcccaggctggagtgcagtggtgcgatctcggctcgctgcaacctccaccccccgagttcaagagattctcctgcttcagcctcccgagtagctgggattacaggtgcccgccaccacgcccagctaatttttttttttttattttggatttttagtagagacagtgtctcaccatgctggccaggctggtctcgaactcctgacctcgtgatctgcccaccttggcctcccaaagttctgggattacaagcgtgagccacggcgcccagcctcaattgtgttttctctgccctgggaagagctcatagacaaatggaggcaggggagctgactcactgatggagcgaggtctgcattccacgggttttctgtgcagttatgggagcatgacaggggaggctccaaaatggaggttgagctgggtcttatagaataaataagtttgctgggaccagagacatgggtgtgcacagactcagaggcaagaaagttgtatgatgagggtgggggggtgtgcggatagaggttgaagcccaaaagccctgaaagttcagtgttgaggctcagggtggggaccctagagaggcaaaagatgcccagccagatggaattggtggtgtgaattgccaggactggaaagagcccagatgggggctgcagcatgggccttggttgaagcctctaatcctgtaagggctgctttggcccaagaggccttagaaacccggtgtaagcctcaatcggtagccggtctggcctctttctcacacttaaccgacacagctcttgctctgatctcatcccaagtcatctcgctggaggacaattaactcggcttcaaaatggccctcagcctggagccaagatttaggagcaagaccgtctagttgggagagaagatgtttttggagagttgaagacttcttgaaaaagttcgaaaagttcttgaaaaagcaaaggatgcttctttccgtctgggagagggaaaacctctcccagggcaaaaggaactaagaccaggggtgggttaaaaaaaaaaaaaaaaaaacctttcactcttgtagaataagccaggagccggcgtgtggtagacttctgggcctgtttcccgacagctggtttcgtttagatttttgtgtgattaactgacatcttcctgttcctttgccacatgtatctagcaagcctcttttaccttataagggaaatcctttgtagcgtgtggaaggctttgattgcaggaaggggtggaacccaaaatgactcggccgtgactagcagtttttcaaaaatacatatatatgtatgcatgtacagatatgcgtgtatctcccaactccagacagctgaaaatctgccaaaagcgttgtttgccaggattcagaatttcccacataagggctactcacttcttaaaagacaactcatgaatcaagcacctctgtttgatctttaaaatcaattcctcgactgctaatgggtacacagttttttgtttgtttgtttgtctttggcgggttatgaaaatgtcctggaattcgataatggtgttggttgcagagtgtttttgcaacatcagttcctggcccagttactgaaggtggtaggaggagttaagatctaggcaattaaaaagaatgaaaggcacccattcatgggaaggcctcagtgacgtttcttaagacagtttcatcagtggttttcacaattctctgcatttggtgtttcagaggacactgcaatacgaaacacctgtgggagtgccctctttctgcttctaggaatctgaggctgagaaaccttcctgactctatttgtgtagtttttcggccacgttagcctcattctatttttttttcccccagtatgaactcagggcaggagagggagtggtttcctaataattttttttttttgagacggaatcttgctctgttacccaggctggagtgcagtggcgcgatctcggctcattgcaaccttcacctcccgggttcaagcgattctcctgcctcagcctcccaagtagctgggattacaggcgcctgcccccacacccaactgatttttttgtatttttagtagagatgcggtttcaccatgttggccaggctggtctcgaactcctgacctcatgtgatccacccacctccgcctcccaaagtgttaggattacggatgtgagccaccgcgcccggccttcctaataattttgatagccttccccagttcagggattcttcatttgttctgataggaaaaagctagcgtggcttcccttttcctctcggttgaggcccgtttgacccgttctcaatattccttccaaagagcaggcatcgctggaaaactcgccttgcctcgtagccctggcaggacctaggggacaggttctgacaaggaagagccctgggtgggtcttaagaggccattcatttcttaccaattctgagtcactgaataaaaccacttcccccagtggggcccctcggtttcttcacctgtaaaatgggtgcgatgtgtgaggatgaaattgcagtaaaataaaaccgtggcagtaagagatgcctttctctggcacatcccacctgctgggcataagcggcgccaccctctggagttacagcctcaaggcagtccggtaactaatcaggctttgggatggagagggccaggatgaggaagcaaccttcccaacaccacgtggctgtgaaaatgacaaagcacggtcgggcgcagtggctcacgcctgtaatcccagtactttgggagaccaaggcgggtggatcacgtgaggccaggagtttgagaccagcctgaccaacaagacgaaaccctgtctctactaaaaatacaaaaaaatagcaaggcgtggtggtgtccgtctgtaatcccagctactcaggaggctgaggcagaattgcttgaacccgggaggtagaagttgcagcaagccgagatcatgccattgcactccagccttggtgacggcgcaagactccatctcaaaaaaaaaattaaaaagaaaatgacaaagcggggattccagcccagcactttttggccctggagttcctggtttaatgcttcccattgtacttcctttcttgtaggtaaaaacaccttgaaaagccaataacactattggggtatgtcttccatgcctgcaaccaagttttctttccctttccatatctttttgtcctgccatctctcagccaggcggattgaaggatggaattccaacgaggctcccccgcctcgtcccaccttggtaattgcatggccaacatttaactgagggctccatagtcttgcatttatcttgccattcaggtgaatgggagcggaactcacaggacacaatgagccgggtcactgatggccttgctttctaagaatctcacagtgagccctagaactctctacgtggtaacactgtgtgcctttttcagagaagagcctatcttagatcttagcctaacgttgggtctattgtgttgctggagagaccagcactgacattcatctcaaagcacatggtatgtttgactcctatgttgactcaactacccatcttgtactgggacactcgctttttttttttttttttgagacggagtcttgctctgtcaccaggctggagtgcagtggcacgatctcagctcacggcaacctccgcctcccgggttcaagtgattcttctgcctcagcctcctgagcatgtggaactacaggcacgtgccaccacactcagctaatttttctatttttagtagagacagggtttcaccacgttggccaggatggtctcgatctcttgaccttgtgatacacccacctcagcctcccaaagtgctgggattacaggcatgagccaccacgcttggcgatgctcatcttttgctatggagtggtagatgtttttcccagacattttccgggaagatcatactgaaattttggtatgagtgtaaattccctatggcctggactcctgggtgggctttgacggggaagatcaggttaacagagggcaggacatgggggaggctcccactggtggctggcctgatacttcttaacatggctgcacctccgacctccccaggctgaaggtgatgtggccgccctcaaccgacgcatccagctcgttgaggaggagttggacagggctcaggaacgactggccacggccctgcagaagctggaggaggcagaaaaagctgcagatgagagtgagaggtaaggacgctttgaatctggtggcatccgtgtttgcttttagaaaatggggatcatgctgccgacctcgcagagctggtgtgaaagtaaacaaggtcacaaggacatgcatgtgtccacaaaaaagtgcatgacagcactttgtaaaccatcactccatgggtagagatgtttatccgtggccaggcacggtggctcatgcctgtaatcccagcactttgggaggccaaggcggacggatcacctgaggttgggagtttgagaccagcctggccaacatggtgaaaccccgtctttcctaaaagtacaaaaaaattagcctgccatggtggcgggcacctgtaatcccagctactcaggaggctgaggcaagagaatctcttgaacccaggaggcagaggctgcagtgagccgagatcgtgccattgcactccagcctgggcaacaagagcaaaactccatctcaaaataaagtgaggggtgtttatccttacggtaaccatgaaaagaaacttccgacagacagaaaggcaaacagaacgggcagatgtgagactgcaagtatgactgtccatggtggtcagtttgcaaagcactgcttctcgtattttctctgaaagccacagtgcctcttagtgttctctagacaccaaatttcaggtaggccggatgcagtgattcctgcctgtgctcccagcactttgggaggcagaggcgggcaaatcgcctgagctcaggagttcaagaccaactggggcaatgtggtgagaccctgtctctacaaaaaatacaaaaattagccgggtgtggtggtgcacgcctgtactcctggctactcaagaggctgaggtgggaggatcacttgaccccaagagtttgaagctgcagtgaggcaagattgtgccactgcactccagcctcagtgacagatgagattctgtctcaaaaaaaaaaaaaaaaaaaaaaaagcagagtactgtggagaggaggaaaggaaacttgggatgcacaggtgattgttagcagagctgtcaggctttaggcttttggacggtgacagctatttcagggacagttgcaaaccagcatggttaatgtacttgcaactgaccatgcaccaggtgccgtggctcacgcctataatcccagcactttgcgatgacgaggcgggtggatcaactgaggtcaggtgtttgagaccagactggccaacatggtgaaaccccgtctctattaaaaatacacaaattagctgggcgtggtggcgggcacctgtaatcccacctactcaggaggctaaggcaagatcccccagcttgaacccaggaggcagagggtgcagtgagccaagatcgcaccactgcactccagcctgggcaacagagtgagactctgtctcaaaaagaaactgaccacgttcctcacccgcccatggtatctgtgctgcaacccagccaccagtagggtgccttctcctcggtagccagatcattctctggcacgccttggcacaggctctctggaagactgagggtagattgtgtaattcacagaagcagcagtctgtgtgtggtggaaaaggagttccttgtgtggcaatggtgtgggcccgaccagtgatcatcgcgtctgcccctcattcacaccggagttctcacttgagccagccaccatgcttttgcagtataaacacctcccaaagattcatttctttttttttttttttttttgagacagggtcttactctatcacccaggctggaatgtagtggtgcgatcacagctcactgcagcctcgacctcctgggctcaagcgatcctcccgccacggcctccagagttccagagtaaagctgggactacaggcgcatgccatcatgcccagctaatttttttttgagacagagtctcgctctgtcgcccaggctggagtgcactggcgtgatctcagctcactacaagcttcacctcctgggttcacgacattctcctgcctcagcctcccaagtagctgggactacaggcacccgccaccacacccggctaatttttttgtatttttagtagagacagggtttcaccgtgttagccacgatgttctcaagctcctgaccttgtaatccacctgccttggcctcccaaagtgctggcacgcctagctaatttaagatgcatttctggttgtgctgctgtgaccactaaccagagattagaaaccagctaaggaatcttggagattgcatgtcacccaagctggaaatttcttcccaagtagtggaacagccagggcagagggaacagacgctactgcagactctgcttcagccactgaatcaagggagagagtggcagctccggcagccacggggcagtggaaggacccagtcacgagagttcctggctgtgcctgtggcctgggttagctgctgttcacagtcagaccagcctggctggatgctgacgttgagggctcccatattggcaaaccaagggaggctgcgaaggccagtctcttgtttgcaccatgtccccagaggcctttggtgacacccctgttaaagactgctgtgtctcagtagaaagaattatatacttgaagcttggggatctagagtcagcttctaccactggcactttctatggagccttaggcaagtcactttgatctcttgggtactacaaggggttttggggcaataaataacccagagagcttgctcacatgctgagggtgagacctcgtacaggtgggggagggtgttttgagacttagctgagaacgggtgacaccccacgtgaacatatttattggacagcaagaagcatatggtctctgtgctgggtgggaatgatacatatcaatgacacattatcccaggctggcctcttcttttcttttcttttcttgttttaaatacacaaggtcttggcagggtgcggtggctcacacctgtaatcccagccctttgggaggcgggcggatcgcttgagcccaggagtttgagaccagcctgcgcaacatagtgagaccccatctctacaaaaaaatattaaaaattagccaggcatggtagtgcatgctggtagtcccagccactcaagggactgaggtgggagaatcacctgatcccaggaaggcaaggttgcagtgagctatgattacaccactacactccagcctgggcaacagagtgagaacctgtctcaagaaaaaaaataaataaatacacaacgtcttgctctgtcacccaggctggagagcagtggtgcaatcacgactcaccgcagccttgaactcctgggctcaagcgatcctcctacctcagcaacattgcaaaacccccacctccacaaaaaatttttttttagtttagctgggtgcagtggtgcacacctatagtcccagctactcaggaggccgaggcaacaggattgcttgagcctgagaggacaaggctgccgtgagctctcagggcaccactgcactccaacctgggcaacagagtgagacaccatctctcaaaataaaagaaaaagaaagggggcacagactctggagtcagactgccaagggctgagcctcagctctaccacttaccagctctgtaaccttaagttacttaccctctctctatgccttagtttcttcatttgtaaaatgtggataatttacctgctccatagggcagttgtgaaagtgaaggcacttagaaaagtgcctggtagtaaagatgaagggaggctgggcgcggtggctcacacctgtaatcccagcactctgggaggtcaaggcgggcagatcacttgaggtcaggagttccagaccagcctggccaacatggcgaaaccccctctctactaaaaatataaaagttagccggtcacggtggtgcatgcctatagtcccggctatgctggaggctgagacaggagaattgcttgaacccaggagatggaggctgcagtgagctgagatcacactactgcactccagcctgggtgacagagcgagactccatctcaaaaaaaaaaaaaaaaaccaagatgaaggaaatgtgtgcacagagttccatctttgcagtgtgttacagtgctcagtagattcagagactcatttagatgagagatgggactaggggtggtgtctcacgcaattagccagacatggtgacgggtgcctgtaattccagctactcaggaggctgaggcaggagaatcgcttgaacccgggaggtggaggttgcagtgagctgagatcgtgccactgcactccagcctggatgacagagcgagactccatctgaaagaaaagatagatgagaggtgggtggaggggtgtgagtgaacggccgtcctgatgagattgctccttgcagaggaatgaaggtgatagaaaaccgggccatgaaggatgaggagaagatggagattcaggagatgcagctcaaagaggccaagcacattgcggaagaggctgaccgcaaatacgaggaggtgagtggggctggcagatggcgcagcagcaggaagtgggaggaaatgcatctgctgagatagggaggacaccggggccaacgaaaggaagctctcggttaggtcagctgtcctcctgcgtgaacatatgtttgtccagagacaaccacttggctaggaaactatctcccacgatgccagaaagtgctgcggacgcttgtctaacgtaatgggaaaaccgaatgatcagctcacttgtgtcgttagctgggagttttggcacagttgggcaaaaatggaggattgtggtcccaagccatggagtttcagaccatgcaagctcaggccctcctttgcctccctcgatggctcggctcttccctcccgcctcttgtctgcctcgctcctcaggcttgaggaagagaatcaggatttcctccaggccccaggatggctctttcagttgaagcgccagcaaaaggccaggcgcggtggctcgtacctgtaaccccagcacttcgaccgaggcgggaggatcacctgaggccaggagtttgagaccagcctgggcaacatagtgagaccccatttctaaaaataataataataataattagctgggtgtggtggcatgcacctgtagtcccagctacttgggaggctgaggcaggaggatcgcttgaacctgggaagtcaaggctgcagtgagctctgaccacgccactgcactccagccttggagacagagcaagaccctctgtcaaaaacataaaagggctgggcatggtggctcacgccggtaatcccagcactttgggaggccaaggcaggcagatcacctgaggtcaggagttcatgaccagcctggccaacgtggtgaaaccctgtctctacaaaaaatacaaaaattagccgggcatggtcgtgcatgcctgtaagcccagctatttggaaggctgagacaggagattcacttgaacccaggaggcagaggttgcagtgagtcaaggttgagccactgcatttcagcctgggtgatggagcgagactctgtctcaaaagaataaaaaaataaaaaagaggccaggtgtggtggctcatgcctataatcccagcactctgggaggccgaggtaggtggatcaggaggtcaggaattcgagaccagcctggccactacggtgaaaccccatctcgactgaaaatacaaaaattagctgggcgtggtggcacgcgcctgtagtcccagctacttggaaggctgaggcaggagaatcgcttgaacccaggaggtggaggttgcagtgagccgagactgtgccactgcactccagcctgggcaacagagggagactccgtccccctgcaaaaaaaagaaacaccagaaaaacccatgttgcagctggtctaggggtctgggtggggcatcattgggggctgtctgcagtggatgggagaggacacggctggtggggatcgggctcagctgggcctttctgtctctgcaggtagctcgtaagctggtcatcctggagggtgagctggagagggcagaggagcgtgcggaggtgtctgaactgtgagtggcagaacaggactgagcgaggctggctcgattcctggggcggagtgggaaggagctggctgtgttgggaattggctctgaccggggtctctgctcaagtggacgggcgtcaggggctcatggctcatcttttctcttggcttctgtgacaaagaggtggtgacttgttcttactgccatgggaagcactgcccacgtgttgaccctttctgcaaagatatgaggaaataggagtgagacaggaggcagcagggaagcccagaagtcccattttcccagagaggatatctcagggggctgtgccatcttaacagaacactgacctgctccagaaggcaggctcccccggtcagtatgtaaatgcttttgctcctgtcagtgtttggccgtgacacattcctggcgggaaggtgagaagcttaaccagaatcccacaagcaagcaccgaaaaacaaaacacctgtcctcttggccccgggtgaggaattcagccccacagagcatccgggagtgctgagagagatctggtttcacaaatccactccgggcttccttcccggagtgtcccctgcaaactcccattgctctctgcccgccttctgccctcagtcccattcttacaccttccggagtcggcctcatcaatcatagatttcacaagtccttgcagccttacccttggcaaaagaccaggagtgttttccaagccctccaaatactcttcgggcgcacctcgcctctgcctggtatgataagcctttgataagcccatagtatcacactgcagaaaaatccattaacattttctccccacattccttctgccccccaccgggggagctgtgtaggtttctcctttggaaaatttattgttggggcgattgctattattgccggctgtaagggaagataagacacaaaaatcctttgtctttgtgcagaaaatgtggtgacctggaagaagaactcaagaatgttactaacaatctgaaatctctggaggctgcatctgaaaaggtaggtggttggcttgagctggagggtggcttgctggactttgttcttttcttctcccgagggatgcaggagcctgtcaggttatggggaatctgccctttatttaacagtagcgttggtgcctggcagccagggtttttcccctacagaaagagctggatttctcctgcacactcttgagtcctcttccatggggtctgagcaccatctttgatctccatctcaggaggatagagatagaacatgaggctcttcttagcgagatctgagcatagttgtataaataaatacagagcctgcctctcacctgattcccctggttcctccagaaataccatctcaaaggtatagcaatgatcagaggtggaattgggctttttagtttgaaacagcacccaaagcagttgctacgtggcagctacgtcgggaacaaaggacacacttccacggccgaaccccactgaatttcccagcctcttcctcattcttgctcctgcttttgcagtttcacagacattctttgttctcccatcacctccaccccccacttttttttttttttttttgagacagagcttcgctctgttgcccaggctggaattcagtggcatgatcatagttcattgcagccttgaactcccaggctcaagcgatcctcccacctcagccaccacctgctattcactcaactgggtgtggctttccttttgcttgataaacccctattcagcctttttttttcttttctttttttttgagacagggtctcactctgtcacccaggctggagtgaagtggcgtgatctcagcttactgcagccttcgactcccaagttcaagcaattctcccacctcagcctcccgattacacgctaatttttataatttttggtagagatgaggtttcaccacattggccaggctggtctcgaactcctgatctcaagtgatctgcccgcctcgccctcccaaagtgctgggattacaggcatgacccactgcacctggcctagagatgagatcttgctctgttgcttaggctggaagtgtagtggcgtgatcatagctcactgcaggccccaaactcctgggcttaaataatcctatcacctcagcttcctgagtagctaggacttgcaggcatgtgccactactccaaaactgtatttttttttttttttttatagagcacagtctatgttgcctaggctggtcttaaactcctggcctcaagtgatcctcccaccttagcctcccaaagtgctgggattacaggcgtgggccaccgtgcctggctaatttttctagtttttggtagagacaaggtttcatcatgttggccaggctggtcttgaactcctggcctcaagtgatcctcccaccttggcctcccaaagtgctgggattactttgggaggccgccgagcctggcctcctgttcatcctttgagcttctgcttaaacatcacttctgagagtccttctctgatttctcatctaggttaggtatttctctgctgtgtagccctgtctatacttttgctggcattatgatttcttacatttattatagttactccattaattgcatgccttccttgctagattgtaagttgtaaggacaggaaccatgtcatcttgttcagagttgtgtccctagtactagcattgtgcctggcatatatctgtagtgtgtgtgtgtaattttttttttttttttttttttagtagagatggtgtttcaccatgttgcccaggctgatctcaaactcctggcctcgagtgatccacctgcctctgtctcccatatgtgccagccctggcatatatctgatactaggatgtgtaaggaatgaatccagttggtgtgtgtatgccagacactgccccgggccagggggatagatgtaacaccactaatacctcagctgctttgttttgttttgttttgagatggagccttgctctgtcgcccaggctggagtgcagaggcacgatctcagctcactgcaacctccacctcctaggctcaagcaattctcctgcctcagcctcctgagtaactgggaatacaggcgcacacaccacgcccagctaatttttgtatttttagtagagacggagtttcaccatgttggccaggctcgtctcaaactcctgacctcaagtgatccacccacctcggcctcccaaagggctgggattacaggtgtgagccactgtgcccagcctggcatctgctcttgaagagctcagagtcgagtctagtggaagggattgacaaagtcacagagtgctttgggaatacaatagagggaccttggtaggttgtgaacggtgtcaccaaggaggcgacatttaaaacagctgtaggtccagcacggtggctcatgcctgtaattccagcactttaggaagccgaggcgggaggatcgcttgagctcagaagttcgagaccagcctgggcaacatggagagatcccgtctctaccaaaaatacaaaaactagctgggcatggtggtgcatgcttgtgatcctagctacttgggaggctgaggtgagaggatcacttgagcctggagggcggaggttgcattgagccaagattgccccactgcactccagagtcaggcttcagtcatgacttgatcacttaatagccatgtgaccctaggcaaaataataacttcacctttctgtgaccctttcctcccctataaaatgggattacagataccaggctgtgatgccattaactatgtctggcccatggtaagcagctaataagtgttagttattattgggaggccgaggcaggcggatcacctgaggtcaggagttcgagagcagcctggctggccatcgtagcgaaaccccatctctgctaaaaataacaaaaattagctgggcatggtggtgggcgcctgtaggcccagctacttgggaggctgagtcaggggaattgcttcagcctgggaggcagaagttgcaagtcacagtgagccgagatcgtaccactgcactccagcctgggtgacagagcaagattctgtctgaaaaaaaaaaaaaagaaaagaaaagtataatttctgatgggtcatcatggggaggggaacattccatgctaaggggtgcattcatggacagggactgggactcaggagtccacagattatgatcagggagtgcctgtcaccctggggaaggtggtggagaatggggttggaaatacagagggggccttgagtaacagattcccagttatctccctttcttcgccatactttttatctcaagttctcagtttaggccttctgatcaataccatcctacaggactctccccaacatcctccacatttcacacatatttcttctgctggggaaaggtgcctgcctctactctgcctacttttttttttttttctttttgagatggagtctcactccatcgccccaggctggagtgcggtggcgccatctggcctcactacagcctccacctcctgggtttaagcaattctcatgccttagcctcctgagtagctgagattacaggcacccaccaccacacctggctaatttttgtatttttagtaaagacagcgtttcgccatgttggccaggctggtctcgaactcctgacctcaagcgatccacccgccttggcctcccagagtactgggattacaggcgtgagccaccgtgcctggcctgcttacttctttttatgcttcttcctccttttttttgagatggggtcctgccctgttgcccaggctagagtgtagtggtccaatcagagctctctgcagccttgaattccagggttcaagccatcttccctcctcagcgtccccattagctgggactacaggtgctcaccaccatgactggctaatttttaaattctttgtagagacggggtctcactatgtgacccaggttggtctcaaattcctgggctcaagtaattctcccaccatggtcccccaaaacactggaatcacaggtgagagccaccacacccagccctccttttctttctttctgttttttttttgtttttgttgttgttgttgtttgtttttttgagatggagtcttactctgtcacccaggctggagtgcagtggcgtgatctcggctcactgcaacctccacctcccaggttcgagtgagtcttctgcctcatcctccccagtagctgggactacagctgcatgccaccaagcctggctaatttttgtatttttagtagagacggggtttcaccatgttggccaggctggtctcgaactcctgaccttgtgatccaccagcctcaggctcccaaagtgccaggattccaggcatgagccaccatgcctggctgggcctccttttcttaaagcagtgttttggtttctcccacagtattctgaaaaggaggacaaatatgaagaagaaattaaacttctgtctgacaaactgaaagaggtgagtgtggtggcacccagcgagctctggtttctcctggggctggtcttgaagccatgatagtaactcctttcttcttatctaggctgagacccgtgctgaatttgcagagagaacggttgcaaaactggaaaagacaattgatgacctggaaggtatgaggttaccatctaaatgtttgccttgccctgccttcccctctgggacacatccacggacagttggggaatgtttgtggaggggctgggttgggctttgtttgccttaggaaagtaaagcgcatagtgatgtcatatctggatgtcctggaacactggaataggataatgcaaagcattcaggcttgaatggcccttttttttttttttttttttttctatgagacggagtctggctctgtctcccaggctggatggagtgcagtggcgccatctcggctcactgcaacctgcgcctcccgggttcaagtgattctcctgcctcagcctcccaggtagctgggactacaggcgtgtgccgccacacctggctaattgaattgccactttcaggaggtaaaatatctctgcttagttagtcccatgagcaagtatagagaaaagagtatggctctctctgattaaaaaaatattaataataaattaaaaatctcaggccaggcgcagtggctcaagcctgtaatcctagcactttgggaggccgaggcgggcggatcacttgaaatcaggagtttgagactaacctggccaacatggtgaaaccccgtctctaccaaaaatagaaaaaattagccaggcgtggtggtgcacgcctgtaatcctagctactggggaggctgaggcagggagaatcccttgaacctgggaggcggaggttgcagtaagccaagatcacgccacagctctccagcctgggtgacagagccagactccgtctcaaaaaaaaaaaaacttcacaatttccttctgtttgctcatttctgatagatgccttgcattttttttttacatgccttgcatttttgcagaagctctgtcccagggagctcaaagcttatcatagtatttaaaaaaaaaaacagaaatacagaaagtgtagggactgcaataaagactagtctgcaagtctggggcccacttctcccagaattttttcaagagttccagtgtttaacattcggcctcagaaattccagaatcttggggttcaaatggaatcttccaaactgcccatcccacccagaaaggacacattcttcagaccatatcttccaatgtttttttggggaagtgaggttcccatataagggaaaatgccccattccaaaatacgacctttggacagggtgacgtcattggaaatccgaaataaactgaggggtggggaccagtggggggaagctctgtcacttctggttaccactgttttgaagcttcattgtggctaatccccctgcagaacctcaaaccacttagagatcaactccatagatctttggttttcttcatctgtttcacatggaacacagctttctcctagtctgtgctttgtttgctcacgtgtttttttcttcctcttgtggttcatctgtggcactccattccgacccttgccttctgtcccctgtacttctgaactgtctccctggggacctccgccctctagatgagttatacgctcagaagctcaagtacaaagctatcagcgaggaactggaccacgctctcaacgacatgacctctctctgagaggcagccaggtcgctgccctctgtccttctcacatggtgcctcctacgcccctgtgggcttctaggagctccggtggcctgccttctggtttgaacgtcagagccttcttctgatgtgtctgtgactctacaaccgaaataaagacgggcagtcctcctcttcatgccccctcattctcattttctccacttgctgcctttgagctgtagctgtgtgcccttaaccatagcctgaaacacaaagtgggtggttagcctctctcactcacaaatgaaaagcttattacaaaaagaaaattatgcctacaggatgcttttctgaagacgtgaaaacaaaagcaaactgggcatgtgctctcagataccgctgttagctaacggcatctgcatgccaataatttttttttgtttttttgttttgagacagggtcttgctttgtcacccaggctggagtgcagtgacaccatcatagttcactgcaacctccacctacaaggctcaagctatcctcccacctcgacctcccaagtagctggaactacaggtgtgcaccaccacacaaggctaatttttgtactttttttttttttttttgaggcggagtctcactatgtcgcccaggctggagtgcagtggtgcaatctcggctcactgcaacctccgcctcccgggttcaagcaattctcctgcctcagcctcccaagtagctgagattacaggcatacaccaccacacctggctaatttttcttttggatttttagtagagacagggtttcaccatgttggtcaggctggtctcaaactcctgaccttgtgatccgcctgccttggcctcccaaagtgcagggattacaggcttgagccatcacgcctggccatttttgtactttttgtagaagcgggagggtttcactatgttgcccaggctggtcttgaactgctgggctcaggcagtctgcccacctcaccctcccagggtgctgcaattacaggcatgagccaccgcgcccatccccaatggtttttccttaaatagaaattgttgtgaatggaggctcatccttgtaaaccgcttaggcagcttaagagtcaacagggatttggaaaaaccagcaagcctgtgtcaaaaatgaggctccccttgaatggggcttgagctacagattcaaacagcggcagtgacattttgatctccatttcctccttttcttgtgtcttttctctgtgttacactgtgagtgtggtgactggggcttcccgtggctttactcttcactgttcatccagctcccagtcctgggaggaagttcacctccacgccctgcccttagaaaactgactgtacaaggagtgaacgggcctccatgaacagggaaagtgctgtgacgtcagaagacgtgaatttagaattcttttcccgaattccagaattgcctgagactgctaacatcaatctccattcatatttcagttagttataacaggaaccttgctttagtttagaatagctcttaaggttgacctgtgggtaataaaaggtcatgctttttcctacatgaggaatatggagaaaacaaggtcactcttttttttttttttttttttttttttttttttttcaagacagggtctcactctgttgcccgggctggagtgcagtggcgccatcttggctcactgcaacctccgcctcctgggttcaagtgattctcatgcctcagcctcccgagtagctgggattacagtcgcggaccaccacactcagctaatttttgtactttcagtagagatggggtttcaccatgttagctaggctggtctgaaactcctggcctcaactgatccgcccacctcagcttccaaaaatgctgggattacaggcgtgagccactttgcccggcccaggctatgctttgcttttttttttcttctttctttttgagacggagtttcgctcttgttgcccacgctggagtgcagtggcgccatctctgctcactgcaacctctgcctcacgggttcaagcaattctcctgcctcagcctcccaagtagctgggactacaggcatgcgccaccatgcctggctaattttgtatttttagtagagacagggtttcaccatgttggccaggctggttttgaacccctgacctcaggtgatccacccgcctcggcctcccaaagtgctgggattacaggtgtgagccactgcacctggcccaagctatgcttttctaatgatcaaaaacataccaatttgtcccaaaatttcaaatagtgcatctggttctcccctgcatcctaccaccactaccacctcaaattatcacagataattgacatttagatgttcaagccacatcttccagactaccccttgaacctggaaatggcatgaaaatctccaactagatcctgaattttcggtatccattgttattcctcatcctatttttttgtccaggtgggaagctctgtccccattactctctctattcatccattcctccaaaatgcacctcccctaaaccacctccacctttccaccctcagcctctccctgctcctaactgccgtccatcctgaacttctgcaaaaaccattcccctcacacattgccatatatatgcccttggaaagattacagactgtgtagggggctggtttttgtttggagtctgtgtgtttgtccctggaatttctccaggcatttctggactccaccctttgaagtaactatgcagcctgtctatccagttattctacctaactaagcacataagtggaatttcagagattagtgctatggccgggcacggtggctcacgcctgtaatcccaacactttgggaggccaaggcaggcaggtcacttgaggtcagaagttcaggaccaacctggtcaacatggtgaaactctgtctctactaaaaatgcaaaaattagccgggcatggtcatgggggcctgtaatcccagctactggggaggctgaggtgggaaaatcaatcacttgaacctgggaggcggagcttgctgtgagccaaggtcgaacctttgtactccagcctgggcgacagagtgagactccgcctcaaaaaaaaagaaaagaaaagaaaagagattagcactatggaggtctacactatctgttgatagtctgtgagccttgtcgtgattctcaagggcagttaacactttcagggaaagtcattttatctcagacctaataacaaaatagatgctaaagcatctgagtgacaagatgaagcgaagtcaggatttgtagtcaagagaccagggtttaaggcctggcgcagtggctcacacttgtaatcccagcactttgggaggccaaggcaggcggatcacttgagctcaggagtttgagaccaatctgggcaatatggcaagaccccatctctaaaattattcataataatattttatttttaaaaaattttttaataaaataataaataaagagaccaggatttaaaatcctagctctactactttaaccatgccaacgtgaacaagctgcttaggttttctgcaaaataaaggtgatatctctgttatgaggattaaatgagataatggagaaactggctcgtccaacatagtcagcattcagttaacatctattcacccagactggataggcccaggtcactgatctgtctgatagaatcctcccaggtcatagtcacttgactctgtgtgtgtgtgtgtgtgtgtgtgtgtgtgatggagtcccactctgtcacccaggctggagggcagtgacgcaatctcggctcactgcagtgtccgcctcccgggttcaagtgattctcctgcctcagcctcctgtgtagctgggattacaggtgtgcgccaccacacccggctaattttttgtatttttaagtagagatggggtttcgccatgttggccaggctggtctcgaactccttacatcaaggatccatggtgtctcatgccagtaatcccagcactttgggaggccgaggtgggtggattgcatgagaccagcttgggcaacatggcgaaaccccatctctactaaaaatacaagaattggctgggtgtagtggcacgcacttgtagtcccagctacttgggaggctgaggtagaaggatcacttgagcccaggaggtcaaggctgcagtgagctatgatcatgccactgcactccagcctgggcaacagagcaagaccctgtttaaaaataaataaataagaaaggctgccatcttctgcagtcatttttttctttctgtaaatttccaggctgatgatatcacattttatgaggcattttgctttcccccagcattttaatgagtcttggccttgtcccttatcagccatcacttactgcaaactaagttctctctcgtgctctgtcacgcatagctctaaatggcgtcttttttctctctctctttcttttttaatttaaattgtttcatcagctcagttacttaataacatgcctgtagaatggcttaaatttcgcatttacctggggtttgtctccgttctcctggattcatagacagttacacaattatgtgtataatttaaacagccattcccagaagctccgaaggaaagatgggttacaggattttagatttaactatcaaaggctcaggggctaattaactagcacttgggtggaaatttatattaagtcacacatatctaggactgaaatcttcatgtagcagcacgtcataggttctgaagtatttctcctttattcctcatcataacccccacaccacgcattgatatcgttacccccatttgacagacggggaaaacagacctaggaaggttagatgcttacttaagtgatacaactggagcttaagttcaggtattctgactcaagggttaccagagttcacaaggaaaaatacaggacaccaacttaaatctgagtttcagataagcaatgaataattttttaatcataagtatatctcttgcataagtacatctcatgcaacatttgggatatacttacactaaaatattatttgtggtttatctgaaattcaatttaactgggcgccctgcattttatcttacaactgtgactcccaaatttggtgcttgttccttagtattctgtgatgttctgctgtaattaaaaatacaaagtactggacaggcatggtggctataacccacctgtattcccagcactttgggaggctgagcagatgggttccttgagcccaggagctcaagaccagcctgggtaacatggtgagaccctgtctctagaaaaaatgcaaaaattggccaggtggtggcatgcacctgcagtcccagctatgcgggaggctgaggtgggaggatcacctgagcccagggaggtcaaggctacggtgattcgtgattacgccactgcacttcagcctggacaacagagtgagaccctgtctcaaaaaaaaagtactttctctcttgtgactttcaccctggcagtttcaggtttagaaatctttgggggggtgctgggcatggtggctcacacctgtaatcccagcactttaggaggccaaggtgggtggatcacttgaggtcaagagctcgagaccagcctggctaacatggtgaaaccccatctctactaaaaatacaaaaattagccgggtggtggtggcacgcgtctgtaatcccagctactcgggaggctgaggcaggagaattgcttgagcctggcaggtgaaggttgcagtgagccaagatcgcgccactgcactccagcctgggtgacagaatgagaccctgtctcaagaagaagaaaaaaaaacaaatctttttttttctttcatttaacaaagacgcttattaatttatctttccccatactcttaatcctcaccagagaaacttgcccaggccaaagaagagaacgtgggcttacatcagacactggatcagacactaaacgaacttaactgtatataagcaaaacagaagagtcttgttccaacagaaactctggagctccgtgggtctttctcttctcttgtaagaagttccttttgttattgccatcttcgctttgctggaaatgtcaagcaaattatgaatacatgaccaaatattttgtatcggagaagctttgagcaccagttaaatctcattccttccctttttttttcaaatggcaccagctttttcagctctcttattttttccttaagtagcatttattcctaaggtaggcagggtatttcctagtaagcatactttcttaagacggaggccatttggttcctgggagaataggcagccccacactttgaagaatacagaccccagtatctagtcgtggatataattaaaacgctgaagaccataaccttttgggtcaactgttggtcaaactataggagagaccagggaccatcacatgggtagggattttccatccagagccaataaaaggactggtgggggccgggggtggctattgtgggaagtcataacccacagatagatcaacctaagaatcctggcccttctccactctccaccatgcaggacaaacatcttctcaagcagtcaacgtagaatgcttgggaaatagtcataattacccacatatagtaattaatagatggtaattaattgatccttgatgtgatgttcttttgcatatttccttcattctaaagttgttccctggccgggagcgttggctttcgcctgtaatcccaacactttgggaggccaggacagatcacttgaggtcaggagttcgagaccagcccagccaacatggcgaaaccatgtctctactaaaaatacaaaaattatggtgacgcctgcctgtagtcccagctactcgggaggctgaggcaggaggatcgcttgaacccaggaagtggagactgcagtgagccgatatcgcaccacagcgctccagcctggtcgacagagtgagactccatctcaagaaaaaataaaaataaagttgttctctgaagagcaaatgtctcattccagtaatgacccactcagcaggaatatggtggagttcagtccaattcaggtcagccatatccaaaagaccacaagtcattactaagttgagcaaaagagtttttatctattagcagaaagggcctctctggcagcagagattaaaaactggcccaacttcatttccatacttcagggaacagcaaattgaggatttacttatctaggacttgaattccttctttgggaccaagttaataaaagaccaagaaactcctgattaaactggataatgaaggattctgtagacagggctgcacgtatcggctttgtttgacttctcttttctcagttaacatctcagagctagaacattccacattccccagcagcgtgtgggggctgactaaagtttacaattccaactaaaaatcaccctgcttctggcttatctgaatcccttacccaccccaccccaccaccctactcctatttattcagcaccacactacccaggaaatacactagcaaattgtgcaatggaataaaatccacactttagattcttgcaactgtatcatatgtaatagtatcactttttctacattttggtcaaataaatttttacataaactacaatttgcgtgaattttagaatgtgtgggggtacacagagcattttggttcaacaaatgttaaagggatggaaagggaaaataaccagagccaagaatgtagacaaggttatctatttgctttatactgtgacttcatgatacaaggatattacagtctcattgcaggcgagagcactcagcctcggtcactcgaaaactcctggccttccttatcccctacgctgcctaagccaggctgtgaagaatgagtaggattttaagagataaaagcagggaaaatcatctctgttgcctgagttaggaagatctgcctagctaaggctgagttacacatacaaaggaaagcagaccagcatgggcaccatagtgagaccccgtctacaaacaataacaaaaatttggccaggtacagtggccaaattacacctgtaatcccagcactttgggaggccgaggctggcggaccgcttagggccaggagttcaggaccagcctggccaacattgtgaaaccccatctctactaaaaacacaaaaatgagctgggcatggtggtgcacacctataatcccagctacccgggaggcggaggttgcagtgag

SEQ ID NO: 102 - DNA, 21625 bp, Homo sapiens
gtacttaaaatgtttaaggaccactgatgtattttggcttcatgtatcaattagatttagattttattgttttagagatgggggtctccctttgtcgcccaggctggagttgagctcacctcagcctcaaacgcctgggctcaaactatccttctgcctcagcctcctgagttgctgggactaccatggtgtgccaccaatttttatagagatgtgatctcgctgtgtttcccaggctggtcttgaactcctggtttcaagtgatcctcttgccttggcttcccaaagtgttgggattacaggcgtgagccaccgctcctggccccgatttattaatagatcttataaggacattttaggcctcacgcatcagtttcttaggacaagcttttctctgcactgcataataaatcagacggcagtgcaacaaaaaaacggtgatgatttcccgaagaacaaaccaagttcagaagcctccctaattgtcagaacagcaggtagcctgggcggagctctgaggctatccttaaacaggcgcactgagacgcaaggcgctggaaacaaaagagctcctccttgcgcccttccgccgccccacttagtcctgctccgccccggacaccccgcggccccgcccctgtgcgcgctggttggtcctcgcaggcatgatgaaacttcccgcacgcgttacaggagccaggtcggtataagcgccagcggcctcgccgcccgtcaagctgtccacatccctggcctcagcccgccacatcaccctgacctgcttacgcccaggtgagccgggtcctgcgccccgtgccctgcgccccgcgccagcatcctcctcgcgtgccctggggctgctccggaaggaaggggtggaggatgcggtcttcagcctggcacccggcagacgcggttcgcgggcgcctgctgatgctgcggctcctgcggtagggagggcggggcggacgcctagcgattgttacgcacctgacagctagcggaaggacctttctgtcctggttccctgaagcatcgagagggaaccgcggccggcaggccggaccgctccggagaggaggcagcggcagtttgagcccctgtaaatgttatatgtgtacttttttttactatgtggcgtcgaagcctgtggacattttcgcggtccgggtccctgcggcggacgggtcggatcgtgctcgtggccagggcgcagtcaggtgtcgcgtggtcctgatctaggaagagactgcggccttatcaccgtctcggtgtctgctttcaccttcaactgcccccctcctcacctggaccgctcaccctcctcctcccctctcaccccgccatccccaccagtccccacctgtctctgtagactgcaagactcatcaagtgacttgctgagcaaaccctgccgagaagaggtctgtttagggacacaggcgaccaagtacagaaaaaggcaaaagaactagcatgcctttttcaatggctgtcattttgcagggctggcttcagatgattgttatagctttaaataaaaaggacagttttcatctcggcccgtggcctacattatttctttactgtccattgccctgggcgcttgactaataatttaacagcagtttttttttttaaattttaaatcatgattcatagcattgctgtaagagtaattagaggtaaagtagggcttgaacctgtctgtagttggttacttactgagatcttaatataaaagtaaagggagagggtgaagttgtaagtagcactaagtggaatagaaattaaatgcactgaaactgccatgtccagttcggtaggcgctagccacctgtaactgttgagcacttgaagtgctggctagtcctaactgagatgtattgtgttaaatacactggattttgtcgttggagtaggaagaacagtgtaaaatatctgctcgataatattttatattgattacatatatgttaaaatgttactatttgggacatactgagttaagtttatttaaaattaatttcacctttttcttttaatggggctactagtatatttaaaattacatatgtggcttacatatatatttattggacagcactgttctagaagtttaggaagaaataagaaaaatattgagaacaggtagcggcagtaggaactttgccctcctataagactgattccaataaaaataataggttatagttttaattggctttttcctactagaaaaaataagtgtactttacatgcctctttgttctccctttttcccctccagtttagtggttagaatgtatttattatagcaggattaatacagggattcactaagcagcgttaagaagacttaggtaactgattccctgatgaccatacttgattttcaaagcactttcctaacccgttttaaattgatatagagtcaaaggcagatggcttattagtagtcatctcatttaaatcttatggaatttttccagtaaatctcaaataatttgttataggctatttgggctatttggtcaagtgcatggaagagacagcataggacatgtggtacttcatttccaaattgcttgagatgattttcattctaaccatatattatttggttctggttttccggaaaagccagctaaacctttggttcttttagatataaatgaaatatcatcaaagaatagctcaaagtgacttatgcaacttgaatgtatattttttccttagggtgtttatcccaaactatttgggcatttgctgcaattcgcagtttttttaaaaaaaacaccaaaatagttatttttcaagttagagatgttttaattaaaacatcttgtttttggtgtatccattgacattctcaaaacggaatgtatctggacctctgtgtacaatcttcgtagcactcagacactgaacagaaaggcagtcatcactgccaaacagggcccaaatgccacacatggtgcaatgtgtcattttgagctggcagcagccaaataaaacagccctttatttcacagttgagaatttgaaattggaaagtaattaacgtatgtaagggtgatttatttgcttccgggcttatagggatgagctaagttttttattagggatgttgttggtgtatatgtctcacctactttgcttccttactgaacaatgcaactttgagacagaaatatttgagaacatttttgtcagtgaggacattttgatagtgaatattttgtatcttctattaacttgaaatgttttatttgttataaagccaggatatctgatatcaaattaaattgttttttttttccctttagattttcttcaatcacatctgaataaatcacttgaaggtaacctagatgtaatatagtgaaatgcttgaaagagctgcgtatcttttacacttacagcagtatgattttctgttgtacccattatatggtacctgcagctagttcagataaagagggcatttaactgtcaagggaacctgagaggagactctagtaatctggaaagtctgttggatctttgagggattttgggatggtgagagtggggctaggatctctggctaggttggagccagcctgcatttgtatctgtatcttggaagcaaacttagaatgcagagacagatgtggcatggacgctgtcagctctagccaaccactaaatcctaaggtgggagagatgcaggctttggctaggtgctaagctgctgtagccggttgaatgtagaggtcactatcttttccgaatacctgtaagtaaattaaatcattctctactcccatgtgcctgccaacctaatgggaaatcgctatagaaaagatggtttaaattttagtctttgaagtggtttatgcacgtttccggaatcaagatttaatgcagagttggattggatattgaatatttttgatttgtctgcttttctctccatagaaagcttatagcttcattgcaccatgtgtggcatttgggcgctgtttggcagtgatgattgcctttctgttcagtgtctgagtgctatgaagattgcacacagaggtccagatgcattccgttttgagaatgtcaatggatacaccaactgctgctttggatttcaccggttggcggtagttgacccgctgtttggaatgcagccaattcgagtgaagaaatatccgtatttgtggctctgttacaatggtgaaatctacaaccataagaaggtgaggagaaagaaaccagatgtctggatgcgattaaacttcagagtttgttggttacgatgatgttacatattctgtatcatgctttttcctttgcaaagcactctatgttcgttatctcatttgctctaagtatgtaaatagggaactgatgaataaaaaggtgagtgaaatgacttggtcacaaaaaaagtgataaaaatggggattacagttcagtttcattgactcttagaattttttctccttctccccagcttttcattttgaaaaaattcctaacatacagtaaagaacagaacaacaagcacctagattaaatagtcattaatgttttgccatagttgcttgatttttctttctacacacacacacacacacacacacatgtttttgctgaatcatttgagagtacagtgcagatattatgacactcctaaatatataagcatttatctcctaagaataaggacattcttctacataacatcaatgccattattaaacctaagagtccataataccacctaatatccagttaatacttaaatgaaatttccctaagtgtcccaagaatatttttatttatttatttattttgagacagagtctcattctgtcacccaggctggagtgcagtggtgcgatctcggcttactgcaacctctgcctcccaggttcaagcaattctcctgcctcagcctcccaagtagctgggactacaggcacctgccaccatgcccagctaattttttgtattttagtaaagacagggtttcaccatgttgcccagggtggtctggaactcctgagctcaggtaatctgcccaccttgacctctcaaagtgctaccaagaatatctttatagctggttcttgtttgttttgagccagatttcattcaaggttcatgcatttggttggtatgtttcttggtattttttgagacttcttgatagatacctgtcaggcattgatagagatttacatcctaatcacattttggacatttttatctgtgaacaatagcttttgtcattgtttgttgcctgctcataggaagactcttaataatagtcttctcatttaaaaagttttaaaatagttattcaggaaattccttttacacatttctttattcctttattaagggtctactatgcaccagacatcatttttctaggtgattggagatgaaatggtgaaaaggaaaggcaagaatggaatttcctgctagtgggaggtagaagaagagagtattaaaaattttttctaagtcaaataatgtcatatacatgagaacgctaggtggtattatggcattatcagcttggctttccccttaaatgaaataggaagtgccctgtttcacttgaacagtgttatttcttttattaaaaagttacaagaagttaaatattttgaaaataattaatttctattctaaattagccaaatgttatatttgtaaaagtagagaagtttgttccattgcttctaccaagcatctaagtttatgtagttggggcagctagcagtctgtctaatgagcagaatgtatactttaggcttatataaagtattcagaaatcccccccacacctcctttttggtaaaaataaagtttaccactacaataaaatacagccagaggtgtactgggagtagaaggagactgaatgaaagaaaggaggaatggggtaaaggctggggcaaagagcaggccctctccctgcaggggagtatcagggcctgcagccaagtcaaatgacagcatgacgtcaggaggcaagatttgagggcttttatttaaggtgcagcattggagtttggttttaggagagtaggaagtaatacatccgttacccaaaggacccttctcctttttaaataagttacctgcaaagtttaggccaaagaggtgggtaaggtagatttgggaagctgttgcttactaatatcaccgaatgctttatggtcactaacccttcaggcagttcagcccagaagagtcagcagaagactgtttacaggcccccacctgctagttacagatcatccctgatagagcagagaggggtgaccaggtagtgactttgtagtcactggaggcaaagcccatttttggacagttcagtgaggacttatagacaaaagattcacaaattatggagtgagttggatggagtgtgaagcatatttatgggtcatgcacatacataataggtttactttttgaaatttgaaagcatgttttaagcttatctaggatttccacctgatttaaacctcttctttctctaatgtcagccaaaaacccgagtacaaagaagaaagaggaatacatcaaggacttttcatcctcatagtttgccattaatggctcatagtttgccgttgatggtggagagtgtcagaattggggagtagcctaatcaaaccttcttactctgcatgcagtggcagacagtccctttgctgttcttttggggaatgcagactaataaagcgccaccgtcattttatctatcagtaaggagtagctttaatgctgctgcagtggtggaagcactgggcattgtcatccacccctggggaccagcagctttgttttggatcatgtatctgttattgtgatggagccatttatttttcagggaatgatgccaaatgatgtttgtccctttgctttacatttttatagctaggactttgaagctgaactggaggaacttcttagccaatactatcttctcaaatcaaaagtttatagttgcaaaagacacgttttttagtgtcatggcaaccaggcaacctattatcttaacttaaatttagaggttgagcatccctaatctgaaaatctgaaatttgaaatgctccaaaatctgaaactttttgagcactgacatgacattacatgtgcattttgatgtcacagtcaaaatgcaggtgtaaaacacgcagtttatttggcgttccctagggaaaaaagaccctctcagcccgcttcagctgcagtataacttttctacacatgcccggatttccccatgcaagcacgcccacaaagggtaatagaatggcacatgttcaagctggatacgccattggcaggatccccacagatgggacttatgtgcattatccattgtgtatttttgcttattttctgctctgtggtgttaagatactgaaaatgtcaaaaagacctgtagatatttctatgagcagcagtgataaggaaaagtagaaacacttataacacagaaagtcaagctgtaggagaaactggactgtagtataaaggtatagatgacatggtgaaaatgtgtgatagagatattgaaggactagagctacctgcattcataacagaacaagaggtcatgtcagtttataaaatcaaagagagccttccaagacaaaagccattgttaatgaagcagatgactctggagaaacatttaaaagtcatctggccgaatgcctcttcaatctcagaggacccgcttcctagttgctcagctgcttctgatgtttcttctcacctgaaaaaggaaaaaaaaatacagtgtatagtaaccttttaatcaaaacgcagcattgtaggtggagtctgaaagcctgccattgtttgtacagctgtttaacagctgatgcaggtattctggtgattctactatgctacttattactttcttactgtattaatggtatgtcatattttataagcatatgaaaatgattgctcatcagcagcataataaattcagagtcaggaatgatggtcaatgatgtcaaacagccacagattttccacatggtagctgagatagtgacccctttgctttctgatggttccatgtatgcaaactttgtttcatgcacaaaattatttgaaatattatataaaattacctttaggttttgtgtataagatatatgaaacataaatgaagttcatgtttagacttgggtctcatgcccaagatatctcacatatatgcaaatattccaaagtccaaaacacaaaacacttctggttccaaacatttcagataagggatactcaatctgtatatatataaatatatgtatgtattacatatatggtatgtatataatatacatttccatccctccacaggttactgttctggcacattcccattatgttctgtttatcagactgcaactaaaattttcatgggttcggctttatgttgaacagaatttgcagaatatgagttgaagcgaaccatagtttaataatgctgtgattctcctaaatcaccaaagtgcatgaaaggattatagagctcagaaatactgaagcatctttgcaataaaaaattattagtgaatgtacaaggagtctaacattttggttttgctttcgcttcctaagatgcaacagcattttgaatttgaataccagaccaaagtggatggtgagataatccttcatctttatgacaaaggaggaattgagcaaacaatttgtatgttggatggtgtgtttgcatttgttttactggatactgccaataagaaagtgttcctgggtagagatacatatggagtcagacctttgtttaaagcaatgacagaagatggatttttggctgtatgttcagaagctaaaggtaataataaatttttctatagattttcattattgtcttggttgtacgttttcttttaaattatatttgaaaatctcttagagagcaatccagaattttacaagtgactaagttatgagtctttacctttttttaaaaaaacagaggagttgtactctccttttcagcacttaaattctgtaatccttgaaggatgattctttagtgcagtcgtttattttttgctgtgctaatatgctctacatctagcttgatcttaagtgcagttttaagttttcctgtgtcatactataatcgtagggttgactctgcaattattgcattgtggtactttgcgcagttatagcacagcaagtgttaggatttctaaaacagctttattgataattcacataccatgtaattcacccacttgaagtatacagttcagtggtttttagtatattcacagatgttggtaaacaacactccaatcagttttaggattgtttttccacctcaaaaaaaaccaaatcaaatcctatgccctttaccttagtttttgctggcaggatcaactaggtttttgtttgtttgtttgtttgaagagatggggtcttgctcagtcgcccagcccaggctggagtgcggtggtttgatagctcagtgcagccttgaactcgtgggctcaagcgattctcccacctcagcctccctagtagctaggagtataggcatgcaccacaacaccctgcctcctgtgccctttagctttgaattccatctctccatatccatcagctgcacccctgcagttgtagccccggcaatcaccagtctttctgcctctggattccctattctgtatgtttcatatgaacgggattatatatcataccggcttttgtgactggattctttcacttggtatagtgctttcaagatttgtctatgccgtagcatgtatcagtacttacttcttatggccaaatgatattccattacatggatacactgcattttgtttattcgcttgtcagttgatggacatttaggacattatttaccccttttggctattatgaataatgctgctataaacattggtgtacaagtttttgtgtggacatttcccttgggtgtatatctaggagtagaattgctgggacacatgataactatgttcagttgaagaactgccagactaatttttgaaatggctgcatcattttttattcactccagcagtgtattaaaatttctgtttctccacatcttcacaaacagtgtgtgactttaattctagccattctagtgtatgtgaagtggtatctcattgtgattttgatttgtattttcctgttgacagtgatgtccagcatcttatcttatgcttattggccatttgtatatcttctttggagaaatatttgttcagatcctttgccatttttttttcctgttagggatcattttattttaaaaacataatagactttatttttttttttgagcagttttagaaaaaattgagaggaaagtgcagagagttcacatatgctccccctacagtgcccctgcccagttttccccactcttaacatcttgcattactgtgctacatttattagatttgatgaactgatacttatatattaactgaagttcatagtttacataagggttcactctttgtgttttatagatttttggatttgacaaatgtttaatgccatgtacccaccattacagtattatgtagaacagtttcattgccctaaaaatctcctgtgctccacttattctttcctcccgtcctcttcctcctaaccccccagtcattactgatctttttgctttctctctcactttgcctttcccagaatgtcgtataatagttgtaatcatatagtatgtagctttttcagactggcttctttcacctagcagtatacatttatagttcttctgtgttttttcatggcttgatagctcatttattattattattattatactttaagttctagggtacatgtgcataacgtgcaggtttgttacatatgtatacatgtgccatgttggtgtgcttgctgaataatattccatttgtttgcatgcaatgcaatttgtttatccattcttgaattacccatttctaattgagttattttgtctttttattactgaattgtaatagttccttatgtattctagatacaaatcccttctgttcatcagggttgcaggatacaagatgaatatacaaaaatcaatggtatttgacacactttaactgaatactacatacttaaaatgagcaatcaaaatgaaattaagaaagcaacttcatttataatagcatcaaaaagaataaaatacttagaaataaatttaagaagtgtaaaacttgtactctgaaaactataaaatgttgttgaaagaaatgagaggagatctaaataaatggaaaagtatcccatgatcatgatttgaaggcttaacattgttaagatggcagtcctccctaaactgatttacagatttaacttgatccctatcagaatcccagatgagttctttgtgaaatctacaagctgactctcaaattcatatggaattgcaagagactaagaatagccaaaacaatcttttgaaaatgaagaacaaagtaggagacctcatattaactgattttaaaacttactacaagacaatggtaataaggacaatataatactgacagaaggatagatgtatagactagtgggatagaattgagagtcagaaatgaacccatacatatatgatcaacttatttttgacaagggtgccaagattattcagtggagaaagaagtttgaaaactggcacaggggcaaccagatatgtaaccatatgcaaaacttggagttgaatctttacccaacatcgtatacaaaaattatggatacagaaaaatggatcaggccaggcgcgatggcttatgcctgtaatcccagcactttgggaggccgaggcgggtggatcacgaggtcaggagatcgagaccatcctggctaacacagtgaaaccccgtctctactaaaaattagccgggcgtggtggcgggcgcctgtagtcccagctactcaggaggctgaggcaggagaatggcgtgaacccgggagacggagcttgcggtaagccgagatcgcgcaactgcactccagcctgagtgacagagcgagactcatctcaaaaaaaaaaaaaaaaaggatcaaatgaatcagttttgaactaatccacttaaatgtaagggctaaaactataaaatcccgagaagcaaacatagaagtaaattgtcatgaccctggatttggcaaagctttcttaaatatgagaccagcaacaataataaaaatcaatgaattggacttcatcaaaattaaacatttttgcacatcaaaggacaccatcaagaaagtgaaaagacggcccacaagttggaagaaaatacttgcaaatcatgcatagcactttttgatggtaaacttgaggaagacatttatcttttatcccttacctgtgcagcagtaacatcctaatatctctctccctgcctctttttgccattctttaaattctttctcacttaattttcagatttaatattggctgaagcagggataatgagatcaatcaaaggggtccttaggacactagtcacagtgtttgtactaatactggaactggcttattttcaggcatttctagtgtgatcagatggcaaagaacaagcatatatatatgtcagttgccaggactgctgggaaagcctggtaaagagaacactggggaaaagcagcctcctgctcccctgggccttctttgagcctgatgatcacttgatatggaacttaccctctgaaattccttaattgttcttttctatatccttgacactgtccttttccagaccaaattatctcatctggaatactgcaacaattttcttttctcagtgcttttagaataacctgtcaaaatctcatctgattatagtattgcctgcttaaaaccttttaattactccccattccctatccgggttgtgtagctcacttgagctctgctggctggtgagggaatctgggtcctttttctggtatttgaattcagtgctacacaggttactggctgggtagacaatctcaaattgtaaatcacgagtattccatgtagatagtccattacgatctacaataaaacattgatgtttgtatcaaagatcatggtgatgagaggttgggtactgtactgtctgtgagaatttattgaggaaatttaagttatatggttttattcacatatagtgtataacaactagttaagggatagatgtcttcttatctgactttaaagtaggtaaaagtggatcattgtacttgttaaaggtctgggaaccatggctgtgttctgaaaatacctcagtgatgacaaataaatgactcccagcctatcataacattaggactccagttcatccctttgcttcataagtgtgtcttttccttttgtgtatttgctttagtatagaaaataggttttcttgattagaaatctaagaagaagaaattgaacactggagatttttctatttctttgaattacgaaaagttagtgtaatttggcagtatatccctgtgccattattgtctctcaggtaagtagatggtagggcttaggaaaatagaaaattttttttcctattttgcttatttaatgggtatgtgtttgtattaaaaagggaaaataggaatgtagatgatgttaactaatcgtgaaagttattgggaagggttacctaatttgaataaaggtatcattgtgaatttctaggtcttgttacattgaagcactccgcgactccctttttaaaagtggagccttttcttcctggacactatgaagttttggatttaaagccaaatggcaaagttgcatccgtggaaatggttaaatatcatcactgtcgggatgtacccctgcacgccctctatgacaatgtggagaaactctttccaggtagcagacacccacccacctattccccatccttctccaagggaaaaaaattttaagttgtattctcccatcatttgaatgattttagtttcaagacctacttcctattttgtttggagggaacacattaagatttggcacactccaccattgagtaaataccatcatgatagatgttgatgattgtgtatttcatttcaataactaatccagcccaagattttctggagctgtttgatttactgctgtgtttataggttttgagatagaaactgtgaagaacaacctcaggatcctttttaataatgctgtaaagaaacgtttgatgacagacagaaggattggctgccttttatcaggtgaagtcaattaaaaaaacctaattatatttcatgtgtgtttaattgaaatgatttgtagccatccctttggtttttactataaaatatttactgtatgatttactctttccttcattataggatggaaatgattttttataagctgtatttaatagtcatagtcatactccaacttgagttacactatagctatgttattggtgttaagagtgagtcagtgaatgttctttagaattctgtgtagtgatttttaaccaattcaaatactactattatcacagtttatatatttttctcttgttgaagttgatttcagtttataaaacttggcggattttaaatagtaaaactatgatcttggtgtttatcaggaatatacatcttctgtccctgtcttatgcaaggcacataactaggacacttccacttcctcttttgcatgtagggggcttggactccagcttggttgctgccactctgttgaagcagctgaaagaagcccaagtacagtatcctctccagacatttgcaattggcatggaagacagccccgatttactggctgctagaaaggtaaggtgctgtctctgtcccttgtgtagtgtagttagagtagacttgttattagaatgaaaatggagtcaataatgggtgattctactgctgctgtattgactgggtcaattgttttaaattgattgtattaaaatagaatgaaatggctgttggatatgcactgtgttgtacactgtcctctgtgtacttttatctgttatgacccatgcaattctcacaaagaccctatgatgataagtatgctcttttgaaagtaaaggtgtctgggcatggtggcctacacctgtaatcccagcactttacgaggctgagggaggtagattacctgaggtcaggagtttgaaaccagcctgagcaacataatgaaactccatctctacaaaaaaatacaaaaactagccaggcttggtgacgcatgcctgtagtcttagccttatgggagcctgggtgacagagtgagaccttgtctcaaaaaaaaaagaaagtaaaggcataagtcaggtgcagtggcacacacctatagtcccagatacttgggaggctgtggggggaggtctgagctcaggagttcaagtccaggctgggcaacgtagcaagaccccatcttgaaaaattaaaaaaacgggttttttgttcgtttttttttttttttttttttaaacgtaaaggcatagtatcatggctaagactgcagactttggaacctgacttgtggtttgaaatcctggctctactcatttatgtaaccaaaataatagtgtctgctatggggaaattttaaggtgaaatgatataattcatgtaaagtaagtagggtagaacttagcatgtagtaagtacttaatgagtgttagctgttattattatttttgaaagtactgtatttagaatactgtgggcagagggcagcttgtctgtattcagtgagcgggagacctagttcccactatggaggactttcgtagcatggatgagaaaaagctagagagcagtctcagtgcaaggtaatcaatgccgagagaatccaaaatagccaaggaaagcagaatgaggggaagggccattctatataagaataacatcctggatataaaattaggcatttaagaaggaccaaaaaagaccaagcttagcgtgggaccatgttggactagagagagatgaggtgggttaggtaaaataggtagagagggaggtgccaactgggagaatggttgaagccttggcaccagaggagctgaggggagacttacttcctggtggtggagttgaagcaggcgagggaacagtgctggatggggcttgtatgtggtgggctgtaaagtcatttttctttttttcccttgtttagttttcaccattgttaattcataaagctttgtgaactcccatcatgtttgattttcaagggaagttattttctttaacaagtaaatgggtatttctttatataataaggtggcagatcatattggaagtgaacattatgaagtcctttttaactctgaggaaggcattcaggctctggatgaagtcatattttccttggaaacttatgacattacaacagttcgtgcttcagtaggtaaggtattatgatattcttaaataaaaagctttttttaatactgaaaaaaatgtaaggtttaaaaaaattatttcaagccatagttttaaaatgttatttaaggatgaatgcaaattaaatccctatgttactgattatttaagaccacttaagaattctctgaatctcttttggagtgaagggaatagtaaatacgtagttcaacctccacattgttggtgtcactgttggtgtttccccagggagcagatacatattttctgccctctacctcccatttctcttatagtttcttgggctacagtctatatacagtgaggaaataggtctttttggtaatgcatttttgataagaaatagtcattttagatatattccatcacacaacttaccagtcactagctatcattgctctgcaaacaatactaattttatcttgtagataatgtatctactgagattggaagtataccccaaatcagactgatccagtgttattgagcctttatatgctactgcctcccttgagagacttgccttggaaggcaaaaatatcttaggtattacaatggtttatggccctccaaaacatcacagtaaataagcagatagacaggatagctctggtattggaatttcatggggctggggtgaggttaggaaaataagtgtctaaaaaggctctctagctgaggtgataataaaaacaaggttgagaagaaacactggtttagagagatgtggtgcaggaccaaggaggcaagtttaataacttatatagtctccccagctttatgtgaaatctggtaaatggggagtggcagggggaaaatacccatcaaaattaacactaaaccaccaaaacggttattcttatttttgtgtcataataccactatgaaaggcatgatttttaggtatttgagtcattgttcagcttagcaaagttttgaggtggacattcttggtctaaaaacattagaattttaaaacctgtttagaaaatgacaaaatggttccgggttattttattttacagtagtacttttggattaagtacatataaatggcttataaatacaaggtcattattgtggaaactactttatattaatatgaagtccagtatagtagtaaagctttcaattatttccaaaaatcaaatcaaaggcatttttggtggaaggttatgttgacattaaagttaatttctctctctcatttaaggtatgtatttaatttccaagtatattcggaagaacacagatagcgtggtgatcttctctggagaaggatcagatgaacttacgcagggttacatatattttcacaaggtaaccactctgaagtggagggatattcatgctatattaagaaaagtatgaattgtttgactattttctatcatctttcagtatgacagtgatatttttgagtatcttgtgaggttacaaaagggaatctgatagtgtttgctttctatctcttggggaagaaagaaattttaatgtgtcagataatttttattctttaaaactagttacagctgggtatgagggctcatgctcatacccccagctgctgaggaggctgaggtgggaggatcacctgaacccaggagattgaggctgcagtgagctgtgattgcaccactgcactcctgcctggttgacagagtaagaccccgtctcttaaaaaaaaaaaaaaaaaagttaaaaataaataaataaaactacttaagcttgagaatcccctttctgccatttcttagcatcctgtggaattatgactgttgcccattgtgttcattttattctaatattagcagtttggtaggaaggaaggcatgttttgtgaagcattgcttacctctgttcagttatttactcccttccctaaatttgtttaactttttgtcttatccacctttaggattggagagggagaaagaaaaactgctttgtgtgccaaaagcaaaactcttggtgtttttgtttgtgaaataggctccttctcctgaaaaagccgaggaggagagtgagaggcttctgagggaactctatttgtttgatgttctccgcgcagatcgaactactgctgcccatgggtaatatttttagaggctattgtaaaacaaaaacaaaaaaacaccaaaaacaaaacaaaacaaaaagctcaataccctgagaaaataaaaatcaatagctgattggctatatgttacatatagttggctatatgttacaaagtgtgacttttatagagaaaatgaagctgtttcttaactttgtcccaaaaggattaggccacatttcaaagtggtgttgtggtatatggagagaagtcttcttccataggttgtttgaggtggagttttcacctttaaagggtaacaacattctgctcacatctgaacaaccaagatggaagaggcaaggctgctacagcagctaccgttaagtgttttaaagagaagtaaagatcgtaaacatcatgtgacaagtagtgagtgcccaccatgcccatgtggtgctgtagtgaccctgagggaatagagtagtgaagatacaaggggtttgattacattataaagaaccaggtttctttggttatcatttctagttgtctaaagttatgttgaagaactgaagacttttactgtacaggataaacaactgacattaaatgtcttagttgcctctgctgaatcacacctagataaggatataattaaatatgggtttgaggaatgaactgaatctggtcattatcctctctgcttgtcctaactagagtcactaggcttcaggaaaccggtgatttggaatttgatgaaatatagtgggacactggtttatatcgcatattgtatgtgaatttttaatcagtggcaaaaaaatactgtatcgtcatcacaattgttagaagagatggtctcacctagtaaacactgagttaggtctaggcaaggtattttcttaatgattgggtcactcatgttttgtaactttttctgctttttgaaatatgcatttaactattcctagaagggaaagtaaaagtaatagtctcagttagttttactccctagatgacatgatatatgtattattttaaatgaagatttattttttgtatctattcattagtgtagggcagtcattaggaggcttgtatgtgactgtatgaccttaacatttcttaagatctggttgaattgatgggaaactgaatcagaacctaacctggcaggcactaaatacccattttaatttagattttcttcttttctcctttaagtcttgaactgagagtcccatttctagatcatcgattttcttcctattacttgtctctgccaccagaaatgagaattccaaaggtaggtaaatcaactcaaggtaaaactgtccattgccatcagattatatttgtaatttttacctgatgctcctttttttgtcacgtcagaatgggatagaaaaacatctcctgagagagacgtttgaggattccaatctgatacccaaagagattctctggcgaccaaaagaagccttcagtgatggaataacttcagttaagaattcctggtttaagattttacaggaatacgttgaacatcaggtataatgtctttaaaaacattttcaggaataagacagtttggatgcagagctgtcattgctgttcattttgtatttagtttgaatgatacatgtatttagtttgaatgatacatgtatttagtttgaatgatacatacatcagatatctctctgataggatgtccctatcagagagattcagagtctctgtaaacaattatctcttttgtaagaattacgtaagaattaagtagcatgaaggattataaagtagcatctagaatcgagagagagaggagacttactactaatcatcactgattttcatttatcagatttttgggcacctgctgggtgccagatcttgttaggcacaaatgactaaaacagagccaccaagtattaaaaatatgcatatgagtgttctttaaaaggcactgcagctatccatattatgaatactttagcattttctaagtgatgggtgattcaaagggtctcatacaagttacagtcacgtcttaacattttctgtttcgtgaaatgagactaaacacaagtatttcctgccattttaagccattttgctcttatatgcttattcttacaggttgatgatgcaatgatggcaaatgcagcccagaaatttcccttcaatactcctaaaaccaaagaaggatattactaccgtcaagtctttgaacgccattacccaggccgggctgactggctgagccattactggatgcccaagtggatcaatgccactgacccttctgcccgcacgctgacccactacaagtcagctgtcaaagcttaggtggtctttatgctgtaatgtgaaagcaaatatttcttcgtgttggatggggactgtgggtagataggggaacaatgagagtcaactcaggctaacttgggtgtgaaaaaaataaaagtcctaaatctaaaccattgctgtagtcatttatgttcatgcagtctcttcataagaggtaactagaactgttttgctgtatcacagtaaagtggagggtaagctaggaaaagggaaaatgatcagatgtctgcaagaactcacagccctctcctggcagagctgctttagatgacatttgcatcttgtgcccgtgtggcttccttccagtccttgcctcatcttagggacgtcatcaaaggactacactatttttgttctgcctacattcctaacagctgcctaggcagactcagacttgaatcttctataggagttcatcacagctctattttgcaagatagtagttcatttttttctcttttatgttgagccaaagccacttctggagacttgtcctagagcaggggtcaggctttttttgaatttttaatttgtttttaataaagagccagatagtaaatattttaggctttgtggacctcttttggaactgttcagctctgccattatagtgcaaaagcagttacataggcaatatgtaaacaaacgagcgtggccatgttctattaaaagttacttatgaaagcagatggtgggccagatacggcctgtgggccatag

SEQ ID NO: 103 - DNA, 13776 bp, Homo sapiens
gtgcgacccgctaagggccccgcgaggtgggcaggccaggtattcttgaccttcgtggggtagaagaagccaccgtggctgggagagggccctgctcacagccacacgtttacttcgctgcaggtcccgagcttctgccccaggtgggcaaagcatccgggaaatgccctccgctgcccgaggggagcccagagcccgtgctttctattaaatgttgtaaatgccgcctctcccactttatcaccaaatggaagggaagaattcttccaaggcgccctccctttcctgccatagacctgcaacccacctaagctgcacgtcggagtcgcgggcctgggtgaatccgggggccttgggggacccgggcaactagacccgcctgcgtcctccagggcagctccgcgctcggtggcgcggttgaatcactggggtgagtcatcccttgcagggtcccggagtttcctaccgggaggaggcggggcaggggtgtggactcgccgggggccgcccaccgcgacggcaagtgacccgggccgggggcggggagtcgggaggagcggcgggggcgggcgccgggggcgggcagaggcgcgggagagcgcgccgccggccctttatagcgcgcggggcaccggctccccaagactgcgagctccccgcaccccctcgcactccctctggccggcccagggcgccttcagcccaacctccccagccccacgggcgccacggaacccgctcgatctcgccgccaactggtagacatggagacccctgcctggccccgggtcccgcgccccgagaccgccgtcgctcggacgctcctgctcggctgggtcttcgcccaggtggccggcgcttcaggtgagtggcaccagcccctggaagcccggggcgcgccacacgcaggagggaggcgacagtcctggctggcagcgggctcgccctggttccccggggcgcccatgttgtcccccgcgcctacgggactcggctgcgctcacccagcccggcttgaatgaaccgagtccgtcgggcgccggcgggagttgcagggagggagttggcgccccagaccccgctgccccttccgctggagagttttgctcggggtgtccgagtaattggactgttgttgcataagcggacttttagctcccgctttaactctggggaaagggcttcccagtgagttgcgaccttcaatatgataggacttgtgcctgcgtctgcacgtgttggcgtgcagaggtttggatattatctttcattatatgtgcatcttcccttaataaagagcgtccctggtcttttcctggccatctttgttctaggtttgggtagaggcaatccaaaagggctggattgctgcttagattggagcaggtacaacgttgtgcatgccccgtatttctacgaggtgttcgggacggcgtagagactgggacctgctgcgtactggcaaagcagaccttcataagaaataatcctgatccaatacagccgacggtgtgacaggccacacgtccccgtgggtctctgtggaagtttcagtgtagcgacatttcagataaaagtggaaaaagtgaagtttggcttttttcatttgtatgcagtcctaactcttgtcacacgtgtgggatttatctttttccataacttactgaaaacccttcctggcgggctgaacctgactcttcctgagctgagtcctggactggcacactgatggctctgggctcttcccggtcaagttataacaaggctttgcccatgaataatttcaaacgaaaatgtcaagatccttgccggtgtcctgggattacaaggtgaatcttgtcatgaagaaattctaggtctagaaaaaatttgaagattctttttctcttgataattcactaatgaagcttttgtggttgaaaaataaaaagtgaggtttatggtgatgtcaggtgggaaggtgttttatacatcaatacattcgagtgctctgaagtgcatgtaataatagctgtttctctgttgtttaaaggcactacaaatactgtggcagcatataatttaacttggaaatcaactaatttcaagacaattttggagtgggaacccaaacccgtcaatcaagtctacactgttcaaataaggtaagctgggtacagaaaaagaaaattaaggtctttgatgtttctactgtcctatgctgaacaagaatgtctttaaagctgattactggatgaaattatttaacagatgacgaagaagaagggattcttggcaattcgctggccggtgtcatactctattaggcctgcaacatttccagaccttaaactgatagaacattttaattgttttaattgtttttggaaatgatgggagagttcctaagtggagtataaactgtggagagatgaaccatcttgagtaggcactgaagtgtgctttgggtcatgatagattaattaatctcatctaaacattgatgtctttttctgttgctgtctagactgtgaacaatgtctaacaccttagggaagaggtggggaggaatcccaatgtatacattgcccttaagcagtgtttgattcattcatctttggactccatgaatcgaaatctggtagaatacatgatcttagtggaggaggccaaatgcgtgactcactgagcctggcagagcagaaatactctgctgtctgcaccctctgggtctggtgtggctctgcttcttggtgcctcaactctgactggcagctgtccccaggaggcgataattcagcatgttcaatctaaaggttatgacttccttgatggttttcaccatattcttggcaagtttttggtttttgaaatgttctaggaggcttggtagagatcttatgaaatagagaatagctgctgtggaaattattttaatgctaattacataaaagtacaaaagtagcactagctaaaacaaaaggtattttgctgttctgttttgttttagcttgtgccaggccttttacagcattaggaatgcaacttctagataacgatgcatcttttaagtgaatgttcttgtttttcaaaatgaacttcatgacagtagttgccaaaccagcaaggagaacttgcatgcatacgtgcatgcatgtgtggatatgtatgggggtggggggagagaaagatgaaggaatttcataacatgaaataatgattacagttctggtcaaacttgtcaattcagatttcaccaattgagaattagtaagtaatttctctgatacaggcctgaagtttaccttagtaaacactttacttccatatggtaaaaattagattttgggaggaatgcttacctcctaaatatattcaatctaatatttgagggacacatgggaatatatttatgattcatctgctttttaaacataagcctttgttaactgtaagttcttgaactttataaggctgctgttatttaaatgagcacagctcctgatctgcaaacagcagagcgcagggctacagcttgggggatgccagccgactcagggtggtcctatggactgaacaatctcttgctgctgtactggagggcctgggagcttttccatcagcctcggcctgaggtgtgcactcttctcctgcccaccccaggaataaatgagattcctggttaaaaaggaccagagcagtcattttacagttgaggaaactgttgctctgagaagtgagggatttattcatgactacactgatggtgagtgcccatgtcaggtctggaaccaaagtctacccagtatccacacaccaccatccctcaggtggctctgccacagtctgatgggaggctccaaagcgggaggaagaaggaaagtcttgcccactgcatctcctcagttggccttcctctctgcctgttttccctccctacagttagcatcttaagcagctgcccctcttccctcccgactgctctcactactgcagcctggctccagccgcaggacactactgctgtgcagaagcccctacttggaactccaactgcatttttcacctttgctaacagttttcagtggtggttgggaaatgttattggcttaagccttagcacaaaccgtcaccggtgatattcattccatggaaatgttctgaattctaaagctgaatttacaaagcttctggaaaacaacctgcaaccaaattagtgactgaattttttagttaactcaaaattccaaatcagagggttttgcaatgcctggaggaaccttggaggcttttaaagtgttaatgctattaatggcattcagagggattttctacagaattgtcccttcattacctgtttatacagttttactacttaccagggtactgtataaatccttgtgctaaattttgctatagagtatgtggtccctgctgtgagctgggaggaaccaaatactgtatctctatgttacatagaaagccctaggagactttctcctgttatctgaacaactatttgctgtactgataaaaaggaaacagcatagtctcattcactttttgaaatggaaatgataaaataaaacacattttggtcattcgggaacaaaataccctctctacttttatcacataaaattaaataaatagaaaccaaaatatttcagtatcaatcttagtttgtgcactttaggataaagaatgtgtttacccaaatccttttggcctggttacttagttcagattttgaaagaaaatatatttgtggcttttatgtgtgaatttagacaatggaatccatgtggtgcctcgttttccctgagattatgtattaattcaacctgtaaatgcaaaccatctaatagtcagcgagaccctatagccctgctgcttaatgggggcacacaagggcatgcagccctcgtaccaggcagactgtgttcatattaacagcatcgtggagaaactcatgctgggggacaggggagggagatgtaaatgctcagcagggagatctggagattcctggagcaggtggagttgggacctggccttgaacgatgggtctggctctggcagtcagtaatgccaaagggaagagcagcataactgtcactttccatgggacagaagtgtgtgaatcaagttgcagtgacgcttcacctatttattattttggtcatttagaagaatttcattgtcagtagaagtcctttaaatcatttccccttcagtgacgtctcacaaaagaaagatctgtctttagctttttagtctcagactttattagacagatactacctgtactcttattctgtaatctttgttgggatggattcacatcttgcaaaggaagggaggcatgtagtataatggggcaaacagacccagctctgccactcgttagatatgtgaccttctgcaagttgcttagtgcctgtgagcttcagtgtcctcatggataagaaagatccaacaccttcttggaaggattatatcaaatgaagtaacatgagtaaagggtccagcagaatacctggcatatagtggagtcaatgaatgattaataatattattaatagtggtcatgagagaatatatgtataacatgttattatgtagactcactatatagactctattctacatagaatatagaacattatataacaaacaactataataagtagactatagtaaacaacctcactttgtctcagttgcctcatcttgatggaaaactgctctttctctcctgttaccctgacagagagcgtctacattctaaaagaaagatatttaacaaaatggttgagtacagatccaagagtcaaatagctgtctggttcaaagtccagctgtgtgattttgagctagtcacccaatctcactttgtctcagtagccttatttgtaaaaacaaggcaaattacagagccatcccctgggttgctatgaggactcaaacatgcatcccaagtgctcggtgttgctaggtatgatggctcacacctgtacattcagcactttgggaggccgaagcagaaggatcagcctgggcaacatagcaggaccccatctctacaaaacaatgtttaaaaaaaagcaaagtgctcagcacagtgactgcatcattaggattgattgtagggctcctgatgttagcacagaacaccacagccaggaagcagtctatcttgttgggtgcaaattgtaacattccatttatgtttcttccttcttttctttctttagcactaagtcaggagattggaaaagcaaatgcttttacacaacagacacagagtgtgacctcaccgacgagattgtgaaggatgtgaagcagacgtacttggcacgggtcttctcctacccggcagggaatgtggagagcaccggttctgctggggagcctctgtatgagaactccccagagttcacaccttacctggagagtaagtggcttgggctgtaataccgttcattcttgttagaaacgtctgaacattctcgtgatcttgtgcctttaggggctacaaaattaaaaatatttattctttttttctcagaaactggtatgtatcacagccctcttcacacattccagatgtggtaggaggttcacagaatgtgaactttggagctgatgacagtgtcatcaagtaactttctcccccagtctgtccccagaccctgttactgtcctcagtaaccggctgaatgtgtgttgggagagggcgggccagggaagcgggtagggataggaaatccaccaaggccggggttttagcttttccctatatatatatcatgtatcctgatttttctgtcccgttatcacactaaaaatcccagttgaggatttttcccaaacggtcataaatcaatgaggaaagtccatggtttccctctgagcccataattagcctaattatgctgaccttttctaatcagttggccatgatttgagttccgtgatgtgccagcacctgcccagccatctgcctgtcaccctcgttctggttttggaaaggtggaatactttcctcctcagcctttgcccctgtaagctggccctaggagccagtaaaagaatgaagagaattcctgtcaagtaggagatttattcttttgccgcaactgtggctctgagctaggcaatttagataaatgcatgtagcacattgagtagagtgaaattagcttctcttgtaaggccagctggttagaatgaaggtgttgtgtgagtgttaggcccagcgagagagaacagtttctcaaggtaggaatggtgaaaagaaggggtggacggacaaccaaccaaccatcctcctctggtatctactttgagggttgaaatagggggcctgaccccaggtgaatgtggctgccttcccagagcccccatttgcaagaccctccagacccccaggtgcttctgcttgtgtcttttgtggcaccaggcaagaatgtagcagcgtcagcagcccctctggtgactgtggcatggttgacattcatttcccccctaattaatggcatcctcatgattctcttttatattaatagttcttgagtttttttgtaagctacttcaaatcctttgttggtgcaagatagaagatattttatgtgtttgttttgcatgtgcacacacatatttggcctgtgaattgatgtttgttttcctgtcatttaaccaaagcacatgagataattgagccattgcagagaccccgtggttaaatccggcttctcgaggtaccaaggacatttcctgggctttctcacagccctacatatttttgaacctaaaatatcgtagtttatgctaccaccctgttcagtatagtagccactagccacatgtggctgttgaccacttgaaatatggctaatgctctaagtataaagtacacactggaatttaagaagtgtagaatatctcaaaacttttttatattgattacacattaaaatgattatattccagatatatgcagttgactcaagcaatgcatggctgagaggcaccgactccctgtgcagttgaaaatccgagtataacttgactccccaaaaacttaactactaatagcctacctatcggttgactgttgactgcagccttaccaataagataaacagtcaattaacacacatttttcatgttgcgtgtattatatactgtattcttacaataaagtaagctagaggaaagaaaatgttattaagaaaattataaggaaaagaggctgggcatggtggctcgtgcctgtaatctcagaactttgggatgctaaggcgggtggatcacttgaggtcaggagttcaagaccagcctggccaacatggtgaaaccccatctctactaaaaatacaaaaattagccaggcgtggttgtgggtgcctgtaatcccagctacttgggaggctgaggcaggagaatcacttcaacccaggtggaggaggttgcagtgaactgagattgcgccactgcactccggcctgggtgacagagcgagactctgtctaaaaaagaaagggaaagaaagaaaaaaaagaaaagaaaagaaaagaaagaaggaaggaagagaaagaattataaggaagagaaaatatatttactattgataaagtggaagtggatcatcataaaggtgttcatcctcgtcatcttcatgttgagtaggctgaggaggaggaggaggaggaagagcaggggccacggcaggagaaaagatggaggaagtaggaggcggcacacttggtgtaacttttatttaaaaaaatttgcatacaagtggatccacagagttcaaacccatgttgttcaggggtcaactgtctttggttaaataaaatatattattaaaattaatttcacctgttcctttttactttttctaatgtgactactagaaaacttaaaatgacatctgaggctccattgtcttccccttgggccagcactaccacagaatgtcttaggattcagctccaggccgccacgcctgcttctttcagggagctggttctatgcacatgttttatatgagagataattaagttgtcaattgtgataacaaaacaggatttgactttgtacagaattctttggttccaaccaagctcatttcctttgtttcagcaaacctcggacagccaacaattcagagttttgaacaggtgggaacaaaagtgaatgtgaccgtagaagatgaacggactttagtcagaaggaacaacactttcctaagcctccgggatgtttttggcaaggacttaatttatacactttattattggaaatcttcaagttcaggaaaggtgagcattttttaatttgtttttatgacctgttttaaattgtgaatacttgggttttacaacccatttcttccccaattcaaaaatagcagaacagagttgttgagaaggtgatggagtagaagggggagcgcgcactgtggggaggggtggacaacaggcctggtcctacctgtgactctgcactaccctgtgactctgggcagggccccctcggagacccaggttcctcagccaaccggctggatcaggtcatctctaaaggtcccgccatgctcacatttctccctctattgaggatcccaggcacaaaatttgtttttggttcaatgcataatactcccttcctttttcttttactgcagatatcttctaaaggggctcaatagggttcaatatgcctaaattggatcttctcagtcttggaaaaggcatttttagcagtgatcaagggaaactgattagcgaagtcacttctaatccttcacgtgtcagctgtgttcttgtaggctttgcttagaacctaggtttttacttccacagtgacttaataaaggggaaagaattgactcagagcccagatgaattaagaactctatctttttacagaaaacagccaaaacaaacactaatgagtttttgattgatgtggataaaggagaaaactactgtttcagtgttcaagcagtgattccctcccgaacagttaaccggaagagtacagacagcccggtagagtgtatgggccaggagaaaggggaattcagaggtgagtggctctgccagccatttgcctgggggtatgggtgctgtgggtgacttctggaggagtagctccaccctcagggctgggatatacttccttggttaaatattcaggaaaacaaactgcctggaggttttttgttgttatttgtttgttttggttttgattttgctttggtacaaaaaagattttggacatttagaaatgtttctgtgttgattgtgcccttgtattagcaggtgttttcttgagcacctgtcatgtgctaagccctctgctgagcactggatacacaaactgtgtttaggatttagcaacaagtcacagatttccctgggcattttttcatgcttaaattctaattctgggggtggcttctggaccagctgcagcaggacacagtagacattcgtgagtacccactgtgggctgttgccacagaggctgtagagtctaacccatcaagggaagggattgagtatatcaaatatacccacatgcatgcatgtgtgtatatggcggacacgtgtgtgtacatgcatgtgcatatgttgggagctcaggcccattgtgcgaggaacagtccctaaccggaagtgctgtgggccttcagactcttgcaggaagctgcaagcctgtgtgtctcgatccatgccttacagggaaagtattctgagtacttccagtgaagaaaagagtcaggggatataaacgatggcttacgctgggtgtggtggctcacgcctgtagtccctgcactttgggaggcccagacaggcaaatcacttgaggtcaggagtttgggaccagcctggccaacatggtaaaagcccatctctactcaaaatacaaaaagtagctgggtgtggttgcacgtgtctgtagtcccagctactcaggaggttgaggcaggagaattgcttgaacctgggaggcggaggctgaagtgagctgagattggaccactgtactccagcctgggtgacagagcgagattccatctcaaaaaaaaaaaaaaaagaaacaacgaaaaaagaaatgatggcttagctccatgtgaagatgatatttgaacattttaaaacactttaaataaactgttctctcctgtttattgccactgacaggagaggtttctctttacctctggtcctgcacccctctgagccatcctacccacagccttcagtcattgtcctaaagcctagctctaattccactgcctctccttttgtgcacacacacttctctgcttccctggccgttctctatcttggagaggcatttcaaacgccacttccaccagaaggccttgctactgcaccaactagttactatctcttcttcacccaaatcctggtagcactttggatctcccactttgcacttagggttcaccttccgttataatcattgccatcaatctcagcatcgtttttaggcacttctttccagccattgttcttacctccaactacatatcttttctggactgtgcattattcagtttattaaatgcccattaaatgtgtttagccattgtcaattactctgaaacgttcaggttttgacaaattctttcctaatgtaagtgtggtggaaagagtgaaagaaagtcaaattgcacaaaaataggatggtgtaatttggggttatgccgtcaattttgtccactgataaatgggatttgagctctccaagttgactagatgccctttatttttcagaaatattctacatcattggagctgtggtatttgtggtcatcatccttgtcatcatcctggctatatctctacacaagtgtagaaaggcaggagtggggcagagctggaaggagaactccccactgaatgtttcataaaggaagcactgttggagctactgcaaatgctatattgcactgtgaccgagaacttttaagaggatagaatacatggaaacgcaaatgagtatttcggagcatgaagaccctggagttcaaaaaactcttgatatgacctgttattaccattagcattctggttttgacatcagcattagtcactttgaaatgtaacgaatggtactacaaccaattccaagttttaatttttaacaccatggcaccttttgcacataacatgctttagattatatattccgcactcaaggagtaaccaggtcgtccaagcaaaaacaaatgggaaaatgtcttaaaaaatcctgggtggacttttgaaaagcttttttttttttttttttttttttgagacggagtcttgctctgttgcccaggctggagtgcagtagcacgatctcggctcactgcaccctccgtctctcgggttcaagcaattgtctgcctcagcctcccgagtagctgggattacaggtgcgcactaccacgccaagctaatttttgtattttttagtagagatggggtttcaccatcttggccaggctggtcttgaattcctgacctcaggtgatccacccaccttggcctcccaaagtgctagtattatgggcgtgaaccaccatgcccagccgaaaagcttttgaggggctgacttcaatccatgtaggaaagtaaaatggaaggaaattgggtgcatttctaggacttttctaacatatgtctataatatagtgtttaggttcttttttttttcaggaatacatttggaaattcaaaacaattggcaaactttgtattaatgtgttaagtgcaggagacattggtattctgggcaccttcctaatatgctttacaatctgcactttaactgacttaagtggcattaaacatttgagagctaactatatttttataagactactatacaaactacagagtttatgatttaaggtacttaaagcttctatggttgacattgtatatataattttttaaaaaggttttctatatggggattttctatttatgtaggtaatattgttctatttgtatatattgagataatttatttaatatactttaaataaaggtgactgggaattgttactgttgtacttattctatcttccatttattatttatgtacaatttggtgtttgtattagctctactacagtaaatgactgtaaaattgtcagtggcttacaacaacgtatctttttcgcttataatacattttggtgactgtaggctgactgcacttcttctcaatgttttctcattctaggatgcaaaccaatggagaagcccctaattagatcagggcagagggaaaaacaaaaaactggtagaaaccggcaaccacagcttcaagctttaagcccatctcctacacttctgctctgtaggtgcccattgtcacttctgttcacatgctactgtcccaagcaagtgaccaagcctgacaatactttgtctactggagtcactgcaaggcacatgacggggcagggatgtcgtcttacagggaagagaaaagataatgctctctactgcagacttggagagatttcttcccattggcagtagtttgactaattggagatgagaaaaaaagaaacattcttgggatgattgtattgaaacaaaattaggtaaaaggacaatataggatagggagagatataagtggaatgagatctctagagtccattaaaagcaagctagattgagagctcttggagggcagggactgggcctagctcatggtttacagctcttgagggtgactgcacag

SEQ ID NO: 104 - DNA, 109476 bp, Homo sapiens
acccccggggccctccggctgggcggcgccagcggatgtgagctcaggctcagcggtcgcattttgcgagtggctccgagacacacaatgcagcagaagtaaattccccagcagcaaagccgcctggccgcacagaagtaagtaactaaccgggcaaccacctagcaccatcttcccgggcacaggagcggagacccggcctcaaccacaaccccaggccagcagcacagacccaagaactgcgtggtcaggcctttccgcgtagccccgcccgcgtagccccgccaaacagccaatggacgcgcagctcgacgctccgcgcacctccgccaaccaactagaaaaggtcgagcagacgggcggggctactccgccctctgcttctgcttctcgattcctcttctgggtctcatgctcctccttcttttgcgccgaatgcgttctccaatcggatccgtcgacccccctaggtgggcgtgcccggcagccgacggggcggggcggatatgactggcgggccgactagtgctggttgccaccgccggtttagaaatcctattctcgcgccggggactggatttttccctacgtcagcgcagctaggcgatgtcgggagcgagctcggaccgagggctcagttgcgtcagtgccgcgcgcgtgctcgtcgggcgcgcgtgctcgtcgggcgcgcgcgcttcccggccagacttggggccccggcagggttggaaaatgatggaagaggcggaggtggaggcgaccgagtgctgagaggaacctgcggaatcggccgagatggggtctggcgcgcgctttccctcggggacccttcgtgtccggtggttgctgttgcttggcctggtgggcccagtcctcggtgcggcgcggccaggtgggtgtccgcgccccgggtcggttgggacggctgcttcctagggacggggcgctcggagtgaacctgtggtgcctgggagtggaggggcccggcctggggatcggacccggggtcggggggcgcggccgctccaggtgtgtgcggaccggggtcgcacccgaggcgcggggtttggcgccccaagcccttcttggcccgggtcctctgcccggcaccgcttcctccgtgtcctgttcgatggagccgttcccagcgtccccccatccctcgccgcctcgcgcgaccccgggtcccccagacgccccgaaacccgctctggggcgggcgctgacctcggcgggccggagccctgcaggctgggcgcgcccgcgggcgttcagtcctccaaacgcctgcagggagggagctggctctcgctcgtggagttaatgtcgcttggaaagagactgagagatgaaacttttgctgcaggttataatttgaaattttgacgttcatggtatccttgggtcaacacagctaaatttaatggtggaataaaggtgggtgggaggacgctcatttctcttgggtcatttttgtagtaagaatattttgtaaacgatgtgctacctttctatagccaaaccattcttaaaaaatctgtgtttttattgggttcgtactgtgttaaatccggacagataatccctgctcttttgaactcacaggattattgtaggaattaaatcatttgtgtgaaatcgtttttgaattgtgaaactgcccttgactatgtaagatacttgtattggagatgcccaaacatagtggaagcagattgtcagcacgctggcgtctttctggaaacaagttgtttattttggattttgtatgatataattgtttgcatggctgtattttctctatcagcgacagaggatgatggagaatgggagtttttactaaatcattgattgaaagttattcaaaggtgatgatagaagatttcaacgcaggactgttgaccttcaggaaactaattacttgtttttcttatctttggctgctttatttgaaattaagtaaatttgccccagtgtggaaatgttgaaactctgacaatgttttgaatgggaagttgccaaatttcttctggttaaaactacttttccggtggtattctagatggttaacactcaccgatgtttaaggtgaagacgattatacatccggagttttattaatctgtgatttttttttgtgtttgtaaatgtaaataagactgtatttttaaatgttaatataaattgtcagtcattaccgacctgcattaggtgagtggaatatcctgatggtctttaactgtggttttggccagctcctcacttcggcatgtgtatgccccttcaaagtttagccaccgtttatggaactcctataaacaccacacagttgattgtagaggggcagaaggtgaccaaatatgctaagcgcatctgagagatgttggggaagatttttagagaaaataatatttgaactgggctacatcggtgatttttcaagtagaatagtagatacattctaagcagaggaaagtttttgcaagagtatggtggggcggggggcgtatgaaagaacatgactttttaggaaatgataaaaatgtcaatatgtcttcatgcagactataaaagggagggatggaagatcaaactaaggtaggttgttaccagttgggaagagtcttctatgctgaactaaggggtttggacttcaccccgtaggaagttctttgggcagtggaggttttaagtaggggtgcgacctaatctcattttctgttaagaaaacgggcaacacggtggaggatagaatctaggagggagagactagaggctgggacaccggttaagaggcttttgtaatagtgtgcagtgagtcaactcttgtttctctcggggaacgttcatacaaaatcagctgaccacatttttgcagtataaggtgtttaaaacgtgcactgaaacattttccaggatcgaaagaggaatttgaggtaccaggcacacgtcagttacattaggagttaattaggttttataggatttttactaccttttataacattgtctcaatgaggaaatgcagtataatttccaaacagctaactttcagtaaactttttttttttttttaaactgacaaaggtaactgtgtcattgtaaaaaataagcggaatcaggtatgaaacctcttctgattttctaaggtagtaattatgaggaacagatttagaatttttttttaaacaaagactggcattctaaagaaaatgactttgaaagcttactcatggtgagtcactgtaaaatcatttgtgtagtaagaacttaggtccatactaatctcgttttcagatgccagcaaaatatttgaatttgatatgtttgtgtttgtgccgataggagaatgtagccttttacatttaagaatgatttggttttcaaccttttaagtaaaaaagaaagcatatataattaaaatatgtacaaacctagttcctggtttccaagacagttttcaaaaagcacttgaagctttaacttaccaaatttatatttgctctttgtaaaaaatctgggtttataatagaatttattatggaatcccccaaaagatgcaagctctaagtaactggaagctttttcttgggaatatccgcaagctcaaacatatgacatagcctcatatttctttttcctttttggtatgtaacatatactggaggcttggagtcatgccatccttttgagtcagcgctatggaactgcctcataaatgaatgcagtccttttgtatctcagtagctaatccctcacagtctttttttttttgagatggagtcttgctgtgtcgcccaggctggagtgcagtggcacgatctcggcccactgcaaccttcacctcccgagttcaagcaattctcctgcctcagccttatgcctggctagttttttgtatttttagtagagatggagtttcacggtattagccaggatggtctcgacctcctgacctcgtgatccgcccacctcagcctcccaaagcgctgagactacaggcatgagccaccgcgccccagcctctctcacagtctttgaatgggtctaatgtggacccaactaaagttgggtagcacaatgttgtttgtatattgagagattattgtagtttattttccatttcatgttgttattttaatcagattattttccctaagtgatcatatgtgggacactgcttgagtcacatcttttttttttctttctgagagacagggtcttgctctgttgcccaggctggagtgcagtggaacagtcatagatcactgtaacctcgaattcctgggctgaagcaatcctcctgcctaagcctcctgagtagctgggactgcaggggtgtgtcaccatgcttggctaattaaaaactttttttgtgtgtggagaggcaatcttgctctgttgcccaggctggtctcgaactcctgggctcaagtgttcctcctgcatcagcctcccaaagtgctgggattacaggtgtgaaccaccacacctggccttaaatcacatcttttaagagtgagctagggaaccttagaaattaacttggtccgttttaaaatatgcagttctgtttgtatttatttatgtttatggtaatgtaagtattgtgttactaaaccttactggaagaaaagaaaatgatatcacccccagacatgttataatgtagggcagaactcaaagggaatgggacgttccctttgatgaattgttcttttaatgagatttttcatgatttaagtcattttaggatgattttaacgtcttccttctagtagtgtagaatcttcatatgagtagaccccaggagagcctgattctaatcagtcttattgaaaggctgagaatcctgttgtgaagatatcttgggcctaacctcccatcccagccacttaagagaagtgattaagcagtctgtggatagcaatacaatgaaatacgattttgctatcaaaatgacaaatgtgtaggctatgtagatttgtagaaaagttgatacaaaagatgttaatcataaaaagtaaggttcactttaagtcatatgtgataattacaactatcagaactatgtttgtttagctgtaaccatcagaagaggttatttattcaacacatattttattgaatacgtactgtaccagtgcaggaagtacatgatgaataagataccgtccttgatctcaaagaacttaaattctttgctggaggaacttaaattgtctagggcattaaatcttagaaatgggtggtgtttttcccaaagggacacttaaacaaacaacagaagccatttctttttaaatgtaaagatgggtaaatatttaagaaaagtgtaacactaaaaaaagtaagagtgtagacctagcagtagaaattataattaagtatgtttgaaggtagttttttttttttttgagatggagtctcacactgttgcccagactggagtgcaatggctcgatctcagctcactgcaacctctgcctcccaggttcaagcgatccttctgcctcagcctcctgagtagctgggattacaggcgcgtgcgccaccacacctggctaaattttgtatttttagtagagacagggtttcaccatgttggcaaggctggtcttgaactcctgaccttgtgatccacccgcctcggcctcccaaagtgctgggattacaggcatgagccaccacgcccagcccaaaggtagttattaatatacggtatgtatttatctggaattgacctggcgaatactagaatgattaaaaaaaaaaaaaaaaaaaaggcaaaaactgcaattacttttgcaccaacctattatatggctcgaaataatagtgctttgtagatctaattgaaacaatttctctacaagaaatactttggaaacagaattatcttatttatcctgaatgtggaggccaggtttatttttattttctacagtggaagtacttaaaagtggctgtttgtttatgtagtaggcaggagaagcccatggtttggagttcacatttgtttgctttgcaattaggtagaattcttttttttttttttttttttttttgagacagagtctcactctgttgcccagactggggtgcagtggcacaatctggggtcactgcaacctccacctcccaggttcaagtgattcttctgcctcagcctcccgagtagctgggactacaggcacgcaccaccacgcccggctaatttttgtatttttttttagtaaagacggggtttcaccatattggccaggctggtctggaattcctgacctcgtgatccgcctgcctcggcctcccaaattgctgggactataggcttgagccactgtgcccggccacaattaggtagaactcttttaactcacttccctgtactacaattactattatgaaaagtgtgctcagacttcctctaaaacacactacagtgtatagaaagatctacggagttagagaaagaaagaagtgcaactaacaccttttcctttctttaagattagacatgttaagtttcatgtttcagtggttcacgttttctcttcaggccgttttctctttttctttttttttagacggagtctccctcggaggttgcccaggctggagtgcagtggtgcaatctcagctcactgcaacctccccctcctgggctaaagtggttctcagctcactgcaacctccccatcctggctcaagtggtctcgtgcctcagcctcccgagtagctgggacaacaggagagcgccaccaggcctggctaattttgcatgttttgtagaggcagggtttcaccatgttggccaggctggtctcagactcttgataaaataaatgattaattgtggcattttggttttcaaaatgagaattgtgtttaaaatgcaaaagagggaaagaaagttatatgtaatcttcctatatttagcttttattttacttcattggcagtctgggtaaaaaattcatagaagacagaagacttggtttctagtcttggcctgaaacttttagctgtcacaactgggggatgctgttggcatctagtgggtggaggccagggatgctgcaaaacattccacagtacacaggacagcgcccttacaggttgaaggtttatacaaataatattaaagctctttttttatattaatgtggaaaaatgttattttggttcccatgagaaactgctactatttggaatttaaaaaaaaaaaaaacaactaaagggaatttggggaaaatctatgcaggatatgaacaggaaaaaagaaaaaaacctgacctagagataagaaaggaattttgggaaaaaaacatgggaaggaggattttcatacaattagtatgtattattttgatgacattcccccagtatgtgcatttgttatgatgttttggaactttttatggcatggctttaattcagaaagtggttgcttggattttagaagcaagatgtcaatatcagaataacagcccttacacacagaaattatttcagggtgctataattttgaaagtcttttaaaaataagtgattagttacggcattttgcttttcaaatgagaattgtgtttaaaatggaaaagaaggaaaaaaagttacgtataatcttcctatatttagcttttattttacttcattggcagtctcggtaaaagattcatagaagacagaagacttggtttctagttttggcctgaaactataagtaaagtaaactaactttgcctataaagtaactgaacctgtttcaaaatgaaagctctttaaatacctgcctgcccataagaactacagatgctttatttttggaggcatttctttttctctgttatgtttggttctgagttgtaacgaaaaaacttcagtttggttctatattgtttagcttctagtgtaacagttgtctgtgtctatcagcatatgtattctttattttttttttttggcagggtctccctctgttgctcaggctggagtgcagttgcataatcatggctcactgcagccttgatctcccaggctcaggtgatccttccactttagcctcctgagtagctgggaccacaggcatgtgccaccatgccccactaatttttaaatttttttgaagagacagggtcttgctctgttgctcaggctggtcttgagctcttgggctcaagtgatcctcctgccttggcctcccaaagtgctaggattacagggttgagctaccatgcctggccagcatatgtaatcttgtctgtaatgatttacttaaagagaatttttttttaaaaagtgaaagcatgtttattaagaaagtaaaggaataaaagaatggctactccacgagcagaacagtggcacgggctgctcagctgagtatactgatagttgcttcttggttatatgccaaacaaggggtggattattcatgagttttctgggaaaggggcaaggatttttagaccatataaggtaacttctgggcattgccatggcatttgtaaactgtcatggtgctggtgggagtgtcttttagcatgctaatgtattataattagcatataatgagcagtgaggacgaccagaggtcactttcctcgcagtcttggttttggtgggttttagctggcttctttaccgcaaactgttttatcagcaaagtctctgtgacttgtatcttgtactgacctcctatctcattctgtgactaagaatgcctaaccttctgggaatgcagcccagtaggtctcagccttattttatccagcctctattcaagttggagtcagtctggtctgagtgctgctgacatattttccctcatccttttacatgggaaccttaatcctaaagattgtagagggacaaagatctatcttctgtgacttcttcaggctgaataggggcaatcatgttcctgcctaactatagggtatcttgtatccggggtagagaggagctcagtcacacaacgtcattatgctgagggccattcacaactctgagttctgttgagttcacaacacaaaaggtgatatctagaagattagtaagattaataattaataagtgttcaatttaagaaaacattcagtaagcttatcctgcattcctacacaaagattacaatagcaatatatttcatgacagtatagcaaataagtaaaattattccaagtaaactaaatagaaagctgttccatgaactgggcaattgttggaacccagctgatatagggtcactaactgattccaatatatgcccagaattagaatactgatccagatgttaacattagccatccctcttgtttattctgagctgcagttagagatcactgattggttcactgaaataagcagagtcagtccaaattgcagggaaaaactcagaaacaactgatgagactagaatttaatgtcaggtgtactatagttcttgaaacgtaatttttccctttcctgtcctccattttcattaaaaacaaatcatgataggactgataggatatgatgggtagcaaaataagctttagtcttattatgcttggcctgattgtttgaaataattgcagtaagaataattatttgccacataggcactttttaattggctttgatggaactttgttccataaggaatctcacctgagatgttttttaaagcagagctcagccatgggtttgcacagttaaatacaggtatgagttgggtaaattcctctcctcttgaggtcccaagataacttgacacacctgggactgtagatagtgacagtctttatttacaacagatcaggaacctcgtacagggactgtgtagacaaggtatgtggccagttttctcaaggggcttttatcggttctataaatcaagtttgattccttaaaggaaagcacaacattccagtcaaaacttggtaaaataaccagtttctccagttgtgtcctgtgcaaaagaaaacagattcttacagaaatataagggattgatgggtaaagagtttaaaagctgtttatacatgcagtacattggatatgatataatttatggtttcttgtttgcagctgtttgtatctttttaatcccaaaccagacaaaattataaacattttatatacaatgttatcttggaaaaagttagatgtaaataattcatcttaatctatatttgagaaatctgaggggtattaggaaactcatgagtgaatgaacatatagattggatcaaaggaggagagtatgagagtagggagaccaggtaaaaaggtatcatagtcatctagaggtgaggttagtaagggttaagccattggtaataatgctggaagaaaaagaggttgtgttggacttatcgagagactatgtattggactcccacatggtgtgtcttcctaagagatttgtgttggcaattttgattatactcaatttcaattcaagtgatgactttagaacccaagccctgcttaagacatcatgattccatgcggatagactgaacagaattggaaatgggagttagtctgcatgactttcagagctcttaactgttaagaaattttgcttaaaatttgtgtttttgtgatggattaatggctataatttgaaagcgtggctacattgttgagtatgtatttgtcagagttaacccatcagatattaaaagtaccttttccctcttacagtccttgtccatttaataagtgtcttagtctgtgttgctataaaggagtacctgagactgggtaatttataaagaaaagaggtttatttgattcactgcaggctgtacaggaagcatggcacaggcatctgcttctggtgagggctttaggctgcttccattcatggcagaaggggaagcggagctggcgggtacagaggtcataaggcaagaggaagcaagagagatgggggagagaggctctttttaacaaccagctcttgagggaactaatagaacaagaactctttctcctaccctggcccctcagggatggcattactctgttcatgagggatccacttcaatgaccccaacacctgttactacaccccacctcccaacactggcacactgggggttaaatttcagcgtgagatttggagaagtcaaacatacaaactgtagcagtaagtatttagtagtatcatctgagaggatgttattcatgctgggtgagggggaggaatgggagatgagtgaagggtgctagactctaggatgcctttcccccatttccccaccaaaccagttcttttctttcttcttgtgtttataccttaagatttcttttgagaaaaaagggttagggtttatagctaaaaatgtttgaaatgattgctatgtatatttataatgtttggataaagactgatattcttttttaagaaaatacattttcctccctcatacttacctaatgcattgctattttcatgtattaatacaactttatatgagtacttttattatatgcatattgtaatatgggaatgtcaggtgatttttctgtgatttgaacattttgatttttcattatattgtgttcccacgtagtttttcagtttcacttattatatttgtttttgccttttctgtaggctttcaacagacctcacatctttcttcttatgaaattataactccttggagattaactagagaaagaagagaagcccctaggccctattcaaaacaagtaagttataattgttgagaaataatatgtggttaatttttttcttttctgttttagcacaaaggtgttatttgtagcagtgatcagttcagtgagttattacttggctgttacttagaatagcaccatatggtactgatgtcccctggatgttatgctagtaaaagcaacatattgagccttaatatcctttttttttttttaaaatggagtcttgctctgtcgcccaggctggagtgtgcagtggtgtgatctcggctcactgcaacctccaccttctgggttcaagtgattctcctgcctcagccttctgagtagctgggactacaggcatgtgccaccatgtctggctaattttttggtatttttcagtagagacagggtttcaccatgttggccaggctgatcttgaagtcctgacctcaggtcattcgcctgcctcggccttgcaaagtgctgggattacaggtgtgagccaccacgcccagccagtatcttttcttttttaaagacaatatgatcaactcgaaacataacagaatagaatagttaaacaaaattgtatcactagggtaggctgctgattatatacattttaactgacaggcaatggtcacagtgattttattataataagaattataattcttactataattatataacctcactcagtttgtgatagctagaacactttatactatatcttcactgacggtggagagtgataatgtgttaaatgcgtatattttatattagggaatatttactaaaatacaagttttattttcatattggaagaaacctactgtgctgtaaatggggtaaccagtgcacaaaaattattttttctactattcttttgtaaagtttgttcagaagtaatcttatttggactttaattttataagtccttcaactttatagaagtataattaaattttattataatttaacaatgacaggtaataatgcatagaatttagcttatgaattgtattaatatctgaattgctgatacactcagaaatgtaaggcagcgtgcctgttttttagggagtgggcattgtaaaaagaacactggagttgaggatcaggaacttttagttttggtcctccctgtgagtaccaccacctactagttgggttggtcactcaactccatttacatctctccaactgaggagtaaatgactctaagatctcctctgtagatgaatttatacattttacttgtttttggtttgaactgggcagactaccatttgattatgttttgtcttaggatagagttaatcagttaatccctgtttgggtgcgatcttggctcactgcagcctccgcctcctgggttcaagtgattctcgtgcctctgcctcctgagtagctgggactacaggcatgtgccactatacccagctaatttcgtatctttagttgagatggggttttgccatgttggccaggctggtctcgaactcttggcttcaagtgatccacctgcttcagcctcccagagtgctgggattacaggcatgagccacctgttttcctccttttctacagtcaatggtagactttcagcctagggaccatgttttctccttttttgtgtctctgatagtatcttcatttagtacttccctcattaatacttgggatcgtcatagataattgtcatttttatgctttggttaatatttggagaagtgatatagtcagtgcatattgaactggattttgctcattcaacagtgaatgtaattaactcgttaaaaagtatttattgagttactattgtatgctaggcaccatttaggtattggggatacggcagtgaacaaaacagacaaaaatttatgcccttgcatgaatgcagtcttgtattctatggagcttgcattctagtgatggggggggggggcagggagagagagagagagagagagacaaaaacaaaaacaacaacaacaaaaacaaacccccccccccaaaccaaaaatgtatattacttcagatggtgataagtgctatggagaaaattaaagcaagaagggggatagggaggctggaaatggtgagttgctggggagaggattgcatttttcagtaggatggccagggaaagccttacgagaaggtagccctttagtaaagactagaaggaggggggtgaacaatccaggcagatacttgggggaggagtaaactatcacaaaacaatcttcagtttctcagatttctttttagtagacatagcagtgatgttattacatcacgtgattatctaagagcagaatgagtagaaaggcacatgacaaagctgtggcaatagaaagagcttggtggttttgctggcccactggagactgaggtagatgatgaagggttcttggattcccatgcaggatgtggaggtggatgacaggatccataggttggtctagcgcttagaagtcagaggcagatgtgccgtggtgaaggggttgatgctgtttcttgacaaaaggttaactgagtctggaaacggaagggaatattaagtagacacttctgataatgttagttgtcgagtccctccatgactttcttttttattaaagagttaaggcgaagtcacatctcttagttccagagatcacgttaagcacttgtggctaatgacatggtgaattgctggggaagttgtttcagagttgcctgaggtagagaagatgatcccatgaattggaggatgtgtatatatgttactttaattccttgactctaagatgccatcaattgtgagacacaccatattgttttatgtaccactaataaagacacggaagtggcccagcagggtggtttatgcctgtaatcccagcattttgggaagctgggtggatcacctcaggtcaggagttcaagaccagccttaccaatgtggtgaaaccccgtctctactaaaaatgcaaaaattagccgggtgtgttggtggacgcctgtaatcccagttacttgggaggctgagacaggagaatttcctgaacccgggaggcagaggttgcagtgagccgagattgtgccactgcattccagactaggtgacagagtgagactccatctcaaaaaaaaaaaaaaaaagacagaggtgctgctagttagtctagactgctttgcctttgtatgatgcatcctcatttcaaggacgttaatgtgagggaaaaaagcatgttttagaattgataaaatgaggtaagccctgtaatttgtatcataaaaggagttgaatttctttttaactttatataagtagaactaggtataatttcttgaaaccaagagtttcatttcatttagacaaaagcaggaactatctttgtactgtaggtaatacatcgatggacttgagaagataatccctgcagttatagctgaattagaaatgaatttaagaagagttagatagacatggggttattttccatgatcagttatgaaaggaaggaagggatgatcagagtatattttttattatttaagaatagacacaaagttcttctattaaatagttcagccaataccaaattattttaattcaggatggaatttcctgcatcttataaatgagatgttgttgaaaagtaatttttaagatgatgttttattcttttccccttctgtgcatttaggtatcttatgttattcaggctgaaggaaaagagcatattattcacttggaaaggaacaagtaagacatttaatttattttggcttttcagtaatgtttttccaatagtatattggttttctttctagtttgatatggtttagtggatcctgaaccctgggattaagcagatttagctcttcatattggtgctgcacagtggcagctggctgggcaggcagtgacttctaaacaggaaagaaggcagagactggaaccaagtacctccagtttattcttttcaaatgcatcactaagggagcaaaggctacacatatgtgggggagttggggagaaggggagcctgcagtgactgaatagggtccaattactggaaagactaaggttccacaggctacttctatgcctactcacatagactttaataaaggtaaaggatataatgcatcaggacaaagaaagtgcaggcagtcatcaaggcatgacccccagagtcctttctcagttgcacagatgtgctttgcctccagattatgaaccgctgagatatgtgtgaggcatcatattttctggggagcccaggcacaagtttactgaaggtatctttcctactttgctgatcatgtagctaaagtcaggctgtgtacctaactaaatcggacaaaaaccttccatttattcatctctagtcaatatagacaggctgtcaaccattgtggaagacagtatggcgattcctcaaggatctagaactagaaataccatttgacccagccatcccattactgggtatatacccaatagattataaatcatgctgctataaagacacatgcacacatatgtttattgcggcactattcacaatagcaaagacttggaaccaacccaaatgtccaacaatgacagactggattaagaaaatgtggcacatagacaccatggaatactatgcagccataaaaaaggatgagttcatgtcctttgtagggacatggatgaagctggaaaccatcattctcagcaaactattgcaaggacaaaaaaccaaacaccacatgttctcactcataggtgggaattgaacaatgagaacacttggacacaggaaggggaacatcacacaccagggcctgtcgtggggtagggggagtggggagggatagcattaggagatatacctaatgtaaatgatgagttaatgggtgcagcacaccaacttggcacatgtatacatatgtaacaaacctgcacgttgtacacatgtaccctagaacttaaaggataataataataaaaaaatatatagacaggctggtcccgggtgcctccaggggagttttgaacttgaaagggcatatttatgaatcactagttagcacattacatctctgacttgtccataaggcctggaaataagcatacagctgctccagtcctgctgcaagagaacgtgatcctcataaacatgcttgatgccactgaacctccttaacatggagtgaagatttggaaatcaggaataattgtttctttcaacaattgagacagaaatttgcctccatacttaggaggttaattcttatttatatagaactttaagaaaagagtgtaaaaaaccatttatttttctaatgtaaatatgatatactgtcaataacccagtttttacttttcctgtgagccatatctgaaaaatttagggacattatttatgttgtcttaaattttttggaactagcattttaagaccattacaaaatgtgtagcttaatattaaatattatttatgaataagtaatgtacactatttcagagttgtccgtttatgagctttttttttttctcctttttttttttttaagagacaaggtcttactctgttatccagggtggagtgcagaggcatgatcatagctcactgcagccttgaactcctgggcttaagcaatcctcccaccttagcttcctgagtagctgggactatatgtgtgtgccactatgcccagctaattttttattttttgtagtgacagggtctcaccgtgttgcttaggctggtctcaaactcctggcctcaagtgatcctcctacctcagccttccaaaatgttggggttacaagtgtgagccactgcacccagctgttatgagcttttaattttacaatagcacatttaaaaataatttatctggtgaaagttcttatttactcctgcttgtctcctctaggaataatgccttatgaatcgtgtccttagttgtagatagataacatatatataaacggtgttttatttctcttccagagaccttttgcctgaagattttgtggtttatacttacaacaaggaagggactttaatcactgaccatcccaatatacaggtaatgtatttttctcttgatcccatagcaaattttaaaacaattataatttaaaaatgagttctgtataggcactcaggactgttacattgcacagccccacagggtacctttaacattataacatatgggttatcttgggaaaagtgggtgcatttctatagactaagctgtaccttacagctctccaggtactcagtagttaaggttttttttttaaagactaggaaaataaatcttctatttaatggtaatccttactgatgagaaaatttgatatgttttgaaaataggagtttctgatttttttgttgaaagttaatatctctaaaagtgcacttattaaaacatttaatttgtcagtgatatttagtaaagaaaaacactcatttgatgttatgtgttctaatgttctaaattttttctgaaaataattgtttcctaaaagaggtgtggtcctctctgcatcagagaacagagtactcctggggacagagctggccagaatacccaaaataattggcagatgtcaaatttggctttctgtgtttattactagagcataaacatttctagttttgtttgagtgttttacagtcctttttggcagttaggtattatacctttttttcttttgcaatggttttcatgagaaatctttattcccattacatgtgtatgttttatttttcttctgaactttgtaatactttgctatgttgaattgtttctgttggtagcgcacttttgcagcattcttcaaataggaggcaaaaaaatctttagattaattattagtacttacaaaaaccaaggaaatgctgacttaggcctatcttctggtccactatctgatttctttatcttagtgtgttgttggtccattgtttaatagaaaattagtagaggagtttgaatttaccttacagcataaaccagatagaaaataacgcattcatccagtcatgcatccaatgattaccaaggcagaaggccaaacaccacataatttgtgtcacttgacaaaagcagtaatgttaaaaggcatttttttcctcatagaggtttcttggcatactttcttcagacatacactgtttgggcttgagttttgactcattatttgctgatgaagctactttaatctgtttgtgccttggtatcttcgctttaaaatgtaataatagttaccactttatggatatactgggaaacttaactgagttaatacttacaagatgcttagaacagtctgacaatttttaactcaacgaatgttattatttgttgctattattgacagcgtatgttcttaaaactgccaaaaattgatttaattatatagaaacttatgtaactattatcttatataatacttaagtatcataagtatgatagagttatgcttttctgggtgtttgaaaaatgtcaactaagacagatggtgtctcacttatttcttggttatttaatattgttcagttagatgaaagtgtgattgtagatttgaaatacaaaataaaacttggatactgtgatttttttaacatggccagactgtcatgtattataatgacatatacttttgtccataaaatgaaattaagtttcactgaaaaatttacatactttcccctggggattctattgcttcagattaaagtttataaagtatcattagtgtcttccacagggtcattttacacaaacacagttttagtgagatgtcaactggcttttgttggttgttggattgactgtgatttaaaatgttaaagatgatataatgcatcttgttctgcttctaggctgaaaggtcactgaggcagagctgtttgtaccttgtatcccctggaattttgcctaaacatttgtgtactcatagggtggtaggagatagtccgcagatggtctaaagaatgccatgtgatactgtgagatgccaataatataaataaaactttgttattattaaacttgactggcctaaagtaattttgttagctctgcaatttctgtgatgattttcagcaatgtagcaatatttgaagataatacagtatttttcatttagaatcattgtcattatcggggctatgtggagggagttcataattcatccattgctcttagcgactgttttggactcaggtaagcaatttcctttatcttctttttttttgtttcccctatgtcttaccctctttcctgtttctgtctccaaattaaatcattttgggcacttagcaaaattggaatttactttgatgttactgaacatttttacagctgtgtttcagatatccttggcatgtttatttaagaaagtattatagttgatgagttttaatatgtaaagaggaaattttttttgagaccactaaatcatttttgctatttaaaatgaaatatactttaaatttctgtagcactttatatttataaaattttcacttgtattatttaagacttgtatttaagtcttattatgactgtgaataagagctcattatctctgtatttaggtgagcaaactgaagttcagataaattatattacaattcaaattaagttattatagtattaacattacattccttgaggtcatggcaacatggcactgtgctggttggttgactgcatgattgcttgaactaaaacatattagttctatataagatgaatatgattatattcacttaggcactaacacttatttggtagttactgtgtgccaggcaatatgttccgtgtgttttctgcttattaagtaattttgttttcagaacaatcctgtgcagagtgcaaaccaaggcagaggttaaatacctcgctgagagtcctgcagctagtagaagacatttggaattcagactcttgtcctctggtccggatgccacattcttagccactattttgtagtgccttccatttcccgtagatcactcagggaggttaagtgacttacaggcagtgacgctgctaagtagctatttgagctttcaatttaggtccgtcccagccctatctgtctgattctaaagcctctattttcttctctatgtaatgctatgcctacttacacatttaagaattaggacttgaacttaggttttctgattccttgtgtattttctttttcttaaaatttgtatacgtgtaatgcaacattcagaggattgctgcatttagagaatgcgagttatgggattgaacccctgcagaacagctctcattttgagcacatcatttatcgaatggatgatgtctacaaagagcctctgaaatgtggagtttccaacaaggatatagagaaagaaactgcaaaggatgaagaggaagagcctcccagcatgactcagctacttcgagtaaggaaataacataattcttcatggctcagactaccattttagaaaaatcatgtatttattcatgaaatcaatactatgagtagtgtttttttttcttttcttaattttgccaaatatatgccagacattgtgataggtactaggggatgaaaagatgagcgatatatagttcctgctaccaagttgagtacagtttagatcctgtgggttttggaaactaggacttaaatctgcaacaatgttcactgtggccttgacctcttgagctcaagcaatcctcctgcctcagcatcccagtagctactgctacaggtctgtgccacccaccgtgcctggctaatttaaaacaactttttgtagagatgaggtctcattacattacccaggctggtcttgaacccctggtatcaagcaatcctcctgcctcagcttcccaaagtgctgggattataggcataagccactgcacccagtgcaatagagtttttatttaggtacctcttagacaactcaaatggtgattcttgaaccctagattggaaaaagagagagatacggctttaggaacttaatgacttcagatgtgtttcaaggacactctgctaatgactttaagtgatgataaactatgtctgagtccctctttggagactgctatagcacttcatgatttactcttgacatgggtgtctcttagactgaaatggttctaggactagatcaacttcagctgcagggattgtacctttctacatatgagattctgttgctgccttgaaagaggcatatttttaattaagttatactagtttatggcattatttttattgcctctgctgctatccactcttttgacttgggctattctttttaactttaaacattggaaaacattaaaatttttgcttattctacttcgcatgaatttctgtaaaatgacaaaactagtcattttttaaaatggcaaccttattctaacttctgctctgggatattagtggatatgttttctttatctctcagcatagtaatgggctttttcattaaaatatgtgtgtgtttgcatgtgtgtgtgtgtgtagttttgattttagaaaattggtaattctgctttgtaaacttaaacccattttatctgtaactaacatttttctcatattagtgcagatagcagataacacttcaaaaacatttttttcccctcagacatagtttatcatcacttaaagtcattagcagaactggacaaagttttcatcactaagaagcagataacacttcaaaaaacatatttttcactttcttgatataggatatgttaagtaaaataattttatgatgttcttagcagacatgaaataagtgatgagagattaggatgtgatcatagccttataacttccttttgcctttatgatgtttgtgtttttgacagagaagaagagctgtcttgccacagacccggtatgtggagctgttcattgtcgtagacaaggaaagggtaagattggtgacaatttttcttcttttccatgaaaaggatatgagaagtgagcatttaatgaaggaaatctaaactacacattgtttgtattgattttacttaaataatgattttaaaactaaaatggtttttttcccttaaactttataccaccagaataccaacagaagctaaatgtagcaaatgtgactgcctttaactttatcttttattaatgatttttttttctttttcttgctgatgacttgcttatgctgaattttttgagtgaatctgtactgcctatcaggctcttgagaacttttcagattactttaatgggctgtggctctaaaaggtttggctttgttggctaataaaattgctttgctttctagaatttgagataacctatattgcactttgagagatggaaaacctccaggtcctggcatgctttagaagggaatagtattaatttccgtgtataggatcacatgagggcattttccttatttatacttaagaaactgaactaagtgctttgctttaactaagagaagtaatgtgtccctattttggcatttacaggattatcagttttagagataatggctgtataatttattttcatgttgctttttttattgatatataatacttcacatgtttagggggtacaggtgagtatttgttacaacagctgtgtaatttaaaaaagagagtatttttagtgttttgtttgacttttacttccaactttgttgtcagtgtgaaaaagttatttgtggaaacttactatgattggcagttcctttcttgtaagctgtagagacagttttgaggttttttttggttttaaaaaaattccttgttgtatgtaggttggaaaataacaagccaccccaaataactaatttggagaaaatattaagagatagacttggatttgtacattataggttcattgccctcaagtggcagaaggaaaagcacatggaatatgaacaagtgtgaactctgccccaaacagtgggcaaaaagcttctgtagaagaatgttttggacaagtcacaaaagtcaagattcaaaatgttttccttggctgggcgcagtggctcacgcctgtaatcccagcactttgggaggccgaggcgggcggatcacgagatcaggagattgataccatcctggctaacacggtgaaatcccatctctcctaaaaatacaaaaaattagccgggcgtggtggcgggcgcctgtgatcccagaacccgggaggcggagcttgcagtgagctgagatggcgccactgcactgcagcctgggtgacagagggagacttcatctcaaaaaaacaaaacaaaacaaaacacacacaaaatgttcttcttcattgctgtctccagatgtatttgttatatacagatagaaaatggttaaaaaaaaggttcaatttcaatcaagccctatcaaatatattaaattaattttttttcttgtttaggaggatcatgattagatccctaactgataaaatctgatatattctgatactaatgcttttagcatagagcaaaatcataaatccttttaaaatttttcttctgctaaattggttatataaattaatgttaaaaatagacatttcagtttagccaggtgtcaaagaaaaattagtcatatttatttggcttaagatggttaaacttttatatattttcatctacatatgattttttaactagtgattattggttaatctctcatttttaattcagcccagcatttagaaatggtttattggtgctgatctgtaaccaatctggctgtttctgtctcagttctattttctgtatgtcacttcgtttttctgtccataaatcttcttccactatgtggctgcacagagtctctctgaacctgttctggtttggaagccacacaattcttgaatcagtcattctttgctcaactaaattctgttaaattaaaaaaaaaaaaagtttattgattacatcattagcttaagaggtgaaagggtcaggaagttctttagattgtcttttattcttttatctatgcattttgattgcttaaaactctacctttgtgaaatgcttgaaaatatttttgcattaaaataaaaggaacattaagaagataattcgttttaaagttctactaatttggataaaatgaagtcttcagtgctctttcattattattcactttacccttttacctgtttttcttttattcctgtcactacaatgtaacctttaaatttcttaatttgaaatgttgataaatgtctaaatgcctcaattttttgttcagaggaaatatttggattcttcatagtaacagacacatttttattttatttttattttttttgagatggagttttgctctttctcccagactggagtgaaatggcgggatcttggctcactgcaacttccacccccacgggttcaagcgattctcctgcctcagtctcctgagtagctgggattataggcacctgccaccacgcctggctaatttttgtatttttagtagagagaaggtttcgccatgttggctaggctggtctcgaactcctgacctcaggtgatctacccgcctgggcctctcaaaatgctagaattacaggcatgaggtactgcacccggccttacatttctattcttaaagtactttggtgataatgattctccttctttgcttttccagtatgacatgatgggaagaaatcagactgctgtgagagaagagatgattctcctggcaaactacttggatagtgtaagttgtattttctatcaaccaggatgattctgtcctattctttcagtcccagaacagaacttaaaaatgtctcattttgagttctgattttcatagggcctcaatgacttagtctttcagaggtctgctttctggtttgttttgtaactctttttaatgtttaaaggaaagtaccagtgtagaaagactgagaagagcaagagatttcatattagcatctactttatcttcagagttgctaggcttaggtgctttggcatttatggaaagatctttgaatttttgtcgaatgcatcttattttgaataaggctgccttctaccctgaaaacatgatatgacaatatttgtgtgtgtgtgtgtgtgtgtgtgtgtgtgtgtgagagagagagagagagagagagaaagagagtgtttggtttgagattttggagttcatccggtgggagatattaaagaattagatatatgttcttataattttatctacaaagctgatatgaacattaaacgtgatgatgacgatgatgatgatagcattcacttgagtacttacagtgtgctagacactgagctaagtgctttacatttattaacccatttactccttacagtacccctatgaaattatgagttccacagtcctttatctgaaacctctgatgtacctgtgattaaaattttagataagtttagaaaaacagtgtgattaactctgtattatataacaccttcgacaggatcttggggtagcacctcataatcagactcattgatatttctgcagtgaaatataggaatatttacattaaataggttaaatgtggactatgaatgggcttgcattatatcagggcaaattttggagccagttttaccaaaaacttaatttccagagtttgtcagattttagaatagaagataataaggatttcgaatctctgttactattattttatggttgaggaaactgagactattgagaggttaaagttttattgtatttttttttttatgagatgagtctcgctctgttgcccaggctggagtccagtggcgcaatctcggctcactgcagactctgcctcccaggttcaagcgattctcctgcctcagcctcccaagtagctgggtttacaggtgtgcaccaccacgcccagctaatttttgtattttagtagagacgggatttcaccatattggccaggttggtctccaactcctgatctccggtgatccaactgcctcggcctcccaaagtgttaagattacaggcgtgagccactgcgccccgcccaaagtctcattgtattaaaggaaagatagttttttttaggcaggggagttttaatttaagtagccgtgttacttcatgtggttaaaagatttttctcacgttctttactatattttatatacttttatttctttcttcccagatgtatattatgttaaatattcgaattgtgctagttggactggagatttggaccaatggaaacctgatcaacatagttgggggtgctggtgatgtgctggggaacttcgtgcagtggcgggaaaagtttcttatcacacgtcggagacatgacagtgcacagctagttctgtaagtattttttttttaagtactattaatgaaataatcaaaataataatttttgcttattttcttgtattagaattatattctcttgaggttttggggtattcatttaaatgaggaaaacttagcttgatgtggcattatcatgagacctcttctgttttggattcctgtgacctttctcccatatcctccttttttcttgagtttacatcctcatttgggtatagtgtgctttgtactagttttttgtgaacggatatatagaaagaaaacattttgacctcctgtgtgtctgaaaatatggtttcccagtttcggaacagaattgaaaaattatctcaatttgagttctgattactctaggcctaagtaactcagtatttcctaggcatgctttgagtttcttttgcgtttgtttttttttttttttttttttttggagacagagtctcactctgttgcccagaccagagtgcagtggcacgatcttggctcactgcagcctctgcctcccaggtcgaagcaattctcctgcctcagcctcccgactagctgggattacaggtgcctgcccccacacctggctaatttttgtagtgtagcagagatggggtctcaccatgttggccaggctggtctcgaactcctgacctcaggtgatccacctgttttggcctcccacagtgctgggattataggcgtgacactgggtataaaattgtatccgtgaaatcctttttcttcacgactttgaaggcgttgctcttttgtcttttttgtcccagcattactattgggaagtctgaaacattctgattcctgaccttttgtatgtggcctgtttttccccgtcactggaaacttgtaggatcttctcttggttcccaggcttctgaattttcctgatgatgtgttttggtgtgggtcttaatttttagtaaaatcgtacgctcacacatcctcgtaccagtgagaatgccatctagttcacaaaataccataaggagcaggtgtcaagcatactcactatgccttgcccaaccacacccaccaaactatcttaaccccctctctttgtgtggtctccatctgtcctgttagagacatttcccagatgcttgatgatttttagttgtttgtttacagttgagaatggggtcccgaaaacctttttggaagccttgagtccatgagtgcattttggggcctatgagttccttatagggtggtttggctggaatgtccttgtcaatctccttatgtcagtacctctggtcatcttctcctggctggtcagatggcccagagaaggatttatccattcatttaaaatatatttattgggtgtataccccagacactgggacatagcagtgaacaaaactggcaaaaattcctgctctcatggagtccatgttctggtggaggagattggctatacatgtgataaataagtacatgtagtatgttaaccaatgataagtggtaaggagaaaaataaaacgggagggtagatataaaagcattggaggttgtgattaaaattttagataaaagtttagaaaaacagtgttattcactgttgaattttgaggtgacatggtctagccagggagatgccttctgagtaaagacctgaaggaggtgagggaatgagtctgggttatattaatattagggaagagaggtccaggcggagggaacaggtgctgaggtacaggtgtgtggggtgtgactggggaggcacacagggcccatcctgaattcttttttttttattttggagacagagtctcattctatcacccaggctggagtgcagcggtgcagtcttggctcactgtggcctccgcctcccaggttcaaatgattcttctgcctcagcctcccgagttgctaggattacagatgtgcgccaccatggctggctaattttcgtatttgtttttttagtagagatggggtttcatgatgttggccaggcttgtctcaaactcctgacctcaggtgatctgcccacctcggcctcccaaagtactgggattacaggcatgagccaccacgtctggcccatccttactcctcatgttcaccctgctcactgccctgcagctgcccgtgtaaacatattcatttcattcgttatctgtctctcctcactaaaatgtgtattttaatatatagttaaatataataagtgtataaataaacctaatgtattttaggagaggtttcacctagaaggtaaaaagaaacaaacttgtctcggtatccagaaagtgtcttcatttgtctgaaaaaattaataagaaggagataaggcataagtatattctgattttagaattttttttttttgccattttcctgccatgttttgtaggttctcccaatccagttgagattattcataaaataaaagcaatgtgttccttttttccccaagaacattttttaacttttacattttcatttagaaagaaaggttttggtggaactgcaggaatggcatttgtgggaacagtgtgttcaaggagccacgcaggcgggattaatgtggtacgttgttcttgatgtttaactttggatgtttgcactgggacaatatcaagcatttattgactgtatacttcctcccctggtccttaaaacaatattttgggtgttatgaggaacacagtagaagtcgcagatgggttctttccccagagactgggtcaagtttttaaatatgtgctatgtgtttattagctcttttcttttttattcattttattttactttaagttctgggacacatgtgcagaatgtccaggtttgttacataggtatacatgtgccatggtggtttgctgcacctatcaacccgtcatctaggttttaagccccgcatatgttaggtatttgtcctaatgctctccctccccttgctccccacctcccgacaggccccggtgtgtgatgttcccctccctgtgtccatgtgttctcattgttcaactcccacttatgagtgtagctctttactttttatgggtgaggaaacatgtactccattttagagaattaaattagaaccattaacttgttttcctataaactaccataagtaatctgttggtgctaaagtggttgacctcttgcttgaaggatccatgtccatcacgtgtgtgattcatgttactttcttactagactgaaatgtataaagactgttgttggatgcttgatttatcacgtaggctgtcaacagtgtagtgaataaatttccttttgtgaaaaaataatctgagcagcaaaacattttctttgcgttcagaaacctaattactaccttcctgttctgaacagtttggacaaatcactgtggagacatttgcttccattgttgctcatgaattgggtcataatcttggaatgaatcacgatgatgggagagattgttcctgtggagcaaagagctgcatcatgaattcaggagcatcgtgagtacctgggttcttcttctcctttatttggtattgtagatccatgtttcttacactgtgagggatattcatgtctacattgggaaaacaggaaatgttatttccggtttgctgaaattaattgcatgacataccaatgagaagtctttttttttttttttccagccttttagatttagggggtacatgtggagtttgttacctgatgtattgctgaagtctattttttaattaaatgattccagagagctttaagaaggcaatacttatgtaggcacaagtatgtaactacactcttctgtaaaccagttatagactgaaagtataagaacatggcaaagtttattatctgaattagaaattaagagggagtttctgctaggttcagtgtggattggattacactgaaggactgcataagaagtttcttcacaaacctctttttgagaaagtgctgcattgtcactgtaggtagaagagatcctgatatatttctattaacaaaccctgttttatagagataaaggtgggaggcaagacagagaagaggagagagaatggttaacatttgttaagctctttttatgtacaggcactattgtagccatttaaaacgtatccactcacttactactcatcagtgaaatgaggtgcacatactttatctccatttgcagatgaggaaactgaggtcacacatccaaattgctgactgggattcaaagtcaggaagtcaaagcctgtgatctgagaaccctttcctgtcccagagctaaaaaataattataatagaagatcccatggtggttgggcatcagaaatatagatttctaatgcagattcgttgtaatgccaacgaggttccttcctaatttagaaggcaggagtcctaagcagagagctgaatgtaactgtagttcgtacgtgtgtagatgttgagcctgagtgaaaattagatatgagaggtgatatctttaacaaatacaggacggacctggtggctcatgcctataatctcagcaattagggaggattgcttgagaccaggagttcaagaccaacctgggcaacacggtgagaccctgtctctaaaaaaaaataaataaataaataaaaaataaaatattaactgggtgtgttggtgcgtgcctgtagtcccagctactcaggaggttgaggcaggaggatcacttgagcccaggagttcaaggctgcagtgagctatgattgtgccactgcactccagcctgggcaacagagcaagaccctgtttcaaaacaaacacagatgaagatttcacatggggaatatccgtggccccaagtgttcatgccacttcccacctccctcaggctcctgaagcactgacagagtaataaaaacttctgtcaaccagcctttcagctgaagttctgagtggacaagacaatttcaatcacatgctagtataaagggaagcactcaagcagaatttacagtttttgaacaaatactaggctcaaaaatagatatggaagagttaaaatagtacttacaaaaagccatgcttcataaaaaaaaaattaggtatgtaaggaacgtcatatgtttgtaaaagatttcctgtaggagagggaagtaaatttaggatttgctttggccagcagtgaagttgagaaagacgtgagttcagggaaacaagaaatgtgtaatgagcaatgagataagtcatagattaaaataaaaaagaagcattcagaggtaaggagggaatgttatgaaacagtgccatagtggaatttaatatggtataggaagcaatgaagagtggacccatactttattcaccaacttgtcaaacatttattgagcactgaccacctgccagactttgttctcagcacttggaatacctcagtgagttagatcgactcacccttcaaggagtttacatctggggggaagacaatctataaacataagaaaatcaataatatagagtgttagaaggcgataagtgctatgggaaataaaatagagcagaatgtggaggattgggaggacggagggtggtgaaacaacagaacaggcttcagtatgacaaaactggatgttaataacagaaacctgagtgagttggtatttaaaaccactcccctaaagtcaaccctgtgtcaagcagacttacagtatacttaaaatattttgaggagaatggtatttttgaatattatatttaaaacagtgcatattgacgtttaaatatgaagataacatgatttcaaatttaaggtatccatcattttcccaagggaagagccaaaaaagtgttgttgttgtttttttttttttttggttgacttgaatgtgtataaacttgctagggatacagtagatagaaagggagtgaactgttcattactggatcttggagagtctctgtagccacaggggagactgaccccataggagttgaggtagagggacactgataacatgaggatactgataacatgaggtagagggacactgataacactgataacatgaggtagagggacactgataacactgataatagagagggttccaggtgaattattcagccttattctcccagtgacttcttatctcttgaatagaagtggccaaagtgagtacctatgtcttgtccagcttagtgggaaagcttttgatttttcactgtggagtatgatgttgtctgtgggcttttcatatatggcctttattatattgaagtgatttccctcttcctagtttgttgagatcttttgttgtgaaagaatgttgaattttatcaaatgcctttttggcacctgttgagatgattatgtgactttgatccttgattctgttaacgtggtgttaatacatttttgtgtgttgaaccgtccttgtgtcccaggtacaaatctcatttggtcggagggcctgatgtttctggtgtgttgttgagttctgtttgctagtatttgttttgaggatttttacatttatgttgctagggatattgacttacaattttcttttctggttgtcccttgtctgactttgatattagggtgatgctgggctcataaaatgagtttggaagtgttccttcctcttcaatattttgagaagacttttttttcttttaagcagttttaggttcacagaataatcaagaggaaagtagaaagactcctcccatatactttctgtccccacacttgcatagtctctccatttcaatatccctcaacagagtggtatggttgttaaaactgacaaacctatattgacacatcatgatttctcaaagtccatactttatggttcagtcttggtgttgtgcattctatgggtatgaacaagtgtatgatgacaagtatccctcattatggtatcatgcagagtatttccattgccttaaaaaatcctctgtgctccacctagtcatctctccccacccctccaacccttggcaaccactaatctttttactgtctccatagtttcgtgttttccagaatatcatatatttagaatcatgcagtatgttgccttttcatattggcttctttcacttagcaatatgcatttaaggctcctcatgtcttttcatgtcttgatagctcatttatttgtagtgctgaataataacccattgtttggatgtaccacagtttaaccatttacctactgaaggacatattggttgcttctaagctttggcaattatgaaaaaagctgccataagtgtccgtgtgcagggttttgtgtgatcatgttttcagctcctttgggtgaataccaagggatgcgattgctggatcatatgttaagagagtatgtttagttttgtaagaaactgccaaattgtcttccaaagtagctataccattttgtattcccaccaacagtgaatgagaattgctgttgctctacatctttgtcagaatttggtgttgtcagtgttctggattttggccattcctataggcatgtagtggtatctcattgtttcaatttacatttccctgatgacataggatgtagatgatctttttccttctttatgtcttctttgtggcatctgtgaaggtctttggcccattgtttaatcagattgtttcttttcttattttttagttttaagagttgcttgcatactttggataagagtcttttatcaaatatgtcttttgcaaatattttctactagtctgcagcttatcttctcattcttttaatattgtctttcacagagcatacatttaatattttaattctttcatggacgatgccttttgtgttgtatctaaaaaataattgccatatccaagatgatctaggttttctcccatgttatctcccaggagttttagagttttgaattttacacttagacctttgatccacatggagttaattgtggaggatgtaagatctgtgtctagatttatttatttattttttgcatatgaatatctaattgtagcagcaccatttgttgaaaagattatcttttattgtattgcctttgctcctttgtcagagatcagttagctgtatttatgtaggactctttttgggctctctatcttgttctctttatctatctgtcaccttttgctaataacacagtcttgaagcttgtgcatgcgtcacatagttctcgtgccatggttttcagctccatcaggccatttaaggtcctttctaccctgtttattctagttagccatttgtctaatcttttttcaaagtttttagcttccttgcgatgggttcgaatatcctcctttagcttggagaagtttgttattaccaaccttctaaagcctatttctgtcagcctgtcaaagtcattctctgtccagctttgttccgttgctggcgaggagctgtgatcctttggaggagaaggggcgctctgatttttagaattttcagcttttctgctctggtttctccccatctttgtggttttatctacctttggtctttgatgctgatgacctacagatggggttttggtgtggatgtcctttttgttgatgttgatgctattcctttctgtttgttggttttccttctgacagtcaggtccctcagctgcagatctgttggagtttgctggaggtccactccagaccctttttgcctgggtattaccagtggaggctgcagaacagcaaatattgcagaacagcaaatattgctgcctgatccttcctctggaagcctcatcccagaggggcacccgcctgtgtgaggtgtcattggcccctactgggaagtgtctcccagttaggctacatgggtgtcagggacccacttgaggaggcagtctgtctgttctcagagctcaaacactgtgctaggagaaccactgctctcttcagagctgtcagacagggacgtttaaatctgcagaagattctcttgccttttgtttagctatgccctgccccaagaggtgggatctacagaggcagcaggccttgcagagctgtggtgggctccgcccagttgagcttccctggctgctttgtttacctactcaagcctcagcaatggcagacgcccctccccctgccaggctgctgcctcacaggtcaatctgcctgctgccctagcagtgagcaaagctctgtgggcgtaggacccgccgagccaggcgtgggatgtaatctcctggtgtgctgtttgctaagaccattggaaaagcacagtatttgggtggggttgtcccaattttccaggtacagtctgtcacggcttcccttggctaggagagggaaatcccctgacctcttgtgcttcctgggtgaggcgatgccccgccctgctttggctcaccctctgtggactacacccactgtccaaccagtcccaatgagatgaaccaggtacctcagttggaaatgcagaaatcaccatcttctgcgtctgttacactgggagctgcagaccggagctgttcctattcggccatcttggaatggccacacggtcttgattactgcagctttagagtaagtcttgaagtcaggtagcaccagtcctccaactttgttcttcttctttactattatattggctattctgggtcttttgccaccccatgtaaactttaaaatcagttttatctatatccacaaactaatttgctgggattttgattaggatcgcattgaatgtatagatcaagttggggaactgacatcttaatattgagtctgcctgtatgtgagcatgaaatatctctccatttatttagttctttgattctttcatcagatagtgttatagtttccccatagagatcttatacatattttgttagatttatacctaactctcatttttgggggtcctaatgtacatgatattatgtttttaatttcaaattctacttgttcattgctggcatataggaaagtaattgacttttgtatattaaccctgtatcctataaccttactgtaattgctttttagttccaggagtctttttcaattctttttgattttctacatagatgatcatattatctctgtacaaagacagtttttctttctttccagtcagtataccttttactttgttttcttttctcactgcagtagctaggactaccaatctgatattgctttaccttcctcacattttttttttagcattgacagtgtgtttttttttatttttaatagttatgcttctaaaacatatttaaattttatttttaatccaaattgaaaatatatgtcttataattatatcacttaatatatttatatttactgtaattactgatccatttaatcaaatctaaatgccattgattataagatacaccactttttccataccactgagaaagaaatatggtgtcaatgaaattaatacgtcaattgtaatctgaaatgaatctcagtttcaaagttatttaaatatggaaagaatgtgttttagaatcaattaaatacagcatttgggtttaaatctaccatcttatatctcctttatttgtcttcttttatggtttttttcttaaaagttttcggtcttaaatatttaagttgatggatgttccaattaccctgatttggtctttacacattgtatgaatggatcaagtgatcacatgtatcctgagaatatatacatctattgtgtatcagttaaaaatgggacgacaacaacaacaacaaaatcttctgtgttatttcttttgggttggtagagtgtttttatatttattttcactttgtagaaatgggttcttgttatgttgcccaggctggttttgaactcctaggcctaagcaatcctcccaccttagcctcctgatgtgctgggattacaggtgtgagccactgtgcactgccagatagagtgtttttagtagatactgtttttcttctagacatatttctagaatggaaattatgcagtcttttattttttttaaagttaccctagaaattattacacatgttcttatttatcatgtctactattaaatcttatccttccccacacagttcaaaggctatatcgtgccttaactccattcatcactttcttgactcatatagctgtgtgccaggaagatattagtgattgtttatcattattcatttagattttgaccactgcccttgctctttggtcctcttgcatctctgaccttccatttggtatccatttttcagtctgatcaaagaaccagttttgactttcctttaatgtgtttttagtagtagtgtatctcttagtttttgtttttgtttttctcctgagggtgtctttgtttctgttttttgaggatatttttgttgaatatagaatcgtagatcatcagttatttttcatcatattgggatttttccattgtcttttgctttccatgttgttgttgagatgtcaaggtgtcagaccattattccattgaaatgaatctgtctatttacctatggctgttttcacaattttgtctttaaacttttttttttgacgtttcattatcatgttcctgttgtagaaagaaaaaaatatacaacatgcatacatacgtatgttatgtatatataacacatttacacatatatgtcttcatatcctgcttagaaattttttagtgttttaaagtttgtggcttgatatttttcatcagtcggaaaattctcagtcatgtctttacatattgcctgtgtacacagggtgtctgcacatttgctgtctctcttacgcctctgtgattctagtgaactgtgtgttagacctcactatgtctcctttgtctcttagttttttaaatatgtttcctatctttttgtgtttttttcttctgtgtaatttcttctgatatctttcagctcactgattctgtcttcatatgtattttgtctgttgttaaacttatccattgaattattaattttgcttatttcatttgtcaaatttatgtctggttctttttcaaatctgatatattagttttgtagattttagtttcctgcccaaattttcatgcttgtcacttttgtctctgatcatagtaagcataaatgtcttatggctatcatttgataatcctagaactagtattaggagtctttattggactttatctgctcgtttttttctttcttgtagtgtattgtggcttcatgtggtattttatattgtgtagctgttatatttaaaattttttttaagaataatttctagaccgggtgcggtggctcacgcctgtaatcctagcactttgggaggctgaggcaggtggatcacgaggtcaggagatcgagaccatcctggctaatacgtgaaaccccgtctctgctaaaaatacaaaacattagccgggcatggtggcgggcgcctgtagtcccagctactgaggaggctgaggcaggcgaatggcatgaacccgggaggcagagcttgcagtgagctgagatcgtgccactgcattccagcctgggtgacagagcgagactctgtctcaaaacaaaacaaaacaaaacaaaacaaaaaaaagaataatttctgaactaggatgaggttatcctaggtaatacatatttttttctcttatttttcctcagattcctttttactaccaagctgatattaaactttctttttttgagggcatatttcctaccctctacttcataggctgtttaataaatgttaattttctatcattttgtttggcttttttttttagatgctagtgatgtacatgtttcattttttccccctcagataactcagtcattgggagccagttccatttaataaaatggataatctaccctcgtaataagatttttttgttattgtttatgatattttgggggcacagtggtattcttatgcattgctgttagattctggaaagtgtgagttgctcttcctgggaggtgcctttctagaaaaatggctttcttaactctgcccctcaatgtcagcaagcttccatcagcaagcttccataatcaggtgtttttttcttaatctaattcagtaccagcacttagaatcttctcttaagacttcctaatcctaggctgtgggaatcagcatagtaatggtgaaaattgtgttctgggaattttcagaggactcaaataaatatgttttgaatgatagttgaaatttttttttttgtcatttccatgtaaaacattttcattattgtcgatctccttttgaagccattttgggaaaatcacctagatgtgagaaaagagaggaggagaggctataaatcattaatattgtagagtctagaggtgatagagagtagaaatacttgagttgctcttcaagccccgtatcaggagaaagatcattctttttgttgccataggtgccagccagtgatggctagtggaagggtattttcactgtagcctctaaagcattttaaagtctcactgaaggccaacacaggggatgttgttactatctcccatctgttaaaaagcaccacaagtgtctatgattttgttatgctttttagttctatagtcaattcatgtgggtgaatttttttttttttttggtagattgctgaaggatcaagcatttgaaacattgtttataagaaaatatccttcaactaccagataatgagcttatttaaaaaataacttgtttagaggtggtagactttatgtaggttgaaattagggactaaaatataggactatacatatgcctgcgcaagttcttttttttttttttttttttttttgagacggagtctcgctctgtcacccaggctggagtgcagtggcgcagtctcggctcactgcaagctctgcctcccgggttcacgccattctcctgcctcagcctctctgagtagctgggactacaggcgcccgccactgcgcccggctaattttttttttttatttttagtagagacggggtttcaccgtggtctcgatctcctgacctcgtgatccacccgcctcggcctcccaaagtgctgggattacaagcgtaagccaccacgcccggcctgcctgcgcaagttctatggccattgtctaattaaatatatgtaatttataaatatatatttatgtagtatatatatttaaatatatatttaagtgtgtgtgtgtgtgtgttttttttttttttttggagacagggtctctggagagcagtggcttgatcatagctcactgcagccttaaactcctcccaccccagcctcctgagtagctgggactacaggtgtgcaccaccatgcccagcttattttttgtagagacagggtctcattatgttgcccaggtggccttgaattcctgggctcaagtgatcctcttgccttagcttcccaaagcattgggattacattattaaatatattcctacagaaaacattattgcatgtataccatgtagcaggcgctgtgcttaccacataaagatcaacagtacaaaataaaaaacaattacaagcctctgtttaaactgcagtcttctttgtttatcaaataattattttatactgctttgacatttttacttgatgtctaataggctcaaactcctgtgatccctcctaaagttgtcctaaaatgtgatctacccatagtcttccccatgtgaattaatggtaactccttccttctagtatcccaggacaacaacctgggagtcattcttgatttctcttttttctcactcttcatcttaatggctgttcctttaaaacaaaagcaatccaaccacttcttacagctcccactgtttcattttggtccatcatcatctgtttggtggatttctctaagagccttctttgtagtcttcctcttaatagaacaagtatggtgatcctattaaaacattagtcaaatcacattactcctgcacttttcatggtcttccccttccaacttccccattccacttagagtagaaagccacattcctacaatggcctattcctgtctttgctgactgtatctctcatgactcatttcctcactgactcagtctgccaggaaagcttctaccccagagtttttgcatttgctattccttctttctatagtgttttcctcccagatacacagttttgattgaactgtcacatatttgaggtgcctgtcctgactgcccttttaaaatcacaagcatcccttcctctgcagagctcatcacacccacaccccgtcgccttttttccccatagcacttattaccttataatatgctatctaatttattatataagtaaatcactgaatcataatcataacctttacatgggcagggatttttgtctgctatgttcacagtttcatcccttgcaccaagaagaatgccttgtacataatagatattcagtaaatatttgttgagtgagtggttgattgatattgcacaaaaggactcctccccacaatattcttagtagcaagaaaaagaataaggaagacaagtctttctgttattgacaaaagccttgtgctaaatgttttctttccgtgagtcagaattttgtctttgcctattcttttgtctcaaaccattgatagtttatgttctttcttttttctttctctgccagtcttttaaaatccttccacgtcctacatctagatactttttttgttttttttggtcaaacagcagttaacagtaccaaaatgttctaggcagactgcattccaatccaagaggcaggagtcagtactatcaacttttctagagaccagttagcaaagaagagtttaacatgactactcagggcaaaaaatatgtttcttagagttccttggatatacaaaagaccaagctatagatagggctgcttcttcattaactagaatgcaacatagctttcactcctgctgctacttctggtaccattgctcaaactgatgaaaagagattcagggtaccaaattcccttgaaaaaatacaaatatatgtaagatataaattttattgtatttaagatgtacaacatgttttgatgtaaatataggtggtgaaatggttagtcaagcagattaacacatccatcattccacattgttgcccattttttgtgtgtgtggcaaagagcacctataatctcttttagcaaaaatcttgaatgtaatacaatattattatctatagtcctcatgctgtacctgagatctctagacttgtttgtcttacatatctgctactttgtatcagacctacatgtcccatttcctccacctccaccataatcagtgttttattttctgtctctggattttccacttctttttttagattccaaaataagtgagatcatgcaacatttttctttttctgtctggcttgcttcacgcagcataacatcctccaggttcctccatgttgtggtaaatgtcaggatctccttttataaggatgaataattaccagtcttatatgtgccacagttttgtccattcaactgttgacactttgtttgtttccatatcttggctaatgctgcactgaaaatgggataatacagacgtctttatgaggtggtgttttcattttctttgggtgtatacccaaaagtgagattgctgggtcatatgatagttctgtttttaatttctttagggaactcctattgttttccacagtggctgcaccaatctacattcccaccaacagtgctcaagattcctttttttctatactctcactagcacttgtcatctcttttatttatttatttatttatttgagacagagtctctctctgttgcccaagctggagtgcagtggtgcaatctcggctcactacaacctctgcctcccaggttcaagcgattctcctacctcagcctcccaagtagctgagattacagacgtgcaccaccacacctggctaatttttgtattttagtagagacggggttttaccatgttggccaggctggtctggaactcctgacctcaagcgatccgcccgcctcagcctcccaaagtgctgggattacagcggtgagccaccatacctggccgttatctctttttgatggtagtcatcctaacaagggtgaggtggtatttcattgtggttttgatttgcacttccttgatgattaatgatattgagcatcttttcatgcacctgttggccatttttatgtcatctttggagaaatgtctatttaagtcttttgttcattttaaaaatcgagttatttgtttttctactatggagttgtgtgagttttaaaaaatatattttggatataagatacatggttataagatacaccttataagatatgtggtttgcagatattttctcccaatctgcagacttttcattttgttggttgttatctttgctgtgcagagctttttagtttgatagctatagtaatcaaaacagcatggtagtggtataaaaacagacacgtagaccgatggaacggaatagagagcccagaaacaaatccaaacatgtgtagtcaattaatttttgacaagggcaccaggaggatacaatggggaaaggatagttctcttcaataaatggttctggggtaactggatttctacatgcaaaagaatgaaattggacccttatcatacaccatacacaaaaatcaactcaaaatggataaaatacctaaatgtcagacttgaaactgtaaaactttctaagaagaaaacgttgaggaaaagctccttgacattggccttaacaatgatttttggatatcacaccaaaaactcagtctacaaaagcaaaaataaaatagaattttaatgtgacatggattcctcaaagatataggtgatgtataggtgtaatttccactagttttcaaaggtaaaaatagccagtgggactacctgaaagtattttatagttattgagtaaagtagtagctaaaaaaaaaatcccaggtagaacatatcaaaattgcatttatataaatctcacatagctcaagttggacatttcttaaaggccaactaactttcaaagtactaaccacggttcccaggaattatcataaaatttattatatgtaaagctcaagttgaaaacttgtcatataggagtagctgaaattctacactgtgcagtctgccttttgatggctagtgtgcatctgaactggagttgcccatttgcattatttttgcagagctcctaataagtggtaatgggcatgggtgaacataaaaatgttatccttcagagtagaaaaaagattggagacaacgtacagctaccttccaatatttgaagaacctttactgtgttagataaataaaactttattctcataggactaaataatttttaaagtctcttctgatgctgagaattatcattttgtatttcaatgtaagtgatatgttttaaagatattttattggaagtacaatatattgtaagaaaagtgaattattatatagtagctgaagtaatgttcaatatttatcacaagtagatatgaattctcatttctgtccacttttattagcttcttttctgtcatttaaaatattcacattttgtgggttaaagtcatgacttaacattttcaaagtgagtaatcactgtgacatagatctttttcttaatgtttattataggggttccagaaactttagcagttgcagtgcagaggactttgagaagttaactttaaataaaggaggaaactgccttcttaatattccaaagcctgatgaagcctatagtgctccctcctgtggtaataagttggtggacgctggggaagagtgtgactgtggtactccaaaggtcagtttaatttttgacttttgccttgtaaaattgccatgatatttgcaagaaataaaatggcttgctttgggcaactctgacataggagctaaagtaaaatttagtggcacagtgaggattgttattttgtttgtatggctgtgttccagggattggtcatctccttcttctcagagtatgactaacggtgccatctgttttgaagtcagggaatgtgccatgtttattctctacttttttaatgctattttctatgatttatggttattagcttatttgctttaaagaatgaatttcacctggctctttatttgtaagctttcaccattctggcactgccattgcaggaatatttatttagctggactcattttaaaaatgaattggagctggcctgtcctccagcgtccttcagtattcaaagttcttgctactcaaagtagcactctaaaaaaaaaaaaattcaagtagtaagtaaaagcaaccttacacacgtttatttcccccataaatcttttacttcctttttttatgtttgatgtttttctttttagactattctgttcatttatatacagtatacagtaggtacatttataaatattgggcttgttttaggatttatttttactttaatgtggtaagaatacttagcatgaaattgatccttctaagagatttttaaatgtccagtacagtattgttaactctgggtactgtgttgtacagcacatctctagaactttttcactgtgtgtaactgaaactttgtatctgttgatcggcagctccccattttccattccacaagcccctgaccaccactattctgttcactgcttttatgaacttgactattttagatacctaatataagtggaatcaaatggtattatgtcctttgtggctgccttatttctcttagcatggtattgtatactcaagtttcatctacgttattgcaatgacaagatttccttcttttttgggaaatagtattccattgtatgtgtgtatatgtatgtatgtatgtacattttctttatccattcaactgttgacagacatttaggtggtttctacatcttggctactgtgaataatgctgcagtgaacataggaatgctaatatctcttcaagatcttgattttattttagataagtacccagaagtgggattgctagatcacatggtagttatatttttaatttttaaaagaaccttcgtactattttccatagtggctgcaccattttgcattcttcccaacagtgcacaagggttccagtttctccacattcttgccgacacttgttgtcttttgtttttttccgtgatagcaatcctaacaggtatgaaattatatttcattgtgattttgatttgcatttccatgatgatgagtgacattgagcatcttttcatatacctgttggctatttgtgtgtcttcatggagcaatgtctattaagtctcaggcctgttttaattatttttttgtttcttttaacatttttatatatttaggggatgtaaatgcagatttcttgcatgtatatattgcatattggtaaagtgagggcttttcatgtacctgtcattcaaatagtgaacattgtacccaaaaggtaatttttcagccctcacacccctcccatgctcccactttttggggtctccagtgtctgttattccactctgtacatccatgaatactgattgcttagctcccacttataagtgagaacatgcagtatttgactttctgcttctgagttacttcaattaggaaaattaacccattttaaatcaggttattagtttttcattttttgctattgagctgtagctcttcctgtatattttgaaagtttaccccttatggtttgcagatatttccccctattccataacttggcttttcactctgttgattgcttcctatgctgtgtagaaggtttttagtttgatatagccccacttgtctatttttggcttctgttgcctgtaattttggcatcatatccatgaaatcattgccaagaccaatgtcatgaagcttttcctctatgttttcttctaagagttttactgtttcaggccttatgtttaagtctttaatccattttaagttgatttttgtgtatggcgtaagataaggttccaatttcattcttttgcatgttgatatccagttttccacgggggaagggactaccttttcaccattctttttcttagcatccttgttgaagatcaggtgatctcatatgtgtgggtttttatttctgcattctttattctgttccattggtctatatgtctgaattttattttattttagattcagggggtacatatgtatgtttgttacatgggtatattgtatcctggtggggattgggcttctggtgtacccattacccaaacaatgaacattgtaccttataaataatttgtcagccctcactctcctcctaccctctccagccctcactctcctcctaccctctcctcttttggagttacccagtgtccatcacctccatctttatgtccatgtgcgcgcattgtttagcccatgcttataagtgagaatatgcagtgtttgattttgtgtttctgagttagttcacttaggataatggcctccagctccatccatgttgctgcagaggacatgatttcattcttttttatggctacatatagtattccgtggggtgtgtgtatgtgtgtgtgtgtatacatacatatatatgtatatatatgtgtgtgcacacatacatatgtatgtatatatgtgtgtgcacacatacctatgtatgtgtatatgtgtgtgcacacatacctatgtatgtgtatatgtgtgtgcacacatacctatgtatgtgtatgtgtgtgtgcatacatacatatgtatgtgtatgtgtgtgtgcatacatacatatgtgtgtgtgcatacatacatatgtgtgtgtgcatacatacatatgtgtgtgtgcatacatacatatatgtgtatatatgtgtatacatacatatatgtgtatatatgtgtatacatacatatatgtgtatatatgtgtatacatacatatatgtgtatatatgtgtatacatacatatatgtgtatatatgtgtatacatacatatgtatatgtgtgtgtacacctatacatgtgtgtgtacacctatacatgtgtgtgtacacctatacatgtgtgtacatacatataggtgtgtgtacatacacctataggtgtgtgtacacacacctatatgtgcgcgtgtgtacacacacctatatgtgcgcgtgtgtacacacacctatatgtgcgtgtgtgtacacacacctatatgtgcgtgtgtatacatatgtgtgtgtacatacatatatatgtgcatatgtgtgtatatatgtgtgtgtgtatatgtgtgtgtgtgtatatatatatatatataaaagatttttctcatccagtcgactgttgatggacacttacattagtttcatgactttggtattgtgaatagtgctgcaatgagcatatgagtgcagataccttttttacataacgatttattttcctctgggtagatacccagtagtggaattgctgggtcaaatggtagttctagttttagttctttgaaaaatctttatactgttttccatagaggttgaactaatttacattctcaccaacaatgtataagcattcccttttttctgcatctgcaccaagatcagcctttttttttttgactttttaatgatagccattctgactattgtaagatgatatctcattgtggttttaatatgcattctctgattttcaatgatgttgagcattttttcctgtgtttggcagctgcttgtatttcttcttctgaggaatggattttattgaatctgcagatcactttgggtaatatggacaatttaccaattttaattattccaatccatgaacataggatgtctttccatttatttgtatcatcttttatttcttttagcaatgttttgtaagtttttagtgtgtgatctttttcctcacttgttaagcttattcacaaatgttttgttttcaatgctattgtaaatagctttgtttccttaatttcctttttgtagttcattgttagtatgtgaaaatgaccttatttttgtgtgtcagttttgtttcctgcaactttactgaatttatttattagttataacaagttttttgatggactctttgggattttctatatgtatgatcatgtcatcttaaaagagggacagttttgcttcatttccgatttagatgccttttagtttttcttgctaattgttctggctaggacttccaatactaagttgaatagaagtggcgagattgggcatccttgcttcatttctgatctcagaggaaaagctttttgtttttcacaactaggtatgattttagctatgggaatttcatatatggcctaattatgttgaagttattttcctttatttctagtttgttgagagctttttgcatgaaagggtgtagaattttatcaagtgctttttctgtatctattgagatgatcatgctatttttatccttcattttgttaatgtggtatatctcattatttaattaattaaatttttttttttttgagacagggtcttactgttgcccaggctggactgcagtgctgtgaacacagctcactgcagctttgacctaatgggcccaagtgatcctcgtgcctcagcctcttgagtagtcgggactacaggcatatgccaccatgcctcacacatttttgtatgttttgtagagaaggggttttgctacattgcctagactggtctcgaactcctggactcaagcagtctgcctgcgtaagacgcccagagtgctgggattacaggtgtgcaccactgcacctgatctcattaattgatttttgtatattgagccttaattgatttttgtatattgagccatcccaatttatacccaaggataaattctactaggtcatgttgtattttacttttaatgtgctgctgaatttggtttgctagtattttgttgaggattttgcatctgtatttgtttggcacattggcctgtagttttctatatttggcatattggccttggtgatacagtctgcatcaggataatgctggcctcataaaatgagtggaattttctcctcctcctctattttttgggtgaatttttagaatgattggcattagttctttaaatgtttggtagatttcaccagtaaagccattggtcctgtgcttttctttgctaggaggtttttgattactgattcatatccttactacttataggtctgttcagacttatttctttatgattcagtcttggtgggatgtgtgtttctaggaatttatccgtttcttttaggtgatccagtttgttgatgtgtaaatgtttatagtagtcttttataattctttttatttatggcatcagttgaaatgtctcctttctcatttctgattttgagtcttctctttctttttcttagtgtagctaagattggttaatattgcttatcttttgaaaaatactaactcttggttttgctgatttttcaattctttttctagtctcaattttgtttatttctgatctgaagttcattatttcccttatgataattttgggtttaaattttctgttgcttttcagatttcttgggttgtaaagttaggttgtttatttgagtttttttttttaatataggttatcacagcaagctttccttgtattttttttttttgacagagtctcactgtgttgtccaggctggagtgtagtggggcaatcttggctcattgcaacctccacctcctggtttctagtgattcttgtgcctcagcctcctcagtagctaggattacaggcgcgcaccaccatgcctagctaatttttgtatttttagtagagatggggtttcgccatgttggccaggctggtctcgatctcctgatctcaggtgatctacccgccttggtctgggattacaggcgtgagccaccacatctgtcctccttttagtattatttttgttttatttcataagtttttacatattgtgttttttgtttgtccaaaagtattttttaatcttgtgtttgatttcctttttgacccaatggttgttccacagtgtgttgtttaatttccacatattggtgaattttccattttcctttctgcttttattgttgtctttttctattctaattgctagtttcatccattttggtcagaaaatatatttggtatgatttcagtcttcttaaatttctgaagacctgttttgtgacctaaaatgtgagcctggagagagttccatgtgtgcctgagaatagtatgtattctgccactgttgggtagaatgttctgtatatgtctattagtttgatttggtctgtagtgttgttcaagtcctgtgtttccgtattgatcttctatctagatgttttatccataattaaaatgcagtcttgaagtttcttactattattgtgttgctgtctctttctttcttcagttttgtcagtgcttgcattacatatttaggtgctctaatgctgggtgcatatatatttattattgttatatcttcctagtgaattgttacttttatcattataaaatgtttttctttgtgttttgtgacaattctgacatagagtctcttttctttgatacaaatataggtacccctgctctctgtggttaccatttgcatggaatatctttatccattcttcactttcagcctatatatgtccttagaactatagtgagtctcttgtagatagcatatagtttttttttttttttttttatccattcagtatgctatgtgtttttgttggggagtttaacatatttacatttaaagtaattcttgatagggaaggatttactgtgattgttttaaatgttttttgtttgtcttgtagctcttttgcctgccctttcttgctgttttcctttgtaattttttgattttgtgtgtgtgttgataattcttttatccctattcctttttcttttgtgtaacttccttctataggtatttgtttatggttaccttagagcgtgcataaaatatcttgtagtaataacagtatttttaagctgataacaacttaacctcaattacatacaaaaactcttcactttaagttctcccattacacagtttatgttgttgttacagtttacaatctattaatattgtgtatcttccaacatattttttatagtttttttttttttttttgagatggagttttgttcttgttgtccaggctggagtgcagtggtgcgatggctcactgtatcctccgcctcctgggttcaagtgattctcctgcctcagcctcccaagtagctgggactacaggtgcctgccaccacgcttggctaatttttgtatttttagtggagatggggttttaccatgttgtccaggctggtctcgaactcctgacctcaagtgatctgcctgcctcggcctcccaaagtgctgggattacaggcgtgagccactgcgcccggcctatagttacattttatactttttcttctaaatttacactagaagtgaaagtgatttacccagtaccattaacagcaacacagtattttgcatttgtctatatatttattcttactaattaattttatactttcttatgctcctgtgttgctgtctagcagtctttcatttcaaggtgcagaactccatttcacatttcttagaagaaaggtctaatcatgatgaacttccctgcttttgtttttctagaaaagtcttaatgtcttcttcatttttaaaggatagttttgccagatataggattctttcttggcagtttttttctttcattactttaatatgtcacctcattaaccttctggcctgcaagatttctgctgaaaaatccactaatggcctgatgggggttcccttgtatgtgatgaattgctttctttcttactgctttcaaaattctctttgtcttttgataatttgattgtaatgtttcttggtgttgatttctttagattcttcttacttaaggttctttgggcttcctgcatctggacgtccatttccttccccagatttgggaaaatttcaaccactacctctttgaaataagctttttggtactttttcttagtctgctccttgtgggattgccacagtgtgtatattagtctcttgatggtgtctcataagtcccttaagctttcttcacttatatttctttttttttttttgctcctctgacttgataaggtaacccgactttgagtttgttgaatctttattctgtttgctctgatctgctgttgaactcctctgttgcatttttccattaagttggtgtattcttcagccccgaaattagtgagaagaccttcactagttaacctggccagagcttttttgggcctctcaaactttcatgtttgttatactgccttttctattgttgttagcgctcagtgtctacaatatgctggagcctatcagtgttctgagaggggagaaagaagtgaatttgttgggcaatccctagaaaagttggaacatgtgacatgtggtccaacagtttctctttccagggaaaagcttggaagtgtttttttttttttttttttttttttaatcactatgttaaactgggtagaggaactgtggcgagtgtctgagtgatagtttgaacaaccaccttcattctttgtagccttcaggggtctagcacataccagctccatctgtgctctgagagaggagagggaaaagccaatttcttgggtagctcctagaaaaattgtagcgttggatgtgtggtcctcctttgggagaagctaggagctgtggcaagtgcccacatgctagtttaacctactacctttgttctctgaaaaccccagggatctaatatattccaggtcctatatgttgtcagaggcagatgagatagaaggtagtccctcaggaagcactctaaaaaactgtaatattggatgtgtggcccaactctttctctcctcagggagatgctgagagctgtttcctcctgatcttatatgacgcgtcatgagttgggattgcggcgagaaaggatctccagttttcctactggtttcagtgtggctggttttacaattgcctgggatgtagtagcctctcaactagtttctggatttctcacaaagggaattgattagtgtgttactgttgaattgctgactttttataggagatttgttagcctccaataaaagttaaaatgtacatgcttttagatctagtaattctacctttatgtaactatcttagagaaatatttgtgtatatacacatggggagtgtacagggatgtttattgcagcactgcctgttggaggaaggagaatccagagctttctattctcccattttggtgatgccactctggcttttatttttgtgcataaataaaatcagacttaatattgtttaaaattgacttaaaatctcttgtgtgcagatttttttctattacgatatcctggacatttttctgtatcattttattatgtagacatagccctttaatttgctgaatagtattccaatacaaggatttactatgatttatttaaccatactctcattaattactgtaattagtgttttctattgtaaacagtgctgccgtatacatccttgtacacacctcatgtgtatatatacaaacatacacacctcatgtgtatatatacagatatacacacgtcgtgtatatatacaaatatttttctatgatagttattgtacataaaggtagaattattgtatctaaaagcatgtacattttaacttatatcagaagctaatgaatttcctataaatagtgtgggtcagtttgcatttctgacaacagtatattatgccattgtgtacccatagtcttaccagcacaggataatatgttttcttaattttggcaagctgatgggtaaaaaataagaagatactgttttagtttacagtttttcatgtgattgtagattataggcatcattttcttctatgaattattattttatgtattccttatcagttctgttggttcattaaatcttcttttaaattgatttttagacctctttctataagatggacataactcctttgttatatatgttctaatattctttatttatagcttatttaacttttcataggttacattttatgttgaaatttaaaatttaaatgaaggcaaacttactaatttttttcctgtaatggtttcagaaatttgtatcttgacctggtttttagtattcctatatatagatcatcatcatagcccctctacaaattattttagttttttttaaatttaaaatttttatgttaactcttttaattgaggagggggcatgtggagtaagcttggaaattaaacttatccactaatgatcagttgttgtggaaccatttaaaatggttcttttacgataacctaagttcctatatacattatctatttcctgattccctattctttcatgaagccaactgtcctgcagtgtttttgaactggccagcattcaccttcaaatctttatgtgaacttatgtttttaatactgttgggtaaatgtcccggagtagaatgacttggttagatggtagaggtatttaacttttcaagaaactctcaaactgttttctaaagtgattgttccatttttcatttccatccttagtgtatgggagttctaattgtttcatatcctgaccaatacttcgtgtggtcagtgtttttaattttagccattctattgagtgtgaggtggtgcctcattgaggttttaatttgcatttccttagtaactaatgatgcattgagcatgttttcatgtgcttttttgccatcaggctatcttatggtgatatgactgttcaactcttttccctcatttaaaaattttgattacttattgttgagttttgagaatactttgtgtattctgtatacaagttctctatcagattgtcaatattttttccaagttgtagcttgcctttaattaacttagcagtatattttgaagagcagaactttttcatgttgatgaagtttattttataaacttgtaattttatcggttgttcttttggtgtcctatctaaggacttcttgcctgctccacagttgcaaaggttttctcctagaagttttatagttttaggttttacatttagttccatgatgcattttgactttttttgggtatatttcaagatgtacattaaagttcatttattttaaaatgtttattatgaaataattataatctgaaaagaagttgcaaaataatatagagtcctgtgtacttttcacccagttttccttagtggtgacatcttataaagctgtaccacagaatacaaaacagaacattgacattgctattttaacagagaagatgtctctgtgggtgggagtttgggggtaagaaggagccatggtggcccagagtatagtgagagaagccaagcaaggtaaaaaagagtgttcagctagggtgaagagccatccaacagagaagttagaccctgagcatgaagataaatgcctttatggacactgacctctctgtgatcatcaaacatactgttatgaactgaatgtttgtgcttccccaaaactcatgtgttggagccagccaccagcatggctacatttggagatggggcctttaaggaagtaattaaggttaaacgaggtcataaggatggggccctgatccactaggatcagtgtccttgtaagaagagacaccaaacatctcacttgccgtctctctgcacacatgcactgaggaagggctatgtcagcacacagcaagaaggcagccctctgcaagccaggaagagaatcctcactagaaactgaactagtaggaaccttgatcttggatttctagcctcaagaactgtgagaaaataaatttctgcagtttaaacctgtggtattttgttatggcattctgagcagactaagtaaggcacatactatatgatttctgtcctttgaaatatgttgagacttatacttgcagctgaagagacattgttaaatccagaaacagtaagcaactgtttctggagggtaactgctacaatcatgttagaatgaagtagattttaggtgtaagatgagaattttattaatgagtattcatgtcaattactaatttctttattgacagtcattttatgttcacaggaatgtgaattggacccttgctgcgaaggaagtacctgtaagcttaaatcatttgctgagtgtgcatatggtgactgttgtaaagactgtcgggtaaggaattcctcccttttggaaacaggaaaaaaaaaaaaaaaaaaaagaaaacctgtgtatatcaaaatttgttttttgagatttctgagtcagcactatttttattttatggtcatgggaaaaattttatgccacttgtgtataattttaaagcacactcttttacgttaagtggtctgttgatattgttttctaagtagaaacattttttttctgatttttagagtaacatatgcctgttagaaataattaaataacatgaaaccatagaaagtagagaatgaaagatcctctattattttatactcttcaggtaaccactgttgataatttgttaatataatcacgttttttctatacaaatgtgagtgtatgtgtgtatgtgtgtttttaagtgggtaagcacagatacatatatttttactacctgcttttttcaatatgacaccatggacttttttcccattcatgtagttctataatacatggttatttaagtaatattacttgtatagttgtaccataatttctttagtcaactaatgatggacattttgattacttccagttactgcttataagagaaatcactggtgcagaatattcatactaagtttttgatatacattttatatatctttcacacatatgccaatctatacttctaccaacagtattatcaaatacttgtttccttatgccaatattgggtactagcaggcactatactcctagttaattcaataggtgtaaagggttcttgtatttttatttagtttgcatttcttttggttacaaatgaggtcatgtttctttactttccatagttaggacttacatgaattacctgttgttagccattgttcatttttctgttgggttatttaatcttttgctattgttagaatgctttatagatgtaaatgctgtggtttcacatttgattaatttgtggacattatcctgatatttctgtttaatttgaattctatttcactagttccttccaggaggtactttatgccgaggaaaaaccagtgagtgtgatgttccagagtactgcaatggttcttctcagttctgtcagccagatgtttttattcagaatggatatccttgccagaataacaaagcctattgctacaacggcatgtgccagtattatgatgctcaatgtcaagtcatctttggctcaagtaagatatcatcatttataattgattgcttcgatattatttatttttgatttagatattttaaaaaaggtaatgaaacattattgataaagttgaggctctcttgtttctcatcgtatttcctttcttctttggaggcagtcatgatcatgaatttaatatgcacagattcagttgatgttttcttatttttactgtctatatctttttatattttgtgtatcacgcacacacacagatacatatatagtatctagttttaataatgttgaattgtgcacaaggatctgctatttgcattgttcactcagaattttcttgaaattcatctatattgatatatttatattatagtacattaaagtattccattagatgaatggatcatgatttagttattctcttactgatagatatttgggatttttaaaaaatttatgtattttttcttttaaaagttcttatttttatcaagggcatacatataaagagccaaattattgtgtaatgcatagtatgaacaaataaggactgttcccacccactattcccatcacttgaggcagttttaccttttttggctaagatttttgttaacttgtgctaggtttttagataatctcttggcaatgcgacgttttgatttttttgttctaggcattagttattaatttctcactatagaagatgagttagttttctttccttctcttccttcaacccttaacaactcccatcatacctatgctgattttccattcttcatcctcccaatagttagggcagtgatgactgtgtattgtataatggccacattaatgctcttcacaactaaactgtatagtaagttataattacttgcctgatttctctagagttactaattctgtctttctgtttctctctctctcttttggtttggttaatttcctatgtactttccattaattgacctgtatattgttaaccattggcctgattgtgccttgagttgattagtggcatcaagtattctatttatttcaatttgttcaaataagtctgaacagaaggcctctgttcctcttcagtcttgactggtttccctctgtatagttagttagggttctctagagaaatggaaccattgtgttgtgcgtttatgtatacagtcatataccgcataacaacattttggtcagtgagagattgcatatacaacagtggtctcataaaattataatgctgtatttttactgtaacttttctatgtttagatatgtttagataccttttctatgtttagatacgtttagatgccattgtgttaccattgcctacagtatttagtacagtgacatggtgtacagatttgtagcttaggagcaataggctgtaccacatagcctagatgtgtagtaggctataccacctaggtttgtttaagtgcactctgtgatgtttgcacaatgacaaaatcacctaacaactcatttctcagatcatatccctgttgttaagtgacacattactgtagatattactgtatatataatctggaggaattattacgtgaatctaatatttatatataatatataatttacatataatatattaaatatataatatcttatatatgtattacatgaaaatcaaatatattctcctggaggaatctgatatattagattcatgtaataaatcctgcgtaatagcatgagcccatatatgaattggcttgtgtgattgtggaagctgctaagtgtcagatctgcagggagagtcagcaatctggagaccctgtagagctgatggtatagttccagttagaagtctggcaggctcatgaccatggaagagctagtgtttcagttcaattccaaaggcaggaaaaaagctgatgtctcattccaaaggccttcaggaagacttttctcttacttgagggaggactggccttttcgttcaagtttaaaattgattggatggggcccacctccaatagggagggcagtctgctttactcatcctactgatttcaatgttaatctcatccaaaatcacccttacagagacatccgtaattatgtttgattaaatatctggggattctgtggctcagtcaaattaactctactaaaaagggtaaaattaaccctcatcaaaaatccactccttgtcagcttgaaacccatagacaccttaaaccataccaaatctccaaatgtggaccttgttaagggcataattccacctagcatgatataataacactatcctgcatgcaactaaaacctcactaacctcttttccagaaaaggaggtaaagtgatgtttattcttcttcttgatatcccataacttaaatactgggatataaaattaacaatacttaaatgctataatatcaagtcaatatgtcttatgctgcatgataaaggtataaggaatgagaacatatttgctcagtacgtgtgtgtgaatgcacacacacatacacacatgcagctattcttaatgaaacagtcttcgtttctgcaactggtcatgtggttgtagctggtatttataactaacttccacccattctgtattccctttgccttcagcaagcacgttagctgtttgtggttctttacctgttagggtgacccaaactgtcgttcttgaagggtctgggccatttgtagtccttcctagattgggttgttaaagttttccattgaacttaaacttaatcatgaagcatggtaatactaagagatgccctaagggatctccggcattctagacatactcttccttgcctccattttggagtagtaggccagtttccctttggtggttcggatcagtaattctacctggcatagaaactgccttctttgcctgttgacttggaggtatgaggagccaatgtggctgggcctctggcttaatttctagttcagtagaatcattattgtggctcctggtggcagcattcctccttttggaactaaggcctctagtccagtagagcataaggtcgtgggaacaggaaacaaaattttgctagtgggtcactatggataatggtgagtggtgtttctcccatttccaccccttgatacctggacacgtgaatcctggttatgggaaaatcagcattggatgttggctgctgattgagagcatatacagccttttggagaaccttgccccagcactgtaaggtattgctacctagtggcactgtaactgagtctccaaaaggcatttccaccatgctgtcagccagctgcttcaggatggtggggaaggaacatggtaaggccagtgaattccatgtgcatgggcccattgcctcatttcatttgctatcaagtgaattctttggtttgaagcagtgctgtgtagaatattatgatggtgggggaggaattctgtatgtccacagaaggtagttttggtagttcacaggagtgttgctacagagatggcaaatctatatcaagagtacgtgtgtctgtcccagtaagaacaaagcactgcttctttcatcatggaaagggaaaaatgtaatcaacctgccaccaggcagctgactgactaacctagggaatggtgtcatactggggactcaggattggactttgctactggagaatttgggcacttagcagcaacaatgccaggtcagttgttgagaggaagtccatgatgctgagcccacgcatcgcctccaaccctgccactgtgagtacgtggttcctgagcccatggatgagaatagttggctggggaaagaatgagtcatcctatctacttgattattaaaattctcctctactgaggccaccctttggtgaacattcacatgggacacaaatatctttgccctacaacccagtcatgggccatagcccataaattggtgtataatcacgtctggctgtttcttctcccaaggaaagtgaacaaccaggtgcacttcagggatgtcccagaaaggggctgcagtgctacagtcatccacttttggttcttcatatcatatcatgtgtagaaccatctgcaaaccaggtctccgtcttcttttctactgtcacctgatgggtaggaagttccccgtgaggtcatagttgctggctaggagagaaaatgtagtgtagcaggagtggggagcaggggcatgtggggcacttctttatgtaacttgtgccttccaggccttggtttggctcaattacatacgtagcacttccatttcatgatggggtgctgctgcatatgcccagctttatagcttggtgagtcagatgacatccagtttatcatgggcaactcaggttgaatggtaacttggtgggtggcccatggttaaatgttcaatttctactttaaggcccagtagcaggccaatagttttttctcaaaaggagagtagttattcgcagaggatcacaaggctttgctccaaaatcctaaatgcctgcactgcacctgacctatagggaactgtcggaggcgctaaacagcatttctgtctgtaactgctgcttcaagcactgtttgatctgcttgatcaagtgggctaagcagcagagcatcttgcctgacagcctggacctattgcagagtttctctttgttctgggcccagctcaaaactagcagctctttgggtcagtgggtaaatgggccagagttatgcaaccaaatgaggaatattttgccttcagaaatccaaatggacctctaaacattgtgccattctgttggttgtgggagtggccagatgcaacttcttcttccccttagaaaggatatcttgacatgtcccacaccactggacatgtagaaatttcactgaggtagaaggcacctgaatttttgtcagatttattttctactttttgtcgtgcaaatatcttgccagtgacaagaatagttgctgtttcttgctcactaggtctaatgagcataatgttttcaatgactagtgtgatattttgtggaaggaaaaggtaatcaagatccccaaaactaaattatgacatggggctccagagttgatattcttcctaagtaggacagtgaaggtgtattgctggccttgccagctgaaagcagctgcttctggtaggctgtgtggatgggtataggtaaaggttttttcagatcacagctgcataccatgtattaggggatgtgttaatttgctcaaacaatgaaatacatttggtatagcagcttcagttggagtcaccacttagctaagcttataataatccactatcattctccaagatctgtctgtcttctgcacagggcaaataggtgaattgaatggagatgtgatgagagtccctgcccctgcatctttcaagtccttgatgttgacacgaatctctgcaatccctccagagatgtggtattgcttttggcttactattttcctaggtagaggcagttctagtgggttccacctggcctttcttaccataataaccatcactccacaggtcagggaaccagtgtggcaattctgccagctgttgagtgtgtctgtttcaattatgcattctggaattgtgggaaaaaacccacaaggtgggttcagggacccactaggcctgctgtgagatggacctgaggtaaaacttcatctatcacctgaccttcataagcccctactctgacttcttgaccacagtgacattttgggtttgctcaattatttcagatatagggttctgtgttcctgaaaggtcgaatttttttctcagtgcacagtgtcttagtctgatcaattctgtctcagtctattttgtgctattataacaaaatgccacagaccgggtaattaatagtgaacagaaatttattggcttctggaggctgggaagtccaagataaaggtgctgccatctgatgagggtcgttttgctgagccatcacatgacggaaggtggatgggcaagagacgaagtggggccaaacgcacccttttataacaatattaatcttatcccagagggcagagccatcatggactaatcacctcttaaaggtcccacctcttaatgctgtcacaatggtaattaaatttcaacatgaattttagaggggacagacatttaaaccatatctggctgctctaacaagatatactgtagactgtgtggcttaaatggcagacacttatttctcagagttctggaggctgggagtctaagatcaaagtgccagtcaatttggttcttggtgagggatctctcttttcttcttataagatcgccaatcccatcataagggtcccatcctcatgatcccacctaactctgattacctcccaaatggcccatctccaaataccatcactttggggttagggcttcaacagatgaattatgggatacacaaacattgaaggggtacacaaacgttcagtatataaccattgccctggtaaaagccataggtcccttggaaatgtctgggataatgattaatagtataaatttttggcattgtatgggagggttcttccttaaagaaacttaccctgcctttagttgagagtttctgtttctgtaaactggctcaactcaaggaattgattaagaggctgtgactttctgtttttatgattcaaattagacttttgtttacttggcctagagttttcttatttggtacaggtcaagtaagactatgggaagctgcctatcttgcttctacttagacagaaacagtgtgatcaactagccaatgccgtaagtttttacatgggtcaggttattctgattgctgctttgactctgctctccattatggtaaccttggctctccattatgccaaccttggctctccattatgcccaccttgcctttggtggttgaatgttgacactttcctatcacctagaatctgatactttcattgcatttaagtttcccaactcagtggccatagctcctactataaggtctgccctttagataagagtgatcacagagcttttcaaggatgctaggcctccccttacaaatttatttcttacagtcttggtgaaaggtgtgttttctggattcttccagggtgggtaaatacatcttaagtgacaaatcgactcaaacattttagtctccctcagactttgaatccctttctctgcattaaactgagataggccctgcattcctgacttgctcactgtgagctgccttttgattcacatttcagccaaccaaccgaacaaactgttagagacctttctaactccctgaatggcaacattcaatgcagactgtctgcttcgtgagtcctcaccaatgaattcatcccaatccaactttatgttcctcccaccattatctcacgcccttaatatccattcccacacatgttccctggatttctgtctgtgtaaattagaaaactcaagtagtcttggagtgtggtgaacctcctcatgggttgtatttagtatttcacctttaggggcattttctatgacttgagtctagttataggtttagaaccaatgagatattttggaggtggatcctgagggaaattggcattatcttgcatggcagctgcctccagggaggctattacagtttcctcaggcaatgcagggttagtcccctcagatgttggagacgctgtttccactggcaaagacgactcatcagaatttagaggctcagccaggcgcctgtaatcccagcactttgggaggtgaggcaggcagatcacttgaggtcaggagtttgagaccagcctggccaacatggcgaaaccctgtctccattaaaaacacaaaaattagccaggcatagtggtgcactcctgtagtcccagctacttgggaggctgaggcaggagaatcgcttgaacttgggaggtggaggttgcagttagctgagattgtgccactgcactccagcctgggcaacagagcaagactctgtctcaaaacaaacaaacaagaaaagaaagagtttagagctcagtgtacccagctttatcaaagtctccccacatgtcctcatttcaactttcaagatccagttccttattgatcaataacctcaatttaacagtagataccctacaaggctaggagttcaatttgctttcagccagtcacaggataagattctaggtttgattttcaacaatctcagctctgcaactaccggcgatatggctgtcctttagggcacacacagaaaatttcaggtcacttatatggtgcttgaactaggaatccctgcgcttatcatcttctttccctactttgtccagtaaaataaggagcaaccaggcaatctcatactgttagtatgagaaaaatgtttgaaggcatcatatacatagttacccagatccttgcttcttgtaaatgtctgattaggagtctctagtgttgatatgtttttggactgcaattaccatatcatgccgtgaactatcagtgctacgttaacttttggaaatagagtcataagtgtctttaaaaatctaatcagattagatagcccattctagaaaccttggaatcaattcagaaaactcattctcaaagttctgttcctctggaaccactgttggtccaaaatctgaattagttagactgcagagaaacaatatcaattggatatatacatattatatatatgtttattcatttattataagcaattggctcatgcgattatggtaagcaactgaaaatcccagatttgtaggatgatttggcaagatggagacacaggagagatgatggtttagttccagtccagatttgaaggcctgagaaccaggattgccaatagtgtaatcagtatttatcctgagatctttcaccataatctgaaggcgaatcattggctctctcccttttgaatctcctgtttgcatttcccatattaccttctttctttgtttatttcctcctttcatggagctttcctttcggtagtttccttagataaggtgaattagaggtaaattttttgagatcctgcaagtgtgaaaatggttttatttggactaaatacttgattgatggggatggaaatcattttctgtcacagttttgaaggcattgctttattgtcttccagtttacagagttgctgttggaaagtctgaagccattctgatttttatacctagcttttccctcaccccctctgaaaaagcttggagaatgacctcttcaaggtgatatgccttgatgtgggtttgtttttattcaccgtgctatgtaattggtgggtacattcaatctgggaactcattttttttagttctggaaatttcttccctttcatttttttggtgtgatttcttttcctggatcacatattatttggatattggatttactagatttccttggattttggatttcctggattttcttatctttcctgtctttttatctgtgtttttttttgttttttttttttgacctactttctgagcaacttcttcaactttatcttctaactcttttattgcggttttcatttcaggcactatgattttagttttcagaaactcttttatattctctgagtttttttcccacttatttttaagaaataatctattcttggccaggcgcggtggctcacgcctgtaatcccagctctttgggaggctgaggtgggcggatcacaaggtcaggagattgagaccatcctggctaacgtggtaaaaccctgtctctactaaaaataccaaataaaaaaattagcctggtgtggtggcaggcgcctgtattcccagctactcgggaggctgaggcaggagaatggcgtgaacccgggaggcggagcttgcagtgagccgagatcgcaccattgcactcgagtctgggcgacagtgcgaggctacatctcaaaaaaaaaaaaaaaaaaaaaaaggacataatctgttcttatttcatgcacgaaacatctctcatgtttgtcagtatgttaatgataatttttttcttttttttaaatatattttaagttctagggtacatgtgcacaacgtgcaggtttgtcacatatgtatacatgtgccatgttgatatgctgcagccattaactcgtcatttacattaggtgtatatcctaatgctatcccttcccactccccccaccccatgacaggccccggtgtgtgatgttccctttcctgtgtccaagtgttctcattcttcaattccaacctatgagtgagaacatgcggtgtttggttttttgtccttgggatagtttgctgagaatgacggtttccagcttcatccatgtccctacgaaggacatgaactcatcctttttcatggctgcataatattccatggtgtctatgtgccacgttttcttaatccagtctatcattgatggacatttgggttggttccaagtctttgctgttgtgaatagtgctgcaataaacatacgtgtgcatatgtctttatagcagcatgatttataatcctttgggtatatacccagtaatgggatggctgggtcaaatggtatttctagttctagatccttgaggaatcgccacactgtcttccacaatggttgaactagtttacagtccaaccaacagtgtaaaagtgttcctatttctccacatcctctccagcacctgttgtttcctgactttttaatgatcgccattctaaatggcgtgagatggtatctcattgtggttttgatttgcgtttgtctgatggccagtgatgatgagcattttttcatgtgtctgttggcttcataaatgtcttcttttgagaaatgtctgttcatctcctttgcccactttttgatggggttgtttgatttttgttgtaaatttgtttgagttctttgtagattctggatattagccctttgttagatgagtagattgcaaaaattttctctcattttgtaggttgcctgttcactctgatggtagtttcttttgctgtgcagaagctctttagtttaattagatcctatttgtcaattttggcttttgttgccattgcttttggtgttttagacatgaagtccttgcccatgcctatgtcctgaatggtattgcctaggttttcttctagggtttgtatgattttgggtctaacatttcagtctttaatccatcttgaattaatttttgtataaggtgtaaggaagggatccagtttcagttttctacatatggctagccagttttcccagcactatttattaaatagggaatcctttccccatttcttgtttttgtcaggtttttcaaagatcagatggttgtagatgtgtggtattatttctgagggctctgttctgttccattggtctatatctctgttttggtaccagtaccatgctattttggttactgtggccttgtagtatagtttgaagtcaggtagtgtgatgcctccagctttgttcttttggcttaggattgacttggcaatgtgggctcttttttggttccatatgaactttaaagtatttttttccaattctgtgaagaaagtcattggtagcttgatggggatggcattgaatgtataaattaccttgggcagtatggccattttcacgatattgattattcctatccatgagcatggaatgttcttccatttgtttgtgtcctcttttatttcattgagcagtggtttgtagttctccttgaagaggtccttcacatcccttgtaagttggattcctaggtattttattctctttttagcaattgtgaatgggagttcacttatgatttggctctctgttattggtgtataagaatgcttgtgatttttgcacattgattttgtatcctcagactttgctgaagttgcttatcagcttaaggagattttgggctgagacggtggggttttctagatgtacaatcatgtcatctgcaaacagggacaatttgacttcctcttttcctaattgaataccctttatttctttctcctgcctgattgccctggccagaacttccaacagtatgttgaataggagtggtgagagagggcatccctgtcttgtgccagttttcagaggggatgcttccagtttttgcccattcagtatgatattggctgtgggtttgtcataaatggctcttattattttgagatatgtcccatcaatacctaatgtattgagagtttttagcatgaagggctgttgaattttgtcaaaggccttttctgcatctgttgagataaccatgtggtttttgtctttggttccgtttatatgctggattatgtttattgatttgcatatgttgtttaaaaagttttctttcttctgcgtaacctctgtttcatattaccttttttctttgtttgagtttccatctttcacattagccatgttcctcagctctcccatagtccctggtccaaaggaggggaataagaagcagagaggtcactctaggctcatgggggaggcttgttaactgaaagctttcctataggatgatacagctgaactttttaattagggaaatggaaaatccacatctttaggtttttttcctcttgggcttgttaagattcccttgtgaagaccttatctatctgcatcctggagggccaagtcctagctgtcagtcgggcacggtggctcacacctctaatcctagcactttgggaggccgaggcatgtggattgcctgaggtcaggagttcgagaccagcctggccaacatggtgaagccctgtctctactaaaaatacaaaaattagcttggcatgatggcgggcacctgtaatcccagctactcaggaggctgaggcaggagaatcgcttgaaccagggaggtggaggttgcattgagccgagatcatgccattgcactccagcccgagtgacaagagtgaaacttctcctcaaaaaaaaaaaaaaaaaaaaaaaaaaaaaaaaaaaaaaagacctgactgtcagcattctgggagggaaacaggaggtgagggaaaataaggctgggacctcagtatgaggtaggtaaatgctcagttcatccccttgtttttagaagagtttctgtgcctgttactgtgcctggtatctcttgagtcctggaaccttgtgttctactctctccagaaaataaacctccagtgttttgccagggtagagaagagacagtcacttggcttcacaaagatggtaggtgacttgtgggccaaactgcttcttaagcagatttaaaatttttcctctttattcctgccacctgcccctccttattctctatagccagaggtacctattactaccagtttcttatctccgaggaattctacggtgtaaaaagggttgatctcagttttttctgttgccactttaagattcagttttctgagatacattgagtcatttattacttcaccaatttcttttcggcttctaagttttgtgcagtctcctttcccagttccattgtctgtgggtttatgaattaaaaaaaaaaaactactttctgtgggattttaggagggagggaaaatacgtgcatgtattcagacttcttacctgaagtttgttgatggcttctgattttaaagataagtcaattctggtgttataggtctagttttcattcctttgaacatttgaacatgtggagaataaggatttaaaagtccttcactagctcatgcattctcaaattccttatatttttagtaaacaccaaataaatatttatcaaataagtgaagaacttgagagctaacataagagaaggtattgacgcttactatcaaatttggcccttaaaaaaccttatgaggaaggcagggctcagagagctaaatggtttgcctgaggtcacacaacagaaagcagcaaaaccatgatctcatccaccgtgagcatggtgagctgatgaagacttactgctagaatttatcaaagacattgttaaaggaaaataacttacattggtttacttcttaaatggaaataggacatattgaaatattgaatatacaaataagcaaaaggtagaaaataaatatttcctctactgtcaatattctggataagtaactgttgaaaatttcatgaatatctttcacttattttttgtgcatatgagtgtataatatacaaaaatggtatcatattgacatactgctttaaaacctgctgcctttcagcctgggctgcatagcaagaccttgtctcactaaaaaaaaaaaaaaaaaaaaaaaattagtcaagtgtggtggtgcatgcctgcatttccatctacttaggaggctaaggcaggaggatcactttagcctgtgaggtaaaggctgcagtgagctatgaccttgccactgcattctagcctgggcaacagaatgagactctgtctcaaaaaaaaaaaaaaaaaaaaagctaaaatgtaactgcccgttttcaatactaacaataaattgtgaatacttttccatgttaaccatttttctacaacattgtgttaatgatatactataatttatttaaacagtcaacagtgttagcagtaaacatctgtatggtttagttgtggcctccatttatccttctggataaatttccagaagcaggattcctgtattaaaggcttctaagacatttccacataatctccagaaatatataccactttttaccttcatttgctatacgtgactgttcattccttcatatgtttccaacatcaagtatttccatttttaaaactttgccaattgaatagccacaaaacatatttttattatttaaaaatatgcattttgcaacataggcaacatagcaagaccccatctctacaaaaataaaaacaaaaattagccaagcatggtggcgtgtacctgtagttctagctgtttgggaggctgaggtgggaggattgcttgagaccaagagttcaaggttacagtaagctatgaacgtgccactgcactccagcctgggtgacagagtgagatcctgtctcttaaaaaaaaaaaaaaaagggaaagcaagaatagattgttactttgtcatctgtcgtcagtgtttgtcaatgtatttaattagtagggacatctaaaccaagcatccatatatgataaatgaaaaaaacaaaagtattagctggcagtgttttctccaacccttcctagctgatctaaccagtggtgcagttggtttatatgtgagagcaatgagaatgaatatgctgcaaatggtactatactgtgcatggtttttaatttacttataatctattatttaatagtgtttcttttagggcttgagtttgaattcaggctaacttttaagtacaacttaagatttatttttacattttgtcattacatatgaaatgtggaacaaaaatgtatcatgtgtgaggcaggaaaggttttccacggtgttgaggggtattgaggctgttcatccaggtgtttagactgttgtagggaatacttttatttcaaaagctaaattgccataactttttttttctttttttaaatgtttaatgttacagaagccaaggctgcccccaaagattgtttcattgaagtgaattctaaaggtgacagatttggcaattgtggtttctctggcaatgaatacaagaagtgtgccactgggtaagtggaggtgcggtcataatggaatatgaaagattataagatccgtcatctctagtatcttttttttttttttttttttgagacggagtcttgctctgttgccaggctggagtgcagtggcgcgatctcggctcgctgcaccctccgcctcccaggttcaagtgattcccctgcctcagcctcctgagtagctgggactacaggcatgtgccaccacgcccagctaattttttgtattttagtagagatggggtttcaccatgttggccaggatggtcttgatctcctgacttcgtgatccgctcgcctcagcctcccaaagtgctgggattagaggcgtgagccactgtgcccggccgtctctagtatcttttacaactgctctctgtgaccgctgattttctcccccttaaatacctaacttttcaaacattttacaatgcaaagcttcagagagactctggtgttaggaaaagaactggtaacataatttgtccctttagacatcaactacaatctagtggtttttagactcttattttgtttatccttgatttataataagaaccccaactaaacaccattttcattttcctttccataaaagattatgttactaagtccctagataaaggtacctgcagaagaaactctgaacttcattattttcttctagctttgtataatttcaagatgatgaatttaaaatattttatatttctacaattaacatttgctttttgtaaaacattaataatgaaacattacaaaggaggaaaaagtcatgtataatctcaatccatatatgttcactaatatcagtgaaattattttcttcttcacactaacattttacatagttggaattattctgtaatattatcattgcttctacccattctacctcctatgctatcagttaagctaagcaactacagtaaaacagtgcttgctaagaagaaatagcaacaaagacccccatgtcactcaatctgacagtcgtttttaggtcttcatacaatagtacttgacctgtcagtagcattcaattatgctggccattttctccttcttgaagaaacctctttttttttggtgattgtgtagggtgttcttcttctcccctgaccccatgtgatttcgtttacttccgtggcttcatttgcctcctctctgagaagctccagccctgctggcctgcatgtggcctgcggccacagggctctgcacctgctgttccctctgttcagcatgctgtctttccccctctcagcctgctcagttcttcgtcctccagatctcaggtgaagtgtggtttccttacagaagacttcttccacttcctcaacaggaccagctctccctctgacaggtgttcttgatgctgtttgcttctttttcatagaatttgatatgttttcattattttttagttcatagtattttctaatttacactgatttttttcctttgactcgtgttattgaaagcctattgcttaattcccgagtagttgggaatatactggttatctgtttggttttgatgtctagttcaattccattgagaacacattctatatgatttcacttttttggaatttgagatgtgcattattcagttacacttggaacattcatccatacagactaatatgtgggccagcctcttaataccagaccaatatatggtctgtatgggtaaatgttccatgtataattgaaagaaaaagtatattctgcagttgttagagatgttattctataaatgtcaagttaatagtcttattcaaatatttcatatctatggtgtacgtgtgttatatctgttccttcaatttctgagagaggtgtgttgaagtctccagttatgattgtggatttgtctatttatctttttaggtatgtaaatttttgctgtgtatgttttaaatttgttactaggtgcatacacaattaggattgttatgccctcctgatgacttggagggcattagcaaatttatcattagcaaattcttttcatttctggaatattcttttgaagtatttgtcagtttcattaattatgtagctcttttgttatcgctgttcctcactaaactgtaaggttcagtgacacattttatcttgcatttagcataatgcttggaggaaacataataaatgactattaaacattgaatgaatgaaggtacagatgatatggatgaagaatgaatgggtggagaattaatataaccgattgaatgaactgatttaaaatctagggataagtggattaatgcagacttggaaagaatttgctggacatataccatattcttgtctttagccttgtcttgtttcatatttttatgaatatcttattgaaaatagcaactatacttatcaaactttaaaattactgagtcatttaggaagcattttatgtaatagtagtatacaaacaatatagtcattaagaatatacatttgaagttagactctttggatttgaatccttgttcaatcacttaacatctctgagtctttggacaaattacttcacatacatacctcatttttctgttctgtaaaatggggataataatggcacctgtttccaagtgttgttttgaactgaatgagttaatgggtgttagtactaagaggaatatctggttcattgtcacattcatcatcatcatcactatttttgttgtcatcctccttggagaatgtgtaaaatctggaaaagtcttttctacccattgaaactaccaaaaacatctagaaacatttaaagaaaggattcacatatggtcctaccatccagagatatttccttaagtttttgttgtatttcttttttatgtgtatatacatttataaacataagccaaatgtttcctttcactaaaagggttatcttttagtacatagacaatgtcattttttcaagcattataaaaaagaaattccaaatatacagaggagtagaaagaatagtgtgatgaacaccaatatatcccagaccaagacattattaatgccttatcattatttgcttcatcaagattttgctgaaccattttaagtaaattatagacatgatactttactcctaaattcctcagcatccgtcttcaacaaataaggccattcacatgatcacatcacacctaacaaaatgaatgatttcctaatatcatctagtatctgatcaatattagtatttccataagtgtcctcaaactgtcttttatagccggcattttccaacatccggactcaatcaaggatcacacattgcatttagttgttatgtcacttaagtcacttttaatccagaataccttttagactgattttttttcttttcagtgacattgatttatggaaatggctgggccagtgggctcatgttctggatttgttttagtttccttttggtgttgcttaacttatgtctctatcatccgaattttatttaaatcagaagttaagcccaaaatcttttttttttttttttttttttgagtagagcctcactctctcgctcaggctggagtgcagtggcatgatctcagctcactgcaacctccacctcccagattcaagtgattcttgtgcctcagcctctggagtagctaggactacaggtgtgcaccatcatgcctggctaagttttgtatttttagtagagatggggtttccctatgttggccaggctggtctcaaattcctgacctcaaatgatccgcttaccttagcctcccaaagtgctgggattacaggcgtgagccaccgcgcctggccctaagcccaaaatcttaattgaattcaggttaaatatttttggcgagaatgttcataagcaatgcattatatcaaggagtcacttagtgctgggtagtcttattaatattagtgatactaagtggcaatgaccagatcttgctattgtggagttatgctttttaaaattgcagctgtcaggtaatatgtggagtgatgagtttgtgccatatgaatatccagttcctgaccagtgtttcactttatggatgatccttgcctgaagcaattattttactgagggttgtaactgaattttgtttctgttagtattattcaacagtgaatgagcatctcagttttgttggctgtttacatttcttattttatgagctgcctgtttacatctttgctaatttttctgttgaagtgattttctttgtcttaatgatttgtaacagctttttatattctaagagtattttcctttactttttaatgtatcaccaagcctatgtatgaaatactgagtatatcatagcaatgtgaattttggtaggccccaacagatcttaactgaggtctactttatgctacactttgtttttgaggttttcatatctaatttcagctaattatgtgagataggcatcatttatctcatttttttcagctgaagaaactgaagctcagaaaatgtaagcacttctctcaggtcagctagcaaataaatggtgacataagaataaatgtaaagttgggacaaaattattaactcttaaatgcaggatgaagggaagatgaagacttaatagcagcacaacaaaaattaggagttttagtgatatattcaaggacatcaataatataatgtagttataaaagctattgtaatcttgaacttaatagaagtacagtatctagaataaacaagagctccatttttttctttgctcaccaggctgtcactgaaatttcatgctccattctgagcactatgcttcaagaggcagtgaggcaaactggaacatatttaggagggagcgtccttgttgcatgaaaagtgattgtaggatagtgacctggtgaagtaagtatttaggagctgcataataattgtcctaaaatagctgctgtgtgaaagaaggaaaagatatctgtgtagtctcatggggaagatctgggaccaatgaggataaatgctttacagatgtagatttttacctaataagcagaaagaagaacgtgatgggagctagaatgggcagtttcaggagggtgtaaattagagatattgggaaaatatatcctatgatgactgggcagtgatatcatagagaagattcagatatagagtaggtgcttggatcagatgacaatcagttaaacaggaaatctcagtacagcatcataagagttattgttggaaatacctagagtgttatgaaaggatataggaagggcatttaattcacacagccttggcaataagaattatggtcagggaagccttcatagagttctgatatttaattaatgaattaacgagttaatgaattgattctttaaataagtaaccaagagttagccaggaaaagaggggtggaatcctttcttagttattttgcattatagaatctaatttcttctttatcataactctgtaagaagacataattgaattttgatattgctatattattttctgtataatagaatttataaaattatacttagaaacaactttattagttaggctgttgagctctagacagacagtgaagaagattaagtgtggtaaaagaagaagcatcagcaccagctggtgccctaatttgcatcttagcatccacttaactcttttttcgccttttctgccgtatttaaagagagctactttgacctctcttgctctcatacactttctctgttgagattccctccatagcagcaaactctgtccatatgcaaatatataaattttttcttttgttatgtatactggatgcattttatgttgcattatttctctctctttataggaatgctttgtgtggaaagcttcagtgtgagaatgtacaagagatacctgtatttggaattgtgcctgctattattcaaacgcctagtcgaggcaccaaatgttggggtgtggatttccagctaggatcagatgttccagatcctgggatggttaacgaaggcacaaaatgtggtgctggaaaggtaatcaaaatattttttatttacaaagtaaaatgaaaaaaattaaaaaaattattatacatagtaagtggttgctcttttctgattgtaaaagtaatctaaattcattatagaaattttagaaaatacaaagccaccaaaagaaaattaagaactataattctgttatccacatttccttactggggtcagataaccagtgttttccactttgcaatatactgtgcatggttccctcccctactgatatgctacaatttattagccagtttgctattactgggacactttggcgatgtcctgaatttcagggtgtgtgtctgtgtactagaaatgtcatggagcttgtcctgcccatgttcctgaccacctgagctctgctgtttggattagatagaaggccagagtcagtcagcccatgacttattactagtggtttcatatgagaagatgccctgggccaaattcctttttttggagaatataaaattaaggagggtaattaagagtgcgggcagaaactgtaagaattcgttgggagatgctgtgaagtaggagctggggtagaagggatgtggcagccttaagccatatacaagagatatgagggagcaggattgttgagtaagttgaagaaaccaactcagaggagagagagaaggagaatatatgattgactgattagcccatgaaaaagacaggtgggtgggccttcaagttacttcactttctcccaagttttcagttccaattctgtttctcacttctctttacaagaagatccatatatttttggtcctgtccttgcaactaaataaacttgatcgttgcagctgttataaacaatgataagagatatatacatttaagtttttgatagtgcaatttccctttcaataaggtggtaacaatctatatcccagcctaggcagcagaggaagactctgtctcaaaaaaaaaaaaaaaaattgtgctgaaaggctcatgacaaaaacaactctctgacatgctcttatctaatctgccagtctagacgcctagaagcaactgtggttacttctgttaattacctccctattttaaattagggctgggcacggtggctcatgcctgtaatcccagcactttgggaggctgaggtgggcggatcacttgaagtcaggagttcgagactagcctgaccaacatggtgaaacctcgtctctacagaaaatacaaaaactagccagtgtggtggtgcatgcctgtagtcctaactactcaggaggctgagacaggagaatcgcttgaacctgggaggcacaggttgcagtgagccgagattatgccactgtactccagcctgggcaacaaagtgagactcccatctaaaaataaagtaaaataaaataaaataaaatagtatgctatttctagatttatctattttagacattatccactagttttatttttgatagataagaattcaattttcttatgcaaatcccagtttccctgctgtaccttttcaaaataagtgcttaatatttacataattaatattggggtgttattgaatgagtccacaacatctcactgttcactgggcatattccagacgaggtgagagaaaacaggggaggctaaacaattggagatcaaaggatcatttttattaggaagaaagcatgtaacatgacttaagtagatagcaaaaatgggcttcctaatgctgccctacacagttaaacttacctgtccagccttacctgcgaagtttaactgcatggttgaaagggcagaccagaatgcaccctttctgccacctcagcttactactagctggcaccacaggtgtaaccagcatgcctggctaattttttttaatttttctgtagagacaggatcttgctatgttgcctaggctggtcttcagctcctgggctcaagcgattctccctcctcagcctcccaaagtgctgggattacaggtgtgagccactgcacctagctgggcatctttccatgtctttattagatccatgtatttttttctgagaagttcatattgatatctctttttctattagcttgccattttttgaggcttctcatatgagaagaatattaactgtcagtcagttatatctatgtaaatatgatcaacaatttgacataagcctattttaaaatatcatgaattttttttttttttttttggagcctcactctgtcacccaggctggagtgcagtggtgcaatctcagtgcaacctccgcctcccaggctcaagtgattcttgtgcctcagcctccccagtagctgggattacaggcatctgccaccatgtctggctaatttgtgtgtttttagtagagacggggtttcgccatattggccagactggtctcgaattcctaacctcaagtgatctgcctgccttggcctccaaaagtgttgggattacaggcgtgagccatggcatccggccttaaaatatcatgaaattatatcagtcttatctgttttgtcttggtttcatgtcatgtttagaaaagctttttgtatctcagtataatatgaatatctggcttttattggcacaatttattaacatttcatcctatttctctgatcttattgctgctgttaaatattttcttgatattttctactttatcttcctcttgcagtattacacaaattatttatttgtgtgtggggtgtgtgtgtgtgtgcacatacactttggtagttgtatgtctttctattctgcttgtttacttaataacaaaaaaatgaatatatttttctcaaagttgtcgtgattaaaaatagtatctactgattgttgcagtgtaagctataccactattacttccaaacccccatgtcccagtttttacttggtaggaaaaatattggctttagattccaggttgttattaacatatatcaatgtatttttaagaccttttgtctttctggattttattgctaactgcatagttttctagctatgacaataatatttatgtacaagaaaggatagcaagtggttggtgtgtgtacctggactgatacaccttgacccaaactgacatgccgttgagaccatataccacacgttctgtacagctgtaactttgtaactgttggtttaatctatgagtctaacacccaagttttcacacggcagataggatcctgtcccttctggtatgtaccaaagcctagactggacagtttgagcagactgacaacttggtacttcttcagatctgtattctttatatatttattcaacatttatttccaggacaagctaaacgtggggtagggggaaaagtggaaaataagaactcctcaccttcatttttattgtcccaggtagttcaattttgctccccacttgcatcctgaaatcagtaaaccagaagtcctatagtcaagtttgctctacttgctgcgtggtggttgttggtggtggccatgggtggtagggggagtggtagtagtatgtgagaggatggtcttaccttcccactgtgagagttttttttttttttttttttgaggcagggtctcgctctttgacccaggctggagtgcagtagagtgcagatcttggctcactgcagcctctgcctcctgggttcaaacgattctgctgcctcccaggtagctggaattacaggcttgcaccaccatgcccggctaatttttgtgattttagtggagatgggggtttcaccatgttggccaggctggtcttgaactcctggcctcaagtgattcacccacctcggcctcccaaagtgctgggattacaggcgtgagccactgcacccggtccccactgtgagagtttttgggtgtattcctttcagtttgatttttcccattccacaaggtaaacactgccaatcagaacaccctttctctggaggacttggaattttcctgccccttaaagtaaatctgccagttattaacacatttcatcttatttaacacttcaggtgtccgctatgaatcaattattgacaggaaaatcttcttttaactggtagggaaactcttggtaaatatctcctctaaagacttgcggatgtaagaaaaaagtattttgaaatctttattcaggagtagtgcatggctagaggacacatgaggagtgacttactgtagaatcttctgtaattttggaattttaaatcatatatgtcctatttaaaaattaatggaaaattggaggaaacagtgtttggagatcttttgactttaaaagtacaattctgtttaaacctgtgtattttttagagtggtaaggctatcgatatttcgttgtaggtttgttctctaattgttctttatttcatttgagcatttaaatattctgatcttgtacacaagatcagttggttagttacctaataaaattttaaaatagcactcaacagtcttttaaaacgttagtcttctttttttcctctaacatcacaacagagcagttttcacaaagatgtcaactaaaaaatttctaaaatgtgttgagctgatttctttagatcttaggtttaatatttttttctgaggtaatggtttttatctctcagtagctaggattcatttctgtttcatatctcatcatatgaactagaatttcttgaaccatgtaagattataacttattttcaacagtgcttttaatagaaatatctaatcatggtactagaaaacagattttatcttgtcaacaaagtacccttttatttttgaaagaattttaaaaattaaaatgagttttaaatattatccttttgatatctgtcatagtaacaacactttatgagaggtgtaatagaaatagaccttctatccttgaaactttcttgtagtcctggggttaactctatctagttacttttgatttgaaaaagtctatttgtgaatattttatttaggatcttcacatcaatattcacatggaaggatagataatagttttatctttgtttttggtctttatgtcatctttgtgttttttgataattaattttgtatcaattaattaatgccacttatttttctgcatttttaaaaatataatatgggaattaatggttccttgaaagtttgaaagaattctgcaatgaaataatctgtacccaggtcttttttctgggtactttttaatgactgtgctcaatctttctttacttagttcatttttttttttttcagatctgtagaaacttccagtgtgtagatgcttctgttctgaattatgactgtgatgttcagaaaaagtgtcatggacatggggtaggtaatgttttcttttggcttgttcctgaaagtagtgctaaataatgagaaatctcaggactagatgagagttcccaggattttcagatgttggggaatttagattcctgataaaattttcattcttaaacagtgtcagtaagcttgtatgaatttagtcctttctcttggtttccattcttgagttgatgatatagagcaacattcacaattaacaaaagtggtattttgattgttttgaaggtatgtaatagcaataagaattgtcactgtgaaaatggctgggctcccccaaattgtgagactaaaggatacggaggaagtgtggacagtggacctacatacaatggcaagtaatatagaagaaaattagtgtgatctcccagtggcccaaggcataaattgggcatcctcgtacctctccctcacttcccacatcagttatacatttaattatgttgattcagcctcctaaattccttgtgactgtttccatttttctcatccccatttattactttcaatttcttgcctggacatacatcatagcctcttatgtaggctccctatttttcatcttgcttcctataatccatgtttcactctacattacagtttcagtgttttcctacaagaattcagttttgattttgtcagcgtcttgctttaattcagtgcgtctgcattgctattagaatgaagtccacaactccttaacatgggttaaatgccctgcatgacttgcccctagcttgcctttcaagcctcatttcactatgttgaagacatattgtaacttctttgatttcctgtactaggctactatcttttacctgtgggctttcataccgtattattttcacattgttggcccttggctaattgctatttaggtttcagattatacctcattttctaaagaaagtttcccctggctgcttaaatctaaattatcatttccttctattgcttttctagtactgttagcactatctgttagcactaattgctatactaattactgatttgctttttaaaattccctgatagaccatgagctcccagtttatcggtatctttctagtgacatcatatgctttttttctcttgggtaactaccagctagaatgactagtcatatagtaggtgtatgttaagcttttaaagaaactgccaaactgtttcccaacgtggctataccagtttacatccttactagctgtatatgagagaattcccccaatttccccacatcctctctaacagttgctattgtcagtctttttaatttttagccattccagtaggtatgtagtggtatttcagtgtggttttaatttgcatttctctaattactaatgatgttgagcatcttttcttgtacttatttgccatctacatatcttctttggttatgtgtctgtttaaatcttttttccagtttttaatggattgtcttaatgagttttgaaagttctttgcatgtcactgattcaagtattcaagttctttatgaaatatgtgccttgtatatattttctcttagtctgcttactttgggtttcatttgttctttttctagtttcttaaggtggaggatgaggtcatctttttttttttttctgatacagacattttattgctatcagttttcctttaattcagaaattttgacatgttatacctccatgttcattcagttctgaataccttctaatatgctttttttttctttgacttacaggttatttagatatgtgctatttcttttgaaatacctgtggattttttagttatcttaatgttactaatttaaattttactgtagcaagagaacatattgtgtatgacttgaatccttttttttttttaaacttgtcttgtagcccagaatgtggtttatcttagtaaaagttctgtgtacacttgaaaagaatgcgtattctactattcttaggtggaatattctgtaagttattagttcatgtcagttaataggtagtcggatctttcatatccttactgattttctggtctacttactctgtcagttattgagaggaatattgagttctttggctataactgccaatttgcctatttctcttaatagttctatcaatttttgctttatttattatgatgttctgttattaggtacataaacacttagaattattctatcctctttgtaaattgactctttatccttatgaaatagccttctttttccctagtaatattctctgccctgcaatgagatattgttaatatagctactccagattcctattaattagtcagcatggaaaatcttttcccatccttttacttttaatttctttatatcatgctatagtaattagtacatatagttggatcttgctttttatctaatctgccattctctgtctttcaattaagttgtttcgataatttatatttaacttgactattgatgtgtttatgtttaaatttactgtcttgatattttccatcagtctccttgtagtgatattgtaacacttcagtatatttccatttctctcattttgtgccattgttgtcacatgttttacttctactaatgttataaatcccacaattcattgttactcattttgctttgaacagttgattatctttcagagacttaatggtagaaaaagtctttatatttacccatataattaccatttctggtgtttttcatttatgtaaatttgcatttcaatctgatttaatttctgcttgaaggatttccttttacatttcttataataccagtgtgctagtgacaaatatttttagcttttgtatgtctgaaaaagtctttaatttgccttgctgcttgaataataatttaactgggcaaggattttgggtgatagttttcctcccgttttacttctaaggatattccttgtcttctgacttgcattgtttttcctgaaaaatctgctatcatccttttctttgtatataatgtcttccgtatatgtctttttctaatctctggtcacttgtaatgttttgctctttatctctggtttttatattgtgccttggtgtagttgggattttttgagctttttggatctgtgcttttatagttttcttcaaatttggaaaatttttggccatcgtttcttcgaatatttttttctgtcttcctctttctcctcatccaggtcctccaattttatgtatatttggctgcttggtgttatttcacatgtcactgattggctgttgattttttatttttgtttttttttcttaaattttaatttaactttactttttttgagacagagtcttgctctatcacccaggctggagtgcagtggtatgatcttggctcatggcaatctctgcctccggggttcaagcaattcttatgcctcagcctcctgagtagctgggactacaggcgtgtgccaccacgcctggctaacttttgtatttttagtagagacagggttttacgctgttggccaggctggtctcaaagtcctggcctcaaatgattcacccacctcagcctcccaaagttctgggattataagtgtgagccagcatgcctggctggctgttgatttttaaaaattattccttattctccatgtttaattttgagtaacttctgttactcttcaagtttacatttcttgtgtgaagtctaatttgccattaacttgatctagtgtgtttttcattttagacattgtagtttttatttctggaagttccatttgtttcttttatatatctttcatgactctacataagatgctcaatctttacttttttgaacaaatagaatacagttgtaataactgctaatgtccttgtctactaattctgtcatatgggtaatttctcagttttgatatttttccctcttttattttctgtatttttgtaggccttatacatttttattagatgccagaagttttaaatcctactttgtgggttattggatatttttggatttctattgatgaggtttgtactagtatgtttgagttacgtcgacatagtttgatccttctgggtcttgcttttaagcttttaaggcaggacctgaatagcatttagtctagggctgattctgcttcattactgaggcaaaaccacttctgtttatcctgcttagtaccacgttaattatgagatttcccactgaattataggagcaagtgctcttcctagtcctgtgtgagctgtggggcttatttccaccaatcttttcacatggttctttctccagcttcatgtggtctccttacatgcatatatccatcagcaccgatgcagatctttcagctttttctctgtagctctcttccctttggtactttgcctaggaactgtagctgccttgccctcttcagaataccagctccatctctttaactgagggagaccactgggttttgctttggtgcccacacccgagtgtctgttaactttctttaggcactaaccttggacaattctaaggctcacattttttttttctgcctctcagggatcattgctctttgttgcctgatgtccagtgtcttgaaaactgttgtttcatatattatgtctggttttctggttattttagctggcagagtaaatctggtccctgttattccaccttggctataactggaagtcagaactatggattttaatggctgtgtatcatttcatccagtggatgtgctataacttcacttagctgttttctaattatttgacatttagattgtttctaaggttttgataactcactgttaacattgtagtgtacatgttaatgtgtatgcatttttccaattgaagaatcaattgccagtaatgagattagtttgaagagaataatcctttttatggttcttttaggagtaaaaattcctaataaatgatacatttgtgtaatgccactaacagtgcgaaggtatcagtttcaaaataatcttgccagtgttgaatgctttaatttaaattttgtgtactcattagtaagtataaaatgatatatgaagcttgctttaattttttatacagttgaccgttgaacaatgcaaaggttaggggctccaactccctgcatagttgaaaacccatgtgtaacttttggcttccccaaaacttaactacgaatagtctgctgttgactggaagacttaccaataacataaacagttgattaccatagattttgtctgttatatgtattatatactgtattattataataaagcaagctagagaaaagcaaatttattaagaaaatcataagagaaaatatatatactattcattaagtggaagtagattatcataaagaccttcatcctcatcatcttcctgtagagtaggctgaggaggaggaggaagaggagaggttggtctcaggggtggcagaaacacaagatagcctgcatataagtggacctgcacagttcaaacccacattgttccagggccaactgtattttgattttcagttgggataaatattgtttcatatagttttatacaactttttttttttttgagatggagtctcgctctgttgcccacgctggagtgcagtggtgcaatctcggctccgcctcccgggttcatgccattctcctgcctcagcctcccgagtggctgggactacaggcgcctgccaccacgcccagctaatttttttttgtatttttagtagagacggggcttcaccatgttagccaggatggtctcgatctcctgaccttgtgatccgcctgcctcggcctcccaaagcgctgggattacaggtgtgagccactgcgcccggccagttttatacaactttttacagaaatttctggttcttttacaaacttaaaattatgaatcagtttaccactcccgtttatatctactatattgtttctcaaaagaacacagaacagataaaatacttaaagaatttgtaaaagttctaatgaaacttaaaatctagaaggcgtaaaaataagattgataaattcaactatacaaaaataataaacttttccgtggagaaaagcatagtgccataggttaaaatggggaaaatatttccaacttgtatcatggacaaagctaatctctctaatatataaagaacttttagaaattaagaagaaaaaagcaagagtccagtagaaaaacagtcaaaggactgagcagaaaaaaataaataatgtttccttaagaaaaaagtgaggccaggcacggtggctcacgcctgtaatcccagcacttagggaggccgaggcgggcagatcatgaggtcaggagttggagaccatcctggccaacatggtgaaacctgtctctactaataatacaaaaaaattagctgggcgtggtggcgcatacctgtaatcccagctactcgggaggtggaggcagcagaatcgcttgaacccaggaggcagaggttgcagtgagtggagatcgtgccattgcactagcctgggcaacagggtgagactccatctcgggaaaagaaaagaaaaaaaaattatcaactcatagtataaaaaaatgtaaattaaaattctataagagaaaatttttcacctgcctggttggcaaaaatccggaaatttggctctgtgggtgaggctatggggaattcttatatattgcttgtaatattcttataaattgtaaccattactattgaaagacaatttgacaatacctaaaagaaatgatgaatgcacttatttattgatacagcatttctgctttagggaaattattctgtagttattatacctgcactaatatgatacaacatatgtgcaaggttattcattatagcagtttttttggtagtagcaaaagattggaaaaatataagtgtttatcagtagggtacaagttaaataaactctagaacatcttcacaatggagtttcatatagctgtatggaaaacgaggaggtccactatgtacagataagtggaaaaaaactgatgcaccaaatggtatataaatagtatgctaccttttgtgtaagaaagtgttgacagtagaaacgtattttgttcttgattgtttgctcgaagaaatactgtaaggttacagaagaaactaataaaagtggttatttttgtgaaggcagaagtaaagcggacaggaatgaactttgtggaagacttctcaatatattcaattaatatcagtttgatttttgagtaatgtgaaaattaatgtaaagtgtttataatcatctagtattttctgcctagtatgagtttggtgactgttgatgtaaaattcttctctctagaaatgaatactgcattgagggacggacttctggtcttcttcttcctaattgttccccttattgtctgtgctatttttatcttcatcaagagggatcaactgtggagaagctacttcagaaagaagagatcacaaacatatgagtacttagatttttttcttttaattcctatattaaatatatacatacattttctgagacagaatctcgacttccctgggctcaggtgattccccctgcctcagccttccaagtagttgggattacaggcacaccaccacacccagttaatttttatatttttttgtagagatggggtttcgccatgttgcccgggctggtcttgaactttttgaagccatccatctgcctcagcctgccaaagtgcagggattactggagtgagcctccacgctcagcctatattaaataatttataaagtattaatgctgatagtcatatcaccagagattggtaatcctctaaaatagggttctaagttatttctctgaccttttgacatgattagcatgggttgaaaggtggtggtgaccaagccacctcttttaatggggaggagaaaggcttatgttggtcagcctttaggctgctgaaagtgaccctcagggttcattttgcttaacaccaatttctgatagaggactaagtagatacttcgtatcatacttccaactgaccagtctatgcaaataactcccccatctgcatttttgaagtttgagttccataactacagctatctttcatacatctccactgcactgatttgctgtcacttcagcatgtctaaaacttacctattacctttccagccaatccattcactacccttggatttcctaatttttaaaatgactacttggcaacctgagaatatgcttttactcttctctgattttaggaagacttgagaaaagttagggaacattggcctaattgaccaaatttcacaatttcttaaaatttcagtttaattataaaatgtggttagtaatgctttctaataccataaggattaaaaatacgtgaaagctgttaaaatgccctaaaaatttaaaccgtatcatgattatcatccccaccactaccaacatcattattctgtatttgggaaaatgcaaaatgtgtgtaatatttcatgtagaaatgtttttatcttaatttagatcaaaagtaattgtatctttcaggtcagatggcaaaaatcaagcaaacccttctagacagccggggagtgttcctcgacatgtttctccagtgacacctcccagagaagttgtaagtataaaatgaaaaattatttttctttactgtattaaaggatcaaatgcttaaggattaaaaacacagttatatagctatagctagaaacatagataccttcttaagaattcaagagtattgtaggtggtccctgagttttttgtttttgttttcgagacagagccttgctctgttgcccggggtggagtactgtggcacaattgcgtctcattgcaacctctgcctcccagtttcaaatgatttcgtgcctcagcctcccgagtagctgggattacaggtgtgtaccaccacgcctggctaatttttgtatttttcatagagacggggtctcaccgcattggccaggctggtcttgaactcctgacctcaagtgatccacccgccttggcctcccaaagtgctgggattacaggtatgagccactgtgccctgccccctgagttctttaaaggaaaaccagcggagtccttggctcagaggacacagaaaaagacagctggacattaggaatgccttgcctagcaaccaggattgggaaatgacatgggacgtatgctatcactgcttttttctgtgtctgctcttttcctattttcaatacctgtctccatctccctatgggatgttaccaaagacctggtgctgagctcttggatcggcctaattgtctaagctgtaggactgatagtcactgttctgcaagtgtattagggagtgtttagatcatgatatacttttattgagtgtttagatcatgatatacttttattgatctgcatgtatccctaagcaatatgtaattttttaatgttttaaaacttttaagaacgttttatttgataatttgcacatatatctgcaacctgtttttccccttaatgtcactttgtgatttatctctatcgatagatatagctgtgattcattcattttcactgttgaaaatgattagaaatccttcattttttaatatatttatacacacacacacacacacacacacaatctccctattccaccccctttatctttataaaaaggagacaaaaatcgttaggccctttctcctcttaaccatgtatcttggagatttttccatgttgttatgtatacaggatggccacaaaggccatatgcatgctagttcaaaattatctgtatactcttcttcatcattgccatatatgtatatatttcttatttggttttggcaaaatatatataaaatttgccattttaaccattgttttcaagatttttttgtaaatttaacagtagtggtaaaaaaaaaacccactaatatttaccatcttaacaatttttacatgtacagtgcagtactcctaagaatatttacctatgttttcttttagtagttttatagtttcaggtcttatgtttaaatctttaatccagtttgagttgatttttgtatatggtatgaaataccagttcattttcatttttcttcatgtggatatgaagttgtcccaacactattaattgaagtgactgtcccttcttcattgtgtattcttggcaccttcgttgaagattagctgaccataaagttgtggatttggggttctctattctgttccatttgtctttatgtctgttttatgccagtagtatgccattttaattagtatagctttgcagtatattttgaaatttggtaatgtgatgcttctagctttgttctttttgctcaagattggtttagtgattctgggtcttttgtggttccatatgaattttagtattttttctattgttacaaaaattgtcattggaatattaatagatattgcattgaatctgtagtttgctgtggttattttaatattaactcttccagtcagtgagcatgggatatctttccatttatttatgtcttcaattcctttcatcaatgtttcatagatttccttgtacagatacttattttttgtggttaaatttattcctatattatttatgtatgtatttttgatgtcattctaaatggaattttttttctggatttctttttcagatagcttgttgtagtgtatagaaatactagtgattttcatatgttgattttgtattatgcaactttagtgaattcattagttctaacagttttttggttgactctttagggttttctatataaaagaccatgtcatctgcaaacaaggacagttttacttcttcctttccaatttggatgtcttttatttctttttcttgcctaactgctctggttagaacttctagtactatattgagtagaagtggtaggagtggacatccttgtcttattcctgatcttagaggaaaagctttcagtttttcattgttcagtatgaagttagctgtgggcgtgtgatgtacagcctttattgttctgaggttcattatttctttctttctttttctttgtttttgagatagagtctcgctctgtcacccaggctgcagtgcagtggcacgatctcggcttactgcaacctctttctcacaggttcaagtgattctcctgcctcagcctcctgagtagctgggattacaggcatgtgccaccctgcccagctaatttttatatttttagtagagagacagggttttgccatattggccaggctggtcttgaactccggacctcaggtgatccacctgcctcggcctcccaaagtgctgggattacaggcgtgagccaccatgcctggcccagtttgttctttctatacaaatttgttgagagtttttatcatgaaagaatgttgaaatttgtcaaatgcttttccctcatttcttaaaatgatcacatggtttttgttagtctatgttcttcatttctgttttttgtttgttaatgttgttatttattgatttgaatatgttaaaccatcctcgcatccccagaataaatcccacttggtcattgggaaatatccttttatgtgctgctgaattcagtttgctagtattttgttgaagatttttgcatctgtgttcataaaggatattggcctgtaattttcttttcttgtggtgtccttgtctggctttggtttcagggtaatgctggccttgtaaaatgagtttggaaatattccttcctcttcaagtgttgggaagagtttgagaaggattgcattagttcttctttaaatgtttggtagaattcatctgtgactttatcaggtcctgagtttctttaatgggagactttttaaagttactaattcaatctccttacttattattgatcttttcagattttttattttgtcttgattcagtctggataggttgtatgtttctaggaatttatttttttctaggttcaatttgttggtgtatgattgttcatagcagtctcttataaaactttctatttctgtggtatcagctgtaatgtcttctctttcatttctgattttgattcctctttctttttttcttagtctacttaatggtgtgttaattttatttatcttttcaaaaaaccaactcttagttttattgattctattaatactatttttccagtatttcattcatttttgctctgaacttcactattccctttcttctactaactttaggctcagattgttcctctttttctaggtcttgaggtgtaacattaggttatttgagattttttaaaaaatgtaggcacttattggtatagacttgctataaacttcccccttagaattgctttttctgtgttgcatacattttgttatgttgtgtttctatttttgttgtctcaagatatagttgtttcttggtacacattggggattggttccaggacccctacatatagcccaatctgcctatactcaattaattctgttggccctgtagaacccacatataggaaaagttggccctctgtatatgtgggtcatgaatactgtattttcaatctgtgtttggttgaaaaatatctgcatatagatgtacctgtgcagttcaaacccgtgttgcttaagtgtcagctatattttaaaatatttctttttatctgtcattgaccaagtgattgtttaggagcatgttgtttaattttcatgtatttgtgactttcctaaatttcttcagttattgattttgagtcctaatattgtagttggaaaacatacttgatgtcagtcttttaaaatttgttaaggcttgttttgcagtttaacatattatttgtcctggagaatgttctgtgtgcgtttgagaagaatgtgtattctgcttttgttggatggaatgtgtctattagatctgttttgtttaaagtctagtttgagccaaatgttttcttactgatttgttgtctggatgacctatctgttgttgaaagtgaagtattgaagtttcctagtagtattgggttgctatttagctctctctccagattaattaatattcgctttatatatttaggtgctctaaattggctgcatatgtatttacagttgttatatccttgtgatgaatcgacacctttaccattaatgcactttttcatctctgtttttattgtttttgatgttacatcattttgtctgatgtaagtattgctatccttgttctcttggtttccatttgcacagaatacttactcatatttaaaagaattactgatagatggggacttactattgctattttgtttttgacccttccttcttcccttgctgcattcttttgtatttctttttaattaaaaaaatcaattatggatacataatagttgtacatatcacatggggtacatgtgatattttgaaacaagcatatagtgtgtaatgatcaaatcagggtaattgggatagtcatcacctcaaggatttatcatttctatgttaggaacattccaactctactcttttagctattttgaaatatacaataaattaatcattttctttgtttttttgtagtaatattttgattctcattttcctttgtgcatattctatagcacatatattgtgatatctttgcaattacataaaatattttataaatttatagcaatctattttaaactgattacttcaatcacaaaaactctacccctttatatttcttcttcttccactttatgtaactgatgacacaaaattacctctttttatattgcttatcattaacacagattcattactttttatgctatgcttttaacattctaacaagatttaaaagtgattttcacactcacattacagtactacaggattctctgtctatacacttaccattattatcgagttttatattttcatatggttttgtgttgctatttattttcctttctcttcaccttttttgctcctctgccactttgattttgaatatactagtctttgagtccactgatgctttcttctgcctcatcatgtttgttgttgaatccttttagtgaatctttcaatttagcattacagtagttttcagctccagaattgctgtttggttcttctttatagttcctgtctctttgttgatattctcattttgttcatacatcattttcctgatttcttttagttgtccatctgcattctcttttaattttttgaacatcattatgatggtaatttttgaattctttggtaatttatatatatctgtttccttagggtcagtttctggagattgagtttgtttctttaaatgtgccatgtttctatttctttgtattatttgtcatttattattgggattttggcatttgaagaattagctgcctttctcagattttgcagccttgttttgtacaaggaggacttacgctactcagcctggctagagattctggtagcctctcaaatcttttttggggatgtgtcctctgtgaggtttttttctgcagtctcctaattgtggaggtttgctagtttctactcaagagcacccccaggtgtctgtgatactgtggtctctctgactttttttttttttttgagacagagtctttctcggttgcccaggctggagtgcagtggtgccatctcggctcattgcaacctccgcctcccaggttcaagcaattctcctgcctcagcctcctgagtagctgggaatacaggcatgcgccactactcccagctaatttttgtattttttagtagagatggggtttcaccatattggccaggctggtctcgaactcctgacctcgtgatccgcccgccctggcctcccaaagtgctgggattacaacttgagccactgagcttggcctgttgtctagtattttaagtcttttttttaaaaaaattctacaatatagatatgactattgaattatgaaatgtttgtttaggtttgtgaggccatacaccaattaaattaattaagaggatggactgtgagccaaactgcccagtttgagtactgcctttgtcactttataagctgtgactttaggcaagattctcaaactctttctgtacttgtttcctcatctgtaaaataataatagtactaatcacaaatgacttttgtgaaaatcagagggattcgtatgtgtggagcactgagaagtgcttgtggcacatgtgaagtgctctgtgagctttagctattttcccatgtgttgattgtctgctttcaaccttattgaatctcagcttatttttctgatatatctacttcaactgggtatcttttagaagttcccttagcgaaggtattttggtagtaaattctgtcagtttttgtcttttccggatgtttttggctgacagcttttttttttcctaagaactttaaatagactatattttaacatcctttgttgcaatttaaacattgtctgttactctaattgatgctgtagatgatatcttttccatgtggctttttcttctgtatctttagactatttggtgtagatgtggacttaaaaaaactcctttgccagtaaatagacttccggagttgatttacatttttcagttctagcaaattcttagcaattatttctttattgcctctgtctcattatctaattaactctttcatgcatttcttgcatgttagactttttactatctctgtttcttaacctctctttggtatttccaatattcttgtgtattccattctgattatattggatctaccttctattcactaagtctctactaaactatgccaaatctacttaaccaactcattgaatatctcatttcactagttttatagtacatttaattcctgtagttctacttagttctatttcgaatctgcctggttatttgtgattgtttgttatagttttattatctgttttaaagcttttatttcttaaagcatattcaaacacctaatttttgtgctgtatctgatcattttaatatgtatgcccttggtgggttctcaggtttgttatttctgctgactctcgtgatggctcatttcttagtgcccttgtgatgttgattgtaaactcaccttctttggaactttatattggaaataaatatatttgaatcctgaattatagtgggttcctaccgagagtatttttctttgccagatgcttgggggcatggtcaatctttgatgtctttaaactgaaatttttgttgatatatatatatttttttgccacacaaatgttaggaactctggtccccaaactcttatgaggatgggtgtgtggtaagaatttctccatggagactatttttttagttccccatctatcagcaccaaggcagtatcaccacgggccttccttgaggcaggtttttgtttttctagttaacccatggggataccacccttcatatgtctaggctttgtatagggccttgtattcaccattccatccagctcaggccccagcttttgcctcctttatctatgggtcactgaaaacgcatactgccacctgccaaggataggaagatttccacaggacaaaggcaactccgtagtttggactctttcatacgttcttggtttttttttggcctgtaagatgtttcttacttcccaccaacccagccaagtgtttcaaaataccttttaaatattttaggcagcattttaggtgtactgtactgggaagtttcctctggacatttggtccactatttgcaagaagtgaacatgtacttcattgtttttaataaccgcatgctgttccctcttataaatttaccagaaatttaaaaacaggttgtttccagtcttataccataaaaaaatgtggcaccaagcatccttgtaaatagatctttgcatacatttaaaagtatatgtcagataaatgccaaaaaagattaaaatttttttaaattaattttagttttaattggcaaatcatagttgtatacatttatggggtacagcatgatgttttatgtaaacaatgtggaagtgattaaatcaagctaattaacatatccagcaccttgcttgcttgtaatctttagcttgttttcattaatttatatttaattgacaaataataattgtgtatattttggggtatcgtgtttgttttttttttttttttttttttgagatggagtctcgctgtgttgcacaggctggagtgcagtggcatgatctcggctcattgcaaccactgcctctcgggttcaagcaattcttctgccttagcctcctgagtagctggaattacaggcgtgcgccatcatgcccgggtgatttttttgtagagacggggttttgccatgttggccaggctggtcttgaactcctgacctcatgtgatccacctgcctcagccttccaaagtgttgtgattacaggcgcctggccacaatgtgatgttttggtctatgtataccttgttgtaagattcagtcggctgggcgcggtggctcatacttgtaatcccaacactttgggaggctgaggtgggcggatcatgaggtcaggagatggagaccatcctggctaacatggtgaaaccccgtctctactaaaaatacgaaaaaaaaattagccaggcgtggtggtgggtgcctgtagtcccagctactcgggaggctgaggcaggagaatggtgtgaacctgggaggcggagcttgcagtgagctgagatcgcgccactgcactccagccagggcgacagagccagactccgtctcaaaaaaaaaaaaaaaagattcagtgaagctaattcccatacccatcacctcaccacattgtcattccaaaagtggacttgatccctttagagtgctgttcctatggcttgtggaaagggatggagacattttgttgcatttttcacccattttcacagtacatataaatcattctgtggggaaaaaaattgcagatgatagaccacctgttctatggtagaagccagagggtgctcaaggtcttcaccaccactgtgcattctctgccagtcatagaactttaggagttaacagtagatagtaaagaacatcttggtcaaggtcacttcatcattgatttagtaattccatctgatcattcctaacgtcttatagtgtaatgtgatatgtgaaaaatattacttttactttcttatttgaggctaagttatacagtttcactttgttgtaaacttcaactacttcatcaaggaaggatataatgaattccaaaaccgaggattctagctgagtggtttttatagtattagttagatactgtataggtttggcaatacattttggaagattttatttaaaatacattgacataggaaatatgttaccttctaactaatacagttggtttgaaccaagatcttagtactttggtattactgaatttaaaaaaataccttaaaagaattaagtattccacattcagtggtaaagatatgtcaaataagcaaaatatttttgactgtcagcattataaataaatacaggttgagcacccctaatctgaaaatccaaagtgctccaaaacccaaaactttctgagcaccaacatgatgccacaggtggaaatttccacacctgccctcatgtgatgagttgcagtcagaatgcactgtttagtacttatatgtgaataaatctaagaaaatgattgcttaccagtagtatataaattcagagtcaggagtgatggtgagccaaacaaccacagattgtccacatgaggggctgagagagtaacacctttgctttctgatggttcagcatacacagacattattttatgcacaaaattatttaaaatattgtataaaattaccctgaggttatatgtatgaggcctatatgaaacatcaatgacttttctgtttagacttgggtcccgtccccaaaatatctgattatgtacgtgcaaatattccaaaattggaaaaaaaatctgaaatttgaaactcttctggttctaagcatttctgataaggaatattcaactgtagtctgtttattgattttaaatatgtagatttcttctatttagaaatcatatttatgagcacatagtggtaataaccttattttttttttctttttagcctatatatgcaaacagatttgcagtaccaacctatgcagccaagcaacctcagcagttcccatcaaggtcagaagaaaatttgcttagattttttggccagaataaaacctaggggttaatgtctaataatttcccctgtattttaatgtaatttagtgaaaggtatttattgtcaacagtttacaagaatatgatttgcagaaaggttttaaaataactttatataaattttatcatattggtacagggtcaaaatgaaatattaaataagcttgagcaagacagattctgctgccacagctttcatgtgcatacgatttagaagcaagggcctttgagataaccagcagtaggaaaccagatgggttggaacagccttcccgtcaaaaacagctaaaaaagctggacaatataagaaaatatgtgtttgaaggcatagaagactaaagaagtgaggaattgtgggggtaaggtcaggagaggaaggaaatctagaaatgatcccagctttgggggccacttttccttcctagatgagtttacctgttctgacaacagagaggctaggaagctgaggagagctttctacaaactcacagggcagaggggacaaaatttagaatcctgccaaagaggaggcaccctggcaaacatctcagggtctgtgctgggacccagaagtaagagtgaactagaccttcaactgatttctacaatttcttatgttttgctcatgatcaaaaaaagccaagtgtaaaagaaaagaaaatatgactaaaaccaagaaacaatagaccatagaaacagactgagatggtatccagttaatagacatggactttaaaataactatgatgtcatggaattaaaagtcaagattgagaatttcagcacagaactaaaaactaaaagaatcaatgcaaattctagaactgaaaaacacaggaactgaagtgactcaatggatgggcttaaaatcatcaggaaggaagataatttattacttcattttgtatcacataaaatgcaaatgcatgtgaccctcccatcccctagaagtctttcaaattacaattgcgttgcaactctgaggactatcttcatatgtaatctttattatacagtaagaatacattgaaatccgactgaggatcagggaaagagtatataaattgtgagggaaacattcaccaggtagtgttctagtgttactggagtagaggtgtactagaattggatgatgaggttaggagcgggtgtccacaggtggaagtatgaggtttgagatggacaggtatagaagtcataacacttttaattctcagagtgaatctcatgttgagggagctataaacagctaggtttacaccagcagtaatttgctgccctcaaattctaacagcacaggcaagtgcttgatcacttagtgtactcacttgtcttttacagtttatctttaccatttcatgtgctttttttttttttgaaaaaacatgtaaactagaaccttcatacaacattgttgattatggagtaatattatttaaagtagttattccattttagactctaattggagccttttagccattgaatatcaccctaatactgatctcagaatgtacagtaccctttcctgttgtcagagatgttgaggatggtgttatgttgagcttgtaatgaatatggcattatttcacccagtctaaacactctattaactatctcttttcccctcgcaggccacctccaccacaaccgaaagtatcatctcagggaaacttaattcctgcccgtcctgctcctgcacctcctttatatagttccctcacttgatttttttaaccttctttttgcaaatgtcttcagggaactgagctaatactttttttttttcttgatgttttcttgaaaagcctttctgttgcaactatgaatgaaaacaaaacaccacaaaacagacttcactaacacagaaaaacagaaactgagtgtgagagttgtgaaatacaaggaaatgcagtaaagccagggaatttacaataacatttccgtttccatcattgaataagtcttattcagtcatcggtgaggttaatgcactaatcatggattttttgaacatgttattgcagtgattctcaaattaactgtattggtgtaagagttttgtcattaagtgtttaagtgttattctgaattttctaccttagttatcattaatgtagttcctcattgaacatgtgataatctaatacctgtgaaaactgactaatcagctgccaataatatctaatatttttcatcatgcacgaattaataatcatcatactctagaatcttgtctgtcactcactacatgaataagcaaatattgtcttcaaaagaatgcacaagaaccacaattaagatgtcatattattttgaaagtacaaaatatactaaaagagtgtgtgtgtattcacgcagttactcgcttccatttttatgacctttcaactataggtaataactcttagagaaattaatttaatattagaatttctattatgaatcatgtgaaagcatgacattcgttcacaatagcactattttaaataaattataagctttaaggtacgaagtatttaatagatctaatcaaatatgttgattcatggctataataaagcaggagcaattataaaatcttcaatcaattgaacttttacaaaaccacttgagaatttcatgagcactttaaaatctgaactttcaaagcttgctattaaatcatttagaatgtttacatttactaaggtgtgctgggtcatgtaaaatattagacactaatattttcatagaaattaggctggagaaagaaggaagaaatggttttcttaaatacctacaaaaaagttactgtggtatctatgagttatcatcttagctgtgttaaaaatgaatttttactatggcagatatggtatggatcgtaaaattttaagcactaaaaattttttcataacctttcataataaagtttaataataggtttattaactgaatttcattagttttttaaaagtgtttttggtttgtgtatatatacatatacaaatacaacatttacaataaataaaatacttgaaattctcttttgtgtctcctagtagcttcctactcaactatttataatctcattaattaaaaagttataattttagataaaaattctagtcaaatttttacagatattatctcactaattttcagacttttgccaaagtgtgcacaatggctttttgttaataaagaacagattagttttgaagaaggcaaaaatttcagttttctgaagacagcatgttattttaacaatcaagtatacatattaaaaattgtgagcaatctcaaatgaaggtccatcgtttcattttaaatctctaaatgaattcatataagactcaaacgtttgtgctgttcactcatgtagcctcagtttttgcaattgtgatgcatatcactgaaattttacagttggtaatgtattaactatgtaacttaacacttggaattaaatagttctttggatatttgactagttaagtttttaaaaagactattggatctgaacttcttttatatattttttaatatgctttatgttttttacttacttggtcatggatgccacttcaaaatttgaaaatattaaaggacatcctttctttcttcaaaaagaataaataagggtaaattatatgcaagtttgacatctctgtttgactctgtatgtcaaactgaccttgttcagagtattgcattctcgctttctcctgtgtctgtaaccatagagttaagcacaatttgggttttctaaactcaaatcagattttat

SEQ ID NO: 105 - DNA, 23101 bp, Homo sapiens
cctcctgcctccggccctgggtaatatgcatgaagtatttagccaactggcacctttcgaggtgcgtctgctgctgctcagtgtctggggttttctccgggagcatgggcccttgcctcagaagttcatcttccaatcagagcggggtcgcttcattcgggacttctccagggagggtggaggtgagggtggaccccatctggctgtgctgcacagtgtcctccaccgcaacatcgaccgcctaggtcttttctctggccgtttccaggcaccttcaccgtccactctccttcgacaggggacgtagccttttcttgctctggaagcccagggaggttgagcagtgagagagggaagggactaacgtgctccggaagggtggaggtttctcttctaagtccttggtctaaagagcgctgtcacttttttctctcccacttttttttttctaaataaaatttgccaacttgagaaaaccagtccagtgcttctgtcatgctgagagcgtgcaaagtctgacagcgcctggctctggacgttcccgcccctggcctgaagccccgccccctgcgataatttggagtgcgcactctaccaatgagacagctgcccggcggcgctcaggtcgaaccaatcataaggccggaaggggcgggaactaggatacgtggctgagcgcgcgcgatggggcgggaggtttggggtcaaggagcaaactctgcacaagatggcggcggtagcggcagtggcggcgcgtaggaggcggtgaggagcccggaatctgggggcgcgcccgggacgcccccagatcccccaagtcccattccactccttcctgtgtgtctcttgacactctgccacccccggcctcgtgaggaacctttgttcctctggaggcggcctcagacgcctccggtctccccgtggtagatccgagcgacgctgggggccttgcctgtggggctccgggctcccgcccggcggtttagtaaagccacagctgtgcgtctttcttggtcttggccgctctcagccgccgccctcctttggctgcttgcggcggtcaacgtcgccgcccccttcctgcagtgcgcggggtcgtcggggcgggggaaaagatgcggcctggcctcggggaatgcagcctgcggccccgcggcccctcggctgagctggaagcaccgggccagcagttaagcctgtactacccttctggctctaccctgtagagctccgaatcctcctctgcccttgtcttcacgtgagcaccagctctggcttagttcagtgtccacggtcgctgggcacggcccagggtccagtaagctcacggcgtggatggtgttgctcaaacacaacatgtaatcgaatggcttggtccacgctctcgggtttatattactggggaaaaaaaaagattcgaaacatatcaccagtgccacaaatgtttactaggacctaacggatatactggggtggggtaggcgtgtactctccaaagcgatgaagaaagcgtggatcataaactcagttccctcggagcctgtgatctgaaacaataaatgcgtgcaacttgccctgcagcttattcctgactttggcctatgaacacctctcttggggtggtcaaggccgccgtgaattccttagggccctccaacaggtcatatctgaaagatgctttaggaatcctatctccattggcatctttccgaaccaattttacagactgtgcaaatagggccccagagggtatttaactcactgtacgtcttttttttttttttttgagagacagagtctcgctctgttgcccaggctggagtgcagtggcgagatctcggctcactgcaagctccgcctcctgggttcacgccattctcctgcctcagcctcccgagtagctgggactacaggcacccgccaccacgcctggctatttttttgtatttttagtagagacggggtttcactatgttggtgaggatgatctcgatctcttgacctcgtgatccacccgcctcggcctcccaaagtgctgggattacaggcgtgagccaccgcgcccggcctcaactcactgtacttctatttactgctgcttttggcaggtggacgtgggtcagtggccaagagtgcctgttgcagtcactcaggtcactcactgcaggacctgtgccgcatgccttgctatggagttttgtggtagcatttattctgcttggcctattaaaccacagtgcctagtgttttcttcatttttctgtctggcctgctgtggaacagttgtttcgtacattcctctggagctggaggagagtcctgtgatgagatcatagtacactctgtgatctcatttctggtaattttcttttagctttcaagcagatgctgaagctaatgctagataactagatacaatgtgtataatagaccctgtctttagttaccttattataggttgtcaaattttatttatttatttatttgtttgtttacttattgaaacagggtctcgctctgttgcctaggatggagtgcaggggtgcaatctcggcttactccagcttccacctcccgagttcaagcgattctcctgcctcatcctcccgagtcctgggattacagacgtgtgccaccgtgcccagctaatttttgtatttttagtagacaccccattgaccagtcttaattaatttacttttttgagacagagtcttgtgctgtggcccaggctggagagcagtggtgcaatcgtagctcatgcagcctcaaactcttgcgttcaggcagtcctccggcttcagcctcctgattagctgggactacaggcacctgccaccatgccttgctactcttttttttttttaagtagagacgaggtcttgctgtgttgcccaatcttccctttttgacctcccaaagtgctaggattatagacgtgagccactgtgcctggctggttgtaaaactttattgcttagaagaaccctcccacccccagtttgaaacactttctcagagtatgctcgtattctgcccatatcagtgtcactgggagagcatgtttaaaatgtggtgtcagccgggcacgatggctcacacctgtaatcccagcactttgggaggccgaggctggcgaatcacctgaggttgggagttcgagaccagcctgaccaacacagagaaaccccgtctctactaaaaatacaaaattagccgagtgtggtggcacgcgcctgtaatcccagctacttgggaggcagaggcaggagaattgcttgaacccgcgaggcagaggttgcggtgagccaagatcgtgccattgcactccagcatgggcaacaagagtgaaactcagtttcaaaaaaaattaaaaataaaatgcggtatccagggtgggtgcagtggctcacgcctgtaattccagcattttggaaggccaaggtggaaagatggctttagcctagaagttcaagacaagcctgggcaacttttttttcttgtttttgagacagagtcacactttgtcacccaggctagagtgcagtggtgcgatctcagctcactgcaacctctgactcccaggctcaaaccattctcgttcctcagcctccccagtagctgggattataggcatgtgccactacgcctggctaatttttgtatatatctatttttttctaggtggtgtttcgctgtgtcgcccaggctggaatgcagtggcacaaccttggctcactgcaacctctgcctcccgggttcaagcaattttcctgcctcagcctcctgagtagctgggactgcaggcgtgtgccaccatgccctgttaattttttttttgtatttttagtagagacggggtttcatcatgttggccaggctggcctcaaactcctgacctcaggtgatccacccgcctcagcttcacaaagagctgggattacaggtgtgagccaccacgcccggcctaatttttgtatttttagtagagatggagtttcgccatgttggccaggctggtctaactcctgatctcgtgatctgcccacctgggcctcccaaagtgccaagattataggtgtgagctaccatgcctggctgattcttaacagacattaaaatttgagaatctctgtttaggatttattcagaatcctaaggatgaatcctggatgaatatattcttcaaactaacttatttaaataagcctattagtctcttatctgtcatttcatagcacattgggaaattgacaattcgtgataaccttgggatgatggtcctcaatgagacaggcccatttcatcctgctagtgattagtgtgctgtattgtgcatcatggtaaagcacatgggccccagagtcaagcacaactgggttcagttcgtttcatcccttaccagctatttaatcttgggtgaactattcaaccttttatgctttaattttcccatctggaaataaaccccaaccctatattcaccaagaaaacaatggaagaaagggaaaagaagatgcatgtaaagaagtggttgtgaacccaggttgctcattagagttgtttagggaactttaaaaaaactttagccagtggggcgcgatgacacaacgcctgtaatcccagcactgtgggagactgagacgggcggatctaggtcaggagttcgatacgagcctggccaacatgatgaaaccccgtctctactaaaaatacaaaaaattagctgggcatggtggtgggcacctgtaatcccagctgctcgggaggctgaggcgggagaatcgcttgaacccaggaggcagaggttgcagtgagctgagatcatgtcactgcactccaacctgggtgacagagcaaggctccatctcaaaaaaaaaaaaaaagtctgatgcccaggcttctctctgattaagttaaaatttttagaagtgagaccaggtcactgatattgttaaaaactgcaggcaggctgggcacagtggctgacactataatcccaacactttgggaggccaagatgggaggactgcttgagcccaggagtttaagaccagcctgggcaacaaagtgaggccctgttgctaccaaaaaaaatttttatttattttttttgagtcagagtcacgctctgttgcccaggctggagtgcaatggcatgatctgctcagtgtaacctccacctcctggttcaagcagttctcctgcctcagcctcctgaatagctgggattacaggcccctgctcccatgcctggctaatttttgtatttttagtagagatggggtttcaccatattggccaggctggtctctttgccagcctggtctcgaactcctgaccttgtgatccgcccaccccggcctcccaaagtgctgggtttacaggtgtgagccactgcgcctggccagaaaaaaaacaaaaaccacaactttttaaaaattagctgggtgctgtggcgagcaactgtagtcccagctacttgggagggtgaggcaggtggatcacctgaggtcaggaattcaagatcagcctggccaacatggtgaaactccgtctctaccaaaaatacaaaaattagctgggcatggtggcgtgctcctgtaattcagttacttaggaggttgaggcatgggaattgcttgaacctgggaggcggaggttacagtgagctgagatcatgccatggcactctagccagggtgatggagtgagactgtctcaaagcaaaaaacaaaaactgcaggcagtattaaaaactagtaatataaagtgattacccaggcccctaggggtgcattagggctcagaacattttagctattgttattttttttcagctttgggtagtgatggtggtgttttgaagatacaggagtagaaatcagagaaacaggctgcctagggtgctagggatgttaggaccctaggaactgtaaccagcaggctagctgagggtacatcttttttttttttttttttctgagagttttgctccatcacctaggctggagtgcagtagcacaatcttggctcactgcaacctctgcctcccgggttcaagcgattctcatgcctcagcctcccgagtagctgtcactacagatgctcaacgccatgcccagctaatttttgtattttaagtagagatggggtttcatcatgttggccaggctggtcttgaactcctgacctcaagtgatccacccgcctcagcctcccaaagtggtgggattacagacgtgacatgagccactgcgcccggccttcatgtttagctctttaactttgcatccacccaatgccttgccgatagaaagatgtggcttgctttgtttctctgttccacgcatatggtactaccatttcctctgagactggctgttactgctcctttcctctgagaggctgatgtcaccagagtcaacaccagggcctctgaaggtgaaagatcctctgtgtactctgcctttttttttttttttttttttgagagggagttttactttgtcgcccaggctggagtgcagtggagtgatctcagctcactgcaagctccacctcccaggttcacaccattctcctgcctcagcctcccgagtagctgggactacagctgcccaccaccacgcctggataattttgtgtatttttaatagagacagagtttcaccgtgttagccaggatggtctcaaactcctgacctcgtgatctgtcagccttggcctccctaagtgctgggattacaggcatgagccaccgcacccggccctttttttttttttttttggagatggagtctcactctgtcacccaggctggagtgcagtggtgcgatcttgactcactgcaagttctgcctcccggattcatgccattctccagctccagcctcccaagtagctgggactacagacacctgccaccacgcccggctaattttttgtatttttagtagagacggggtttcactgtgttagccaggatggtctcgatctcctgacctcgtgatccgcccacttcagcctcccagagtgctgggattacaggcgtgagccaccgcgcctggcttttttttttttttttttttttttgtctagctctgtcgcccaggctggagtgcagtggcacgatcttggctcactgtaagctccgcctcctgggttcacgccattctcctgcctcagcctcccgagtagctgggacttcaggtggccgccaccacgcccagctaattttttttgtatttttagtagagacagggtttcaccgtgttagccaggatggtcttgatctcctgacctcgtgatccgcccgccgcagcctcccaaagtgctgggattacaggagtgagccaccacgcccagcctactctgcctttcaaagggaaggtgtgagtgagccaacttctcaggcctgatccttaaccctgtgtccactctgccttgttttgtatttgatgtgactacatctttctcccctctttcctcaactatcttctagtgctatgacaggaagaagcttttccttttgaagggggccccttctgacctccatgctgattgctctgtctttgtccttttctccttaggtcttgggcgtctttggtactggcttttttaggggtctgcctggggattacccttgctgtggatagaagcaactttaagacctgtgaagagagttctttctgcaagtatgatatttctgggggagagggatggaatgtagggttgtagggtaatgtgggagatatctgtggcagatggagtgcctaaggacactgcaggtgatagactgacttagggacattgcaggtggcctttaccttacttcccaacccttcacttggcaggcgacagagaagcatacggccaggcctctctccataccgagccttgctggactctctacagcttggtcctgattccctcacggtccatctgatccatgaggtcaccaaggtcaggagagacaaggaagagtctggtgggggtggggcaatggctgtggggtaatttggaaagggggaaattgtggccaacatcttgtcccagcctaatctttggacttttactttatgaagaaatgtgatcttggcctttaggcaaagggctcaaaggaagaaaccccttaggagagaatgggttcaaagagcattccatggtgtatcccatttcctttctccagatccaaacctctgtccccgcaggtgttgctggtgctagagcttcaggggcttcaaaagaacatgactcggttcaggattgatgagctggagcctcggcgaccccgataccgtgtaccagatgttttggtggctgatccaccaatagcccggtaaatttttcctgagaaacatccatttctgtggcccctttctccttcctgatgaacctttttttggttgctgatattctttcccaaaataaggtagtagttaactagcatagcaccttgccatactcctcaacctttccccacctcttcttctgtttcacttttctctttatccctttatcctcattcattcattcagcaaacaattattgctttttcctccctgacaggcctgggctggatgctggttatataagcagaaataaacaaggccctgtttatttacagatctcgttctccaggaatacaatgtctacctgcttgcttgtttgcttgcttccttccttccttccttccttccttccttccttccttccttccttccttccttccttccttcctcctttccttttccttagatattcagaataggattactcagattcttgtgtcatgatactctgtcaccagtgttccatgcatccatccatgactttctcttaaatacataattcagaaaataacatagtggccgggcatggtggctcaacgcctgtaatcccagcactttgggaggtcgaggtgggcagatcacgaggtcaggagttggagaccagcttggccaacatggtgaaaccccatctctactaaaaatacaaaaatcagccaggtgtggtggtgcggacctgtaatcccagctactcaggaggccgaggcaggacggttacttgaacccaggaggcagaggttgcagtgagccgagattgtgtcactgcactacagcctgggcgacagagtgagactccgtctcaaatactccaccctataaactcttcactcagcccaacccgcactgtcctgtacccttgacggctccagacgtaggtagtcgttattctgaagcttatccttcctttgccttttttttgttcttacagttgtattatgtgtgtatacatatgcacacatatgtctgtgtgcctaagcaataaattatatatattttttgtttttgagctttacagaggaagtgtcttagtgcatgtggtcttctggggtttccgttttttctttttttttttttgagatggagtctcgctgtctcccaggctggagtacagtggcgtgatctgcgttagccaggatggtctcaatctcctgacctcgtgatccgcccgcctcagcctcccaaagtgctggaattacaggtgtgagccaccgcgcccggctgggtttccgtttttcacataactttatttaattccatttcatatagctctagttcattcatttttactgctgcatattattatgttgtatgaatataccccaactgattaatccatttttaggttgataagccttggggttgtttccagtgttttgctagccaaagtgttgctacgaaccttcttgtacatgtctcctgttatccttgcttgggagtttctctttggtgtataactaggagaggaattgcaggattgtagaatatggagatgatcagcttcgcaagataaagccaaagtggtttaccaatttacacttccaccagtgatttataagaagccctcattgaagctgggcaagccaggatggtctcgatctcctgacatcgtgatctgcccatctcagcctcccaaagtgctaggattacaggcttgagccaccacacccggccagccttccctattattaatatgactatggttcatttgtgatacctagtgaattgatagtgatacattagttactaaagttcatacttgaggtttctttagtttttgtgtatgttctttttctgttccaggatttcatccaggatatgttattacatttagttgtcatgtttccttagggccctctagactgataaaatttcttagacttttcctttttcttaatgatcctaaaggtacttttgataaacagaaattcctaattttaatgtatttagatgtatcagtcttttaccttctgttgttagccttttgtttgttgtatttagtctttatctaccccaaggtcagaaaaaaatatatatatatatattttttgagacagagtcttgctctgttgcttaggctgagtgcagtagtgcgatcttggctcaccacaacctccgcctcctgtgttgaagcgattctttcttcagcatcagcctcccgagtagctgggactacaggcgtgcaccactatgcctgagtagctgggactacaggcgtgcaccactatgcccgagtagctgggactgcaggctcatgccactatgcccaagtagctgggactacaggcgtgcgtcactatacccggctactttttgtatttttagtagagacagggtttcactatgttgaccaggctggtctcaaactcctgacctcatgatccacctgcctcggcctccgaaagtgctgagattacaggaatgagccaccatgcctggccaaaaatatattttttaattttcttctaacacttttgctttcatttatttacttattttgagatcgggttatgagactggctaatttttgtatttttggtagagatgggtttttgccatgttgcccagtctggtcttgaacaccagggctcaagcgatccacctgcctcggcctcccaaagtgctgggattacaatagtgggccaccgagcccatcctaaagcttttacttttaaattttaagcaggctgggtgtgatggctcatacctgtaatcccagcacttcgagaggccaaggcggacagatcacttgaggtcaggagtacaagaccagcctggtcaacatggtgaaaccccgtctctactgaaaatacaaaacttagccgggcgtggtggtgggcgcctgtaattccagctactcgggtgcctgatgcacaagaatcacttgaaactgggaggcagaggttgcaatgagccgagattgtgccactgcactccagtctgggtgatagagtgagactatcttaagaaaaaaaaattttttaagtcataatctttctgcagttgatacttgtatctggtattagatagaaatatgatatcaaggggttgggcgtggtagctcatgcctgtaatcccagcactttgggaggccgaggcaagtggatcacttgaggtcaggagtttgagattagcctggccaacatggcgaaaaatcatatctcctaaaaatacaaaaaaaaattagccgggtgtggtggcacctgcctgtaatatcagttactagggaggctgagtcaggagaatcacttgaacctggaaggtggaggttgcagtgagccaaggttgtgccactgtgctccagcctgggcaacagagcgagactccatctcaaaaaaaaaaaaaagaagtacatcatttttcttcatatttggaaaatcattttttttcctatatggaaaatgttttttcagttccatttttgaatagttctcctttcctctctcatctgctatgccacctcttagtatttagtacatttaaaaaagtaataagtggccaggcacagtggctcacgcctgtaatcccagcactttgcgaggccgaggtgggtggatcacctgaggtcaggagtttgagaccagcctcaacatgaagaaaccccatctctactaaaaatacaaaattagccaggtgtggtggtgcatgcctgtaatcccagctatttggaggctgaggcaggagaattgcttgaacctgggagacggaggttgcggtgagccgagattgcgccattgcactccagcctgggcaacaagagtgaaactccgtctcaaaaaaaaaaaagaaaaaagtaataaatatgcttgggtctgtttctgggccctttggttctgtttattaacttgtctatccctgctctgttaccacactgcctatttctcttaacaggtagatttcccccggtcttctaaagtgtcattactcctcttggccctttgtacttccttatatttcttttgatatgtttcccaggctttctgtctctggtcgtgatgagaacagtgtggagttaaccatggctgagggaccctacaagatcatcttgacagcacggccattccgccttgacctactagaggaccgaagtcttttgcttagtgtcaatgcccgaggactcttggagtttgagcatcagagggcccctagggtctcgtgagtacaggggttgggactgcagggaacctagtgtgaaagagcataggggtgttgtgaggtctggcacggggaggagacggtggtgggacagccaggtagggcctgggggctgggagaagctctctgtcagggagggtaggaaccagacccgggtgcggttttttccatttcctgtacagaccaggaggcagtcacttttgtccctgagctgtaccctgggcatctctgggaggcctgcctgggtctgtgtctccttcttccccttctcacatcatcacatttcccagatttattttcttcgtttttatttatttattttttttggtttctttttccccccatctctggaagtttgtcgactgaaactcacttttatgtttctgtttttgtgttggttttgtgcctctttttccccttccctacccatctcctcctgccccagtttctcggataaggttaatctcacgcttggtagcatatgggataagatcaagaaccttttctctaggtaaatccatggccaccggtactgtatctgttcctctgcccttacccattcctcactctagcctttggggggaggtgccccagacccttccagcctttcactcaccccactttcccctgctgtgtgatgtctggtcctgttacctgttaccctggctgggagcccccagaagaaggaaggtgagatactgaaagtcaggtccttcgggaatgtagggagcttattgctttgccaggggatggagagatgctgcctattgctggggttcctgactctcagctgaggggcacctgaggttctgggcagagctacttgcccttgaaagcattttttggcagaatctcttgaagtccctatgtatgtctgtagaggcttggtatagtatgacccacatgcctttgcaaagccattgtgtcaggccaggaggctgaggcccagggagagcacttggggccagaatctctcagtagaggcaacagagccaggattggcattcataacccaggcccctgaatcattctgcctttctcttctgggatgttgacagaggctggtgttcaggcctgtgcctcctggtggcacttattcctcattttcctttctcatttctctccccatcctttgcaaacttatctgctcattgtgggttccctctccaagctttaacatttagtcccttcctccaatgccttcgttcctttggacccttggctctctattccccaacccctccttccactagcccctcgtccctgccccctctggattggagcagacagctctcctaccttccaggcaaggatcaaaagacccagctgagggcgatggggcccagcctgaggaaacacccagggatggcgacaaggcaagttggagcgggtgggtggttggaggatagggctggctgggagggtggaggggagaggcccatgagaaacttgaacttagtctccccatcagggatgggatttagttgatgggagcggggaaagagagaactggtatgattggagagtggtcctcttttcttcttaacagccagaggagactcaggggaaggcagagaaagatgagccaggagcctgggaggagacattcaaaactcactctgacagcaagccgtatggtgaggggctcgggttccttgggctggggtgcagggctcctttccaagcagaagctctgaagcttgtttgtttttcttccaggccccatgtctgtgggtttggacttctctctgccaggcatggagcatgtctatgggatccctgagcatgcagacaacctgaggctgaaggtcactgagtgagtcctatggtgacatcaggaagatggaggtgggcaggaaggagtcaggcctttagggagatgggtgtgcatattggatactctaggcaagcatgggtcatttcttgtgtccagaatcacctttggtgatagaaaattttttgagaaaggacaagaggagcctttgcttatctctcacctgtgtctgtggagtggtgttagcatataacgcagcctggggccagttagcagcccaagtctgtctgtttgcctgcaggggtggggagccatatcgcctctacaatttggatgtgttccagtatgagctgtacaacccaatggccttgtatgggtctgtgcctgtgctcctggcacacaaccctcatcgcgacttgggcatcttctggctcaatgctgcagagacctgggttgatatatcttccaacactgccgggaaggtgagagcacaggcacggggaaaaaggagggagtgaagcttccaggccttgaggcaaataggtatactaggggcattagctatttggggactgggtttaagaaggggctgtgggcctggtgggcagcatttgagttccctaatcactcccaggtgacacgctcactcacattcttagggaaggcattgcctattctgggctgacggaatgcacttattatcagtgtgttacgtgctaggtactcttctgggtgctggggatatagtgttaactgaggttgaaaaggttctgggctgggtgtggtggctcatgcctgtaatcccagcactttgggaggctgaggtgggcggatcacctgaggtcagaagttggagaccagcctggccaacatggcgaaacctcatctctactagaaaaacaaaaattagcagggtgtggcggcggactcctgtaatcccagctattcgggaggctaaggcaggttaattgcatgaatctggttggtggaggttgcagtgagcggagatttcaccactgcactccagcctgggtgacagagtgagactctgtttcagaaaaaaaaaaaagaaaggttctgactcacagggaggaagacacgttaaacacataacaaaggaggcaagatggggccgggcatgatagctcatgtctgtaatcccagcacttggggaggctgaggcaagaggatcgcttgaggccaggagttcgagaccagcctgggcaacatggcgagaccccatctctataaaaacgtttgaaaaataaaaataataagcaagatgatgccgggtgcagtggctcccacctctaatcccagcactttgggagggcgaggtggacagatcacaaggtcaagagatcgagaccatcctggccaacattgtgaaaccctgtttctactgaaaatacaaaagttagctgggtgtggtggtgtgcgcctgtagtcttagctactcgggaggctgaggcaggagaactggttgaactggggaggtggagattgcagtgagctaagatcacaccattgcactccagcctggcaaaagagtgagactctgtctaaaaaaaaaaaaaagaatgcaagatgagtttggggtgattaagtgctaacaaagacatgaaagagagtctttgttagcacttaaccaccccaaactggtggggtaggggtgggggctgtactgctttagatagtgtggtctaggaaagcctcactgaagaggccccgtttagtcttaccgaaagcagcttacatgagccagctctgtgtggactctgggagaaaattgctactttttgtcttggggttggaaaatgggagggcaggaggtgtctgacccctttgtggtcacctatacagaccctgtttgggaagatgatggactacctgcagggctctggggagaccccacagacagatgttcgctggatgtcagagactggcatcattgacgtcttcctgctgctggggccctccatctctgatgttttccggcaatatgctagtctcacaggtacatggttttccctgcctcattcttctgctcttttcttgtcgggtgattctatgtgttttcagagatcctgtgccccagcttgttttctaggtttatacccctcagcctgcctctagttcacaagcctccctcagtttctgggtgttgggcctgatcctcgttgtgacccccatccctcatgaacctgcaggaacccaggcgttgcccccactcttctccctcggctaccaccagagccgttggaactaccgggacgaggctgatgtgctggaagtggatcagggctttgatgatcacaacctgccctgtgatgtcatctggctagacattgaacatgctgatggcaagcggtatttcacctgggaccccagtcgcttccctcagccccgcaccatgcttgagcgcttggcttctaagaggcggaaggtaaggggttgcagtcacgcttggtcttctcagggtagggctgaagcatagtttagccttaaagagacctgaacacccctgttccttgcccccagctggtggccatcgtagacccccacatcaaggtggactccggctaccgagttcacgaggagctgcggaacctggggctgtatgttaaaacccgggatggctctgactatgagggctggtgctggccaggtaagcagacccagaattgagggagagttgattggccagcggggtagaatggtggctcttttgccccttaggggattgagagccacccttaacttctcccaggctcagctggttaccctgacttcactaatcccacgatgagggcctggtgggctaacatgttcagctatgacaattatgaggtagggaaggcctctccccatgacctgcgtctgtctgttccacctgcctccctgaatctctctcggcttgccaacccttctatggttgattgcctgcaacatatcagggggccttgatgatccggggagggccctgaaaaatgcatctttttagattcctaggagctctcttctctgacactgtttgtcttcttcctcccctctgtccttctgtccccattttctgcccacgttcccagggctcagctcccaacctctttgtctggaatgacatgaacgaaccatctgtgttcaatggtcctgaggtcaccatgctcaaggatgcccagcattatgggggctgggagcaccgggatgtgcataacatctatggcctttatgtggtaagggcctgagagaggagagttggtggaaagagggaaaacagcccagagactgagggcctagggaacttgcaccagatgacagctggcttttgctcctcactacccgtctcttctctcctcacccagcacatggcgactgctgatgggctgagacagcgctctgggggcatggaacgcccctttgtcctggccagggccttcttcgctggctcccagcgctttggtaaggtttagagaatggagctgtggcagaagggtgtgaaggccagatctcaggagccatggacctggacctgcctctctgaggaatgggagccacacactgcatctgtttcctctcagctatgcgctttgaaggaagtcagggtgtgggaggtccactccttgttcaaatgttcttgtgaactgcatcttcagcagggttctggggacccagagcggatgtgggaggtcagccatgtaaaaagctgaactcctttaccatgtgcaagctccccacttcttgtcttcctcaggagccgtgtggacaggggacaacactgccgagtgggaccatttgaagatctctattcctatgtgtctcagcttggggctggtgggactttccttctgtgggggtaagacagggaggaatttggggtcttggtttggtgggaaaggggcaaagtagagggcacaggaccaaggtgttgtaagcaaagagagttgagagtccaagttagggccttgggaagtttctcaagcagtatctctccttcaccctcttttccaacctgcttcctctctctcctctaccagcggatgtgggtggcttcttcaaaaacccagagccagagctgcttgtgcgctggtaccagatgggtgcttaccagccattcttccgggcacatgcccacttggacactgggcgacgagagccatggctgttaccatctcagcacaatgatataatccgagatgccttgggccagcgatattctttgctgcccttctggtacaccctcttatatcaggcccatcgggaaggcattcctgtcatgaggtgaggcattcacttgggctgtgaagagtgggctgaggtggctgggggtattagggactgggcttcatctctgggtctctttcttcactcactacagccttgtaaaggatggaaaatcattaaggtcaagagtgaaggggagcttaatggagatgaataatagtaaacatttaaagaaaattgacagcagtcataagctctttcagaaaaataaaacagggtaatgggattaggtggtcataaaatccctttttgaggccgggcacagtggctcacacctgtaatcccagcactttgggaggccgaggtgggcagatcacctgaggtcaggagtttgagaccagcctggccaacatggcaaaaccccatctctactaaaaatacaaaaattagctgggcatcatggcgcctgtaatcccagctactcgggaggctgaggcatgagaatcacttgaacccaggaggtagaggttgcagtgagccgagattgctctgctgcattctagcctgggtgacagagggagactccatctcaaaaaaatgaaaaaaaaaaaaaaaaaaaagttttgagaagaaggctgtgtgagatgaggcctgaatgagtgggacagaccatgttatgtaggaagaatcttccaagcagagggaattgcaagtacaaaaattctaaaggagaaattagtttgttatgtactaggaatagaaaaaaacagtatgtcttgggtaaagaagcagaaggagagctaggagatgagattaagaagaaagtgtgatctgctcctggagggccttgcaagccagggttgcaacccagggttgtaagccagggcggtgaaacatgcaaggaggctactggcaggctgctgtgcagcatggtttcagtagagggcagagaagaagcagggagatggcttaggaagttaaatgtctaagactggattgtataactgagacctgaaccccaacccgactgtctgactgcaaactcctgggtcttaacccctgtgctgttcttttcttttctttttttttttgagacaaagtctcactctcgtcccccaggctggagtgcgatggtgtgatcttggctcactgaatgcactccgcctcccgggttcaagtgattctccagcctcagcctcctgagtagctgggatcacaggtgcctgccaccatgcccggctaatttttgtatttttagtagagacggggtttcaccatgttgttcaggctgatctcgaactcctgacctcaggtgatcttcccgcctcggcctcccaaagtgttgggattacaggtgtgagccaccacacccggcctatgctgttcttttcttattgccagttcctggaggagcatttctgacttgtgccaaaattgaaaagttttcctttattgtctttcttccttcctaggcccctgtgggtgcagtaccctcaggatgtgactaccttcaatatagatgatcagtacttgcttggtgagaaatgaggatagttggtggtgggttggctttgggccaagcagcactgcggatgcccagggagggactagtgaagctggtggtgcagagggcaggcactttggtgttccctgttctgggaactaatccccctattcagagttgattctggcatattttaggggatgcgttgctggttcaccctgtatcagactctggagcccatggtgtccaggtctatctgcctggccaaggggaggtgagttaaggaagggcatggtggggaaagatggtggaagccaaaggaggcaaacaggacgggacccctgtgcactgagtgatccggtatcttacctcttttgtcactcacaggtgtggtatgacattcaaagctaccagaagcatcatggtccccagaccctgtacctgcctgtaactctaagcagtgtgagtaagcctggtctggctgccggttccatctccctgtaaatttccagaaggggagggaatgtgtgccttagggtccagtacctatgtgggcatacatgagtaagcaaaacatgctgtggggcccaaggttggacaagggggcaacttcatcctggcattgctcttgccctagatccctgtgttccagcgtggagggacaatcgtgcctcgatggatgcgagtgcggcggtcttcagaatgtatgaaggatgaccccatcactctctttgttgcacttagccctcaggtaagtgcataggcagcgagtctcctcagccatttgcctgccttcctaggactcagttctctggggttgtgcccctcactccctcttgggctcaggcgctcacctatcccacttcttgctcagggtacagctcaaggagagctctttctggatgatgggcacacgttcaactatcagactcgccaagagttcctgctgcgtcgattctcattctctggcaacacccttgtctccaggtaatgggtcacccactcttccttggctgcctttgctggggcctgatccttgtgggggctcccagttcactgtgctcttttctcacattctgaccttgctttgggtctcctccttccttctgttctgttatttttccccctgatggacatctgcttttaccatctccagctcagcagaccctgaaggacactttgagacaccaatctggattgagcgggtggtgataataggggctggaaagccagcagctgtggtactccagacaaaaggtgagtgaccaatctggcccctaggatgggggaaggaggggaagccggggcaggtttagggatgcccttgcctgtaggaacgttgttgttatgctatagcccattggtatgactatggcactcttttattcctcctccaggatctccagaaagccgcctgtccttccagcatgaccctgagacctctgtgttggtcctgcgcaagcctggcatcaatgtggcatctgattggagtattcacctgcgataacccaagggatgttctgggttagggggagggaaggggagcattagtgctgagagatattctttcttctgccttggagttcggccctccccagacttcacttatgctagtctaagacccagattctgccaacatttgggcaggatgagagggctgaccctgggctccaaattcctcttgtgatctcctcacctctcccactccattgataccaactctttcccttcattcccccaacatcctgttgctctaactggagcacattcacttacgaacaccaggaaaccacagggcccttgtcgccccttctctttcccttatttaggagccctgaactcccccagagtctatccattcatgcctcttgtatgttgatgccacttcttggaagaagatgagggcaatgagttagggctccttttccccttccctcccaccagattgctctcccacctttcatttcttcctccaggctttactcccctttttatgccccaccgatacactgggaccaccccttaccccggacaggatgaatggatcaaaggagtgaggttgctaaagaacatccttttccctctcattctacccttttcctctccccgattccttgtagagctgctgcaattcttagaggggcagttctacctcctctgtccctcggcagaaagacgtttccacacctcttaggggatgcgcattaaacttcttttgcccccttcttgtcccctttgaggggcacttaagatggagaaatcagttgtggtttcagtgaatcatggtcacctgtatttattgctaggagaagcctgagggtggggggagatgatcatgtgtgctcggggttggctggaagccctgggtggggggttgggggaggactaatggggagtcggggaatatttgtgggtattttttttacttcctcttggttcccagctgtgacacgttttgatcaaaggagaaacaataaagggataaaccataaataactggtggtagtctggattctagttctagcctgagccacagaccctagaagcctagagaccttacatttgctttcctttttttttcttttttgagactgagtctcactctgttgcccaggctggaatgcaatggcatgatctgggctcattgcaacctctgcctcccaggttcaagcagttctcgtgcctcaacctcccgagtcgctgggactacaggcatgcgccaccatgcccagctaatttttgtatttttattagagatggggtttcaccatgttggccaggctggtctggaactcctgacctcaggtgatccgcctgcctcggcctcccaaagtgctggaattaaaggagtgagccactgcgccctgggtctttttttttttttttttttttttgagacagagtgtcgccaggctggagtacagtgtgtgatcctggctcgttgcaacctctgcctcctgggttcaggcagttctcccacctcagcctccttaatagctgggattacgggcacctgcgaccatggccagcttcatttttgtatttttagtagagatggggtttcgccatgttagccatgctgatcttgaactcctg

SEQ ID NO: 106 - DNA, 2587 bp, Homo sapiens
tcagcttgtgcctggctttgagcagccacaggcagaaaattgctgcattgtcccgacattagggcaactaatgcggcgttgcgggtataaccagagcatgaagtgcataaagaggcgtcgccttggcatcttcatcagtcccgagggagcccagagccctgtcatagtcagtgaggcagcctgtggccagctggcccatgtacctccccagtaggtgacccctggaatgcttgcactccagggtatcaaggacttggcaagtgggactggagaacttacggggattgggacaggatgggcatggagggggtgggcatggcaggggtcctcagactggggaagtggtggaggccagagagataaggaaaagacagataaaggggaggggggggtccctcgggagacagggggggtcctgaaggtgagaggaagcctaggctatgggagggggctgagggaaggaggtggggagcttcccagtgcgtcctccctcggtcccctcctcctcaaggtttctagagtccagagggcctcattgacatgtaaacgagggtccctataaaggcggcgctgcctcgcactggtgcatggactgcaacatgggcacggagcctgctgcccggggcagcctccccggcaacttccgaaaggtctggggtcttgagggactaggggcaggcacccttccccgggaggtgtgggggggtgccgagggcaggagggtggcagtcctgcactctaaaggctgttcatctgcagatttccaagccgctgatggagaaaaagcgccgggcacgcatcaatgtgtcactggagcagctcaagtcgctgctggagaaacactactcgcaccaggtgagactcaggcggggtgggggtgggtgggtgatacgatcccaacctccctctctccacctcgggaggccggtctaatagacctttccatggtcgggtagatccggaagcgcaaattggagaaggccgacatcctggagttgagcgtgaagtacatgagaagccttcagaactccttgcaaggtataggggagggctggagggaggagggggaggcttgtgggatcagagccagggatgcacaaggccaaataaagagggatacctcaaggaccgcttgaccccgggcttttgagaccagcctgggcaacatggcaagacagcaaatataaagaggacaactcggaggcaggtgcagttggtgaggagggggccccagctcgctagggggcgagggaggagcagtaaagcccgggctggctgtgcgattgcaatctgggtggtaggtctggaccccgggggagacgttcgggtcgtctgacctccgccctcctcttcccttcctcaacacgcttcctccctcctttcccctccacctccactcccctctcctccctcccttcctcccctcccctccctcccccttcccctcctctccctccccctccccttccccttccctctcttcccctccctgtttctcgcgtccgctcttccccacagggctctggcctgtgcccaggggagccgagcaaccgtcgggcttccgcagctgcctgcccggcgtgagccagctccttcggcgcggagatgaggtcggcagcggcctgcgctgccccctggtgcccgagagcgccgccggcagcaccatggacagcgccgggttgggccaggaggcgcccgcgctgttccgcccttgcacccctgccgtctgggctcctgctccggccgccggcggcccgcggtccccaccacccctgctcctcctccccgaaagtctccctggctcgtccgccagcgtccccccgccgcagccagcgtcgagtcgctgcgccgagagtcccgggctgggcctgcgcgtgtggcggccctggggaagccccggggatgacctgaactgaaggcgctccctatttggtctcgcgacacagggactattttcagcacgcccacagtgactgccaggaccccccagtcgtccgttctggtcgtggggcgggggtggcttggagagggccgcgcaccccgcaagcgcagggaaatacccccagccctgccggactgggtctgcgcgtctgggcataatccacccccactctagctccacctacacacgccggaccgctcgctctccgcccatcctccggaggggctgggagggggtgtcctgggctgcgcccctttcccagggacccctggcgggcaacccgcccgcccccacccccgcccggttgccgcgcagcggtgggaatgtcgcagttggcaacagcgcagagctgacccctcgcagcgaggagaatcgctgccccgccccggaccattcagcggaccgcgggcgcccggttcccaccggcacaaagcgcgcctggccccgccccgccggcaaggggcccccagcctcccccaacccgggatcctcttgacttccaaggacctccttcgcaagcggtgctgcccaccgggctggcgcattccccgaggcccacccttctcagaagccccgcccctaagatgcaccgccccaaccggacgccccgcccacgcggttcctggaagggacccattgcttggt